European Patent Application EP 4 640 056 A1, published October 29, 2025. Title: ISOLATED BACTERIOPHAGE AGAINST XYLELLA FASTIDIOSA. Applicant: BIOLINE AGROSCIENCES FRANCE. The sequence listing filed with the application follows.

SEQUENCE LISTING (37 sequences)

SEQ ID NO: 1 - DNA, 55087 bp, unidentified
  source 1..55087: mol_type = genomic DNA
gggggcgctgacctcggtgctcgcgcatttttcggaattttcgcggtttcgtctcctttggacccccggagctgcccgaatttccgaatttattccccgaataaacgcgaatttcctgtgacagtagtgacagtgacgtttttgggtactgtcacaaattcggccccccaagaaatccgctcaaatcaacgatttacaggcgcgaatttactgcgagtttaggctcagtgacactgtgacagtgacttccaatcctttacggcggaaagaaaagttctgcctgccaagaaaattttctcgcgtatgagagaaggtactgtcactactgtcactactgtcacaagttagggaaaaaggtaggcagatcaagcacttgaatttgtgacagtaccttgtgacagtgaccgctttgcgcctcgaagagcatggaaaatagggtactgtcacaagaatcggcctttttccgaatttccgtccatacggttggaattttttccgtatgtgacagtgaaaagaattcggaattaatttaatcggaaccgctgcgaggcgtcgtgcggaaattcggaaattccgggcaataaaaaagccccgggggatgagcccggggccggcactgcggaaattccgccgaattaaattgcgttcttcggcgctccgtcgcctacgcgcacgtcctcgacgttcgagccgttgtcacccgcgcccggcgggagcggatcgctctcgtagcggttcgcgtcggtgttgcccggatcgacgctcgcgttcggcaccgcaccttgctgcttcggtgcgccgaagaactcgccggtctcgcgcgctgtgacctgcaagtcaccgtgcatcgtgatttcgaccgaacggccgggcgcatcgagcactgcatgcacaacgccattgccgtcgaccaactcgactgccttgttgccgatgacgtgcgtgaacttcacggtagatgtcatgtcgtttctcctgtgctcgggattgagcgtcttcgatcatacgcttgcaggcatgaaaaagcccggttgcccgggcttcttcgatcacaccttcagcgacgtgatttctatgtagtcgtcgatccactgctgaaggttcggccgcaccaccacgtcgggcgagcgcgaccaataccgggcctgctttccattcgcgccgcgcgcgcggcccacgtacacgaagcccttcgaggtcaggaagttcgacagcttcggcccgtacggcacgccgacactgttgtccatcgcgaggtcacgcagcttcccgacgttgagcagcaggctcgtcacttccgggtcgcgcgactccgcgatcatctcttcgatttcgtcttcgtcgtcgccgcgcgcgaggtcgatcatgcgcgccttcgcgtcggtcatgggcgcatggccgtccgggtcgaactcaggatgcagcgggtagtcttccagccactcgcggatcgcgcccgggtgataggcgattgcgttgaagatgtcgtcgtagtgatccgggttgcgcgcgcggaacttctcgatcatctgcttcgtctggaagtgggtcgagatgacgaagtagcggcggtcggcgtcgtacaccggcagcgcatcgctgtggttggtcaagatgatcgtcgaggtcacgttcggcacgttgtacgagtcgcggtgcatgcggcgaatcgaaaccacgtcgttcgtgatgaagggcttcagcttgtccatcaccgcgtagcgcgacgtaccgtggatgcgtgcctcttcgagcaccacgaccttgcgcgactcgaagaacgacgtgtacttctcttcgagcgcctgagcgttgacggtctcgacgttgttgcgcgacatgatcgccatgagcatttcaccgacgaagcccttgcctgcgccgtccacgccctgcatcacaaccgcccaacggattttcttgtccatgcgcttgatcgtgtaagccagccacgagagcaggatttcgcgctcgcgctcgatggggtacgaaatctcgaagtgacgcttcacggcttcgactgcgcgccgggccttgctgctcagcttgtcgggcaccggcacgatgtcttccgggttgaacttgttcgcgtgcttctggccgtcccactcgacgatgcggtctgcgccgggcaggtaaacgtagccgctgacgaccgggacttggtacacgttgagcgcgagtgcggcggcctgttgctcaggcacggcttccatgttcgagcggtctttcttcgacagcaggaaacggttgttgcgcgcattgaacgcacgctcgctcagcgcgaggcggttgtccatgtagtagaactcttcctcggcgtcgacgtacaccacgtcgttgcaccaatgtggcagttccttgtagttgaagtcggagttgcggtagccctcgttgatcgccttgcggatcatcgcgatgggaaccttcttccccagctccgcgacgcgctccttgatcgcgccggccaacagctcgacttggaagtcgctttcgagcatgcggccccacttcgcagcgagcgggccaagcaactccatctcgctcgtcgtctcggcgaccttgcgcttgatcttctcgaactgttcctgcgagtgctcctgccgatgctccttcgccatcttgataagcgaggcggccgtcgtcaggttgcggcccatgtcgtcgtggaacgagttccacttgaactccaattcgtcggggtcgtagttgtgcgctggctccgaccactcgtgccacaacgtcaagccttcttcgttgccgtcgaattggtgatgcagcgccatgccgaccttcaaccactgctcgtagtcgtcggcaccgggaacccattgcagcacttcgcggagctggtcttcggtcaggttttccagcgggcgcttgtattccagcagtgcgttgtcgttctcgtcgtcgctgctgcgcgactcgctcggtgcgttgtgcttcttcaacgtccatccgcgacgctgcgcttcgagcttgaacaccgagaagagttcgtcgatgtgctcggttgtgatttccggcagcatgtcggccggcacgctcagcgggttgagttccttgcccgaagtccacttgtacggcttcttggtatcgggatggatgccgatgccgacgaactgctggccgtctgcgagcacttcgatggactgctcgtggccctcggtgtcgaggaacgtgatcttccgcttcgagaacggaatgtcagtgcgatacacgagcaacgtcttcggcgcacggccgacgcgcgtcatcgtcttgccgatgatttcctcggtgtgctcggccatgagcgccgccatctcgtcatcggtgatgtcgatgtcgaccgcaggcgtgtgcttcgtgtggaagccgatgttgccctgcttgtagttgccgctcgcccacttgcgaacgagcttttcggtggcttggattttctgccactgcggttcaatcgggcctttccttcctgccgggatcggcaagatggagtacccgttttccagcaattgcgcgccgtacttacggagcacgctggtgatcggtcgtccagcagccataggtcactccgcgatgtcgtcgctaacaaggtcttcgaggttgaagccgatcttgcggttgaaatccttgtgcaagatggtcgccttgtcgcgcggcacaccgccgaggcgctgccaacgcgagacagtggtctcgtgccagttgtacttctcgcaaattgcgttgagccgaccgtacggcgggtcgagcatgagggcgatgcgccgaagcagatagcgcactcgcgcgtctgcgctgtccagtgaatcaagagtagggtctcggcgcatgaattcctcgcagacgttgggatttaaggggtctgctaagtcggtgagcatgcctattgacttagcatcgggacaggcgcatagtgcgctcgccgggcaggaattgcaatccacccgtcactcccgaaaccaacctagctaggagatacaaccgatgtcgaagatcaacgcgaagaagctcgccgaagccatcaccctcatcatcgaagcagtcggcggcggtgccgccaacgagtccgaggatgcgggcggcgaagaggaagcgccgaagaagggtcgcggccgtccggccggcagcaccaacaaggccaaggccgagaccaagcccgccgccaagggcaaggccaaggcgaaggacgaggacgaggacgaggacgacggtctcggcgacgacgacgatgccggcgacgacgatgacgacctcggtctcggcggcgacgacgaagaagtgacgcaggaagatgtcgtcaatgcgttcaaggcgctgaaggcgagcaagggcatcgacaagtgccgcgaagtgctcgccaagctggacgagagcaacgtgctcaacatcccgccgaagaagtacgccgaggcgctgaaggaaatcaaccgcgccgcgtcgaagaagtaactcggcctgcacgtcacacgaaacgcccgggttcgctcgggcgtttctttcggagaggaacacatgcccggttcgcacgcccgcttcgcaccatcgtcggcgcatcgcatctacgattgcccggcgagcctgttgctcaacgagaacgagcccgaccgcgaaatctacgaagcggccgagggcaccgttgcacaccacatcgcggaaatctgcgcacgcgcgcgccgcgagccggaagagtttctaggaatgacgttcgacagcggcgacctcgacgccgactacgacgaagagcagcattcctcgaaaggcttcgcaatcaccgtcgacgacgagatggtgcagggagtcggggcgtacctcgaccgcatcatgggcctgccgggcgaccactacgtcgagacgcgcgtcaacatctccccgtggtgcccgatccccgatcaattcggcacctgcgaccacgcagccgcgtcgcacaagaagctcatcatcaccgacctgaagtacggccgcgtgcaggtcgatgcgccgcagaacaagcagctcgtgatgtacgcgctcggcttcatcaacgagtacgactggctgtacgacttcgatgaggtcatcatccgcattgcgcaaccgcgcctcgatcacttcgacgtgtggatcaccagcaaggccgaactgctcgctatcggcgagaagatcaaagagcgcttcgcgcttgcgttgaagccgaatccgccgttcggcccgagcgagaaggcgtgccgcttctgcaaggtcaacttcaagtgccgcgcgaaccacgacttcctgtaccacgagcgcatcatgctgctcgatgacgacgacgagttcgtcgagcctgacctcatgctcatgagcgacgacgaaatcgctgcgctgtggctgcgcaagggcatgtacgagaaccgcatgcgcgcggtcgaagactacctgcacaagaaggtcgcggacggcgacttcgtgccgggcctgaagaccgtggcgggccgcagctcgcgctacttcaccagcgaaatcgacgccgagctgctgctgctggaagccggcgtgcccgagtctaagctgtactccaaacccgaattcgtgtcgcctgcgcaggctgaaaagctggtgcgcggcgaggcgaagaagaaattgcaggacttcatcaagtcgaagcccggcaaaccctgtctggtctcttccgacgacaaacggaaagacctgaccgtccagtcgctcgaactgctcgacgactgacgcaaccgttgtacgaatgcgcgaaagcgaactacgaacgtcgaatgacgaaggagaaatcgaaatggcgaagaagaaagttggtgatctggtcgacaagggcaatgggcgttttctgctgaagaacgtgcgcctgagcttcccgtacttgttcgagcccgacgagcaggaagacgacaacggcaacaagaagaagtcgtaccgcgtcaccctgctgctcccgaaggcgacgcacaagcccgtcgcgcagaagctctcccgtctcatctccgagatgtgcgaggaagagtacggcaacccgaagctggcggccgaccgcaagttcctgcgcgatggtgacgagtcggatgtcgaagatcatcacggctgctggacggtgacggttcgcgagacccggaagccgatcctcgtcgaccgtgatcgtcagcccaccgaggaagacgacgagctgctgtacagcggcgcgtgggccaacgtggtgatccgcccgtgggctcagaacggcaagtccatgaagaagaagaacaagtacggcaagcgcatcaatgccggcttcgacatcgtgcagttcgtcgaccacgacgacaacctcgcgggcaacgctcgcccggatgtcgacgaggttctggatgagctggacgacgacttcgcggatgacgacgacaacagcaccagccgcagcaagtccaagagcaagtcgaagggtcgttctcgcgacgaggacgatgacgacgacgggctcggcgacgacgatgacgacgaccgcagctcgcgccgcagccgtccgtcgaagagcaagaccagcagcaagagccgtcgctcgcgcgacgacgatgacgatgacggcgacgaggacgatgacgacctcggcatctaaaatcgggcatcggtaagcggtacctacggtcgcccgggcactccccgggcggctgtttttcagggatacggtatggacaagctgcatcacgacttcgagaccttcagcaagtgcgacctgaagaagcacggcttggcgcgctatgctcgcgacaagtcgaccgaagtgctgttcctgtggtacgcattcaacgacgaggaacccgaagtgtggttccccgcgacggagccgatgccgaagcgcctgcgccgcgcgctcaaagacccgaacgtgcagaagtgcgcgcacaacgctcagttcgagcgcgcgatttggctgcacgtcctcggcatcgacatcccggtcgagcagttctattgctcgatggcgcacgcattctggctctcgctgcccggcaacctcgacgaactctcgggcgtgcttcgcctcggcgagaacgcgaagatgaaggaaggcaagtcgctcgtgaagttcttctgcgggccgcgcaagccgacgaagaccaagcagtacacgcgcaacaccgcgcagaccgatccggcgaagtggaagacgttcgtcgagtacggccgccgcgacgtgatcgccgagcgcgcggcaggtcgcaagctctcgctcttcccgatgagcgatttcgagcgcaacctgtggtacatcgaccagcacatcaacgaacgcggcattccgttcgacaaggaattcgtcgagaccgcgctgcgcgtcatcgcgaaggagaagaagcgcctgctgggcgagatgagccgcatcaccggcctgagcaatcccggcagcggtgcacagttgctcccgtggctgcgcgagcgcggctacccgttcaccaacctcaaatccgcctcgatcaagaaggcacgcgaggattgggactggaacatgaccgatgaggcgaacgcggttctcgccttgcacgcggaagcggcgcgttcgtctgtcacgaagttgcagaagatgctcgacatcgaagtcgacggagtgctgtgctacacgatgcagttcgcaggcgcggggcgcacggcgcgctgggccggtcgcgcagtgcaggtgcaaaatttgccccgccccctccgcgaactagaagagcaaggggcactgctcatggcgcgcgatgcgatcatgcgcgaagacatcgagttccttcgcctgctggtgtcgtcgccgatgggcgcgattgcatcgtgcatccgcaccgcgatcaaagcgccgcccggctacgagtatgcaacgtgcgacttggcctcgattgagtccgtcgtcattgcatggctgtcgggctgcgacaagttgatcgaggtctttcagaagaacctcgacgtgtacaaggtgttcgcgtcgaagatgtacaaggtcgactacgagcaggtcgagaagtggatgcgtcaacacgcaaagcccggcgtgctcggcgcaggcttccgcctcagcggcggcatggagttgggcgagtacccggaagtcatcaagaccggcctgtggggctacgcggagaacatgggcatcgagatgtcgcagaaggatgctgcggccgtcgtgaaattcttccgcgaggaatacaccgaaatcgtcgagctgtggtacgagctggaacgcgccgtcgcgaaggtgatgaacacgaaggagccggtgcgcgttggtccgatcctcatggacgtgaagggaccgttcctgcgcatgcgtctgccgtccggtcgctacctgcactacctgcggccgaagatgatctggaagaagatcaaggtcggcatcgacaagaagaccggcaagccgaaatacaagtcgaagaagggcttcacctacgaaggctacaacacgaagaagaagtggacgcgcatcgactcgcacggcggcaagatcgtcgagaacttggtgcaggcaatcgcacgcgagctgctggccgccggtctgctgcgcgcttggaaggccgggctcgatgtgcgcatgcacgttcacgacgaaatcgttgcgctggtcaagcgcaagctgtcggacatctcggccgcgacgctcgaagagcagatggtcaagaagccgaagtggtggggcgaagacgttccgatccgtgcgaaggctgacgtagtggagtgctatcagaaatgagctggctgaccgattggcgcaacgtaatcaacggcaagccgccgcgcggcgacatcctgccgaccgacaagcatcgcgtcgaaaaggacgtggagcagaagtggtgcgccgttgcgaagcggcacggatggaaggcatacaagttctcgtcgcccggcaacagcagcgttcccgaccgcatgttcatccgcaacggcttcgtcttcttcatcgagttcaagcgccccggcggcaaggcaaccgacaatcaactcgaagagcacaaggagctgcggcgcaagggcatgatcgtgtgggtcatcgactacttcgataaagaattcgccgagtggatttttgaatgaaacaactactgaagcgctccgacctcgacgagtttcaaatcgctgccggcctgttcctcgaacgggtcggcagttgcgcgttgtggatcgacatgggcctcggcaagaccgtggtcgtgctcacgcatgtttcggacaaggtgttctccggcgagtggagccgcgtgctggtcgtaggcccgccgctggtcatctccgatacgtggtcgaccgaggtcaagaattgggagcacacccgcttcctcgactatcaggaactcgacggcgacagcgagcacatgcgcatgcagttgcagcggccgtgcgaggtcgacggcatctcggtgcataaactcgggcgtctcgcggcgctgttcaagcgaggcgacacggtgccgtgggacgcggttgtgttcgacgagtcgagcatgttccgcaacaagtcgtcgaagcgctggaagtacggcgtgcgcctgacgtggggccagccgaacgacgtgatcgagctgacaggtacgccgagcccgaacggcctgcatcaagtctggtcgcagattgcgatgatcgacggcggcgagcggctgggcttgacgtacaagaagttcctgttccgctggttcaagcaggagttcatgggccgcaaagtgattccgaagtcgcacgcgatggcgtcgatcacgaagaagctgagcgacatcgtgtacaccttgcgcgaagaggattacgtcaagttgccgccgctccgctctacgcctgtgccgatcatcctgccgccggatgtgatggctcgctatcaggaattcgagcgcacgtctgtgctgaagtggggcgaagagcaagacccggcagtgcgtgctctatcggaaggcgcgctgtacggaaagctgttgcaatttgcgtgcggtcgcatctatacggattcagagacgaaagagttcgtcgacatacacgacaagaagatcgagcgcctgaaggaaatcgtcgagttcagcgacggctcgccgatcctcgtggcacgtacgtggcagcactcgcgtgatcggctgcgcgatgagttcccgggcatccgctcgttgaagacgaagcgcgacctcgacgcatggaacgcgggcgacatcgagatagccgagacacaccctgcgagcatcggtcacggcacgaacatccagaagggcggcaacaacctcatctggtacgaccacacgcccgacctcgaactctacatgcagttgcgcaaacgactgcaccgacgcggccagacccgaagccacgtcaacatgatgcacctgacagcagtaggcactatcgaagaggatttgacacgcgagctggtcaagaaagaaattacccaagacgccctgagagaacccatgcggcgacgagtcgcagacgtacagagagaactagccaatggccgcacctaagatcgactacgaagaagagtttttcgacggcatgaccgtgccgcgtctggcgcagttgttccgcctcgaccgccgcactgttaccgagaagctgcgtccgctgcgaccgaccggcgaccggcgcggcgcaccgacgcatcacatcgtcgacgctgcaccgtacctcgtggagcccatcgtcgacatcgccaagtacctcgcggaagtcggccccggcgacctgcccgcaccgctgcaagcgcagtattggaacgcgcagaacagcaagttgaagtacaaggaacagtcgggcgacttgtggcgcacgcaacaggtgctcgaagtgctgaccggcgtgttccgctcgctcacgcaatcgcttcgcctgctggccgaccgcatcgaagcgcagaccgggctcacgccggagcagcgcgcgatcatcgagcgcgaagtgtcagacaaggccatcgacatgctgcgcaagcgccttgtcgaagacttcgagatttacgtcggcatcaaggacaaggaacagctcgccgacatcaagctcgacgacatcggcctcgacgaagaggacgaagaagatgtctgacggcagctttttcaacgacctcggcgagctggtcacgttcgttgccgatagcgttctggttccgccggagcgcttgaccgtttctcaggccgcagcaaagtaccgctacctcgacaacgaaggctcgttcgtcggcgagtgggacaacaacgaaacgccgtacctcgtcgagccgatggacgtgctcacgagtcgcgagttcgagtcgtgcatcttcatcggcccggcgcagggcggcaagaccgaaatcatcctcaattggatcgcatacaccgcgaagtgcgacccggccgacttcttcctcatccagaccgcgcgcgacaccgcacgcgacttctcgtatcgccgcatcgacaagatgcaccgcgacagcaaggagctgggcgcgatgctgcgtccgggcagcgacaacgacaacatcttcgacaagttctaccgcaacggcatgatgctgacgctgggctggccgacgatcaaccagctctcaggcaagccggtgccgcgcgtcgcgctgaccgactatgaccgcatgccgcaggacgtggagaagaacggcccgccgttcccgctcgctcgtaagcgtacgacgaccttcggctcgttcggcatgacgctggccgagtcgtcgccgtcgttcgacgtgaaagacccgaaatggaaggcaccgcacccggactcgcatatgttcccgccgtgcgatgggatcggcggcctgtacaacgaaggcgaccgccgttgcttctactggcagtgccctcactgcggcgagtggtttgagccgaagttctcgctgctgaagtgggacatcaagaaccccgacccgttcgaggctgcgatgtcgacgatgatggcgtgcccgcgtaacggttgcgtcatcgagccgaagcacaagtacgagatgaatcgacgcggcgtgtggctgcgagaaggccagcgtattgatcgcgacggcaacaagctcggcgtcggcgttcgctcacgtagcgcatcgttctggctgaaaggcccggcggcgcgcttcattacatggcagaccctcgtcgagcgattcctgcttgcgcaccagacgctcgaacgcacgggcgaaaccaaggcgctgaaggccacgatcaacaccgatcaaggcgaagcgttctggccgctcaacgcgaaggactcgaaccgcctgccggaagacctgcaatcgaaggcgatccagtgggccgacaagaaggtgccgtacggcgtgcgcttcctgctcgggactgtcgacgtgcagaagagccgcttcgtcgtgcaggtcttcggcgtcggcccgagcgataacggcgtcaacttcgacctgtacctaatcgaccgattcgacattcagaagtcgaagcgcaaggacgaggctggcgacacactatgggtcaagccgtatgccgtgcaggaagattgggacttgattaccgagcaggtcgtcgagaaggaatacgagctggaagacggcagtggcttcatgtcgatcaagatgaccggcatcgactccggcggtaagtcaggctcgacgacgcgcgcatacaactactggcgctcgatgcgcgacaacggcaacggcggtcgcgtgctgctcatcaagggcgagccgaagctcggtgcgccgcgtgccgaaatcgacttccccgactcggatcgcaaggatcgttcggccggtgcgcgcggtgaaatcccggtgctgttcctcaactcgaacgtgctgaaggacatgctgctcggcatggtcgactacgacgagaagacgacgctcggcggcaggcacttcacgaacaagtggacgccggaagttgtgtacgccgaactcactgtcgagttccgcgacgaccgtggtcgttggcagaatccggctaagcgacgcaacgaagcgtgggacttgggctactactgcctcggcctgtgcgtgatcttgaaggtcgaaggattcgattgggacgcgcctgagtcgtggttcgcggagtggagtaacaactctcttgtgcgccgtgtggatcaggaaaaacggtttgcgtcaagccccactacggattatggtttcgccaagttcgggaaatccttgggatgacaaatggcgaccctagagcagttgcaagcatggctggcggaagcgcaaaccgcctaccatagcgtcatgatcggcggcggcgtgaccgtcgtcgtcgaccagaacggggagcgggtcgagtacagccgggccaacgcaaccggcctcgccaaatacatagccactttgcaagcgcagatcaattccctattgggggtcgcagtaacaggcggcccccttcgtccgttcttctgagggtaaaacgacatggcaaaagcactcactgtcgtgcgctctcccgagggcgacgaagcgttcaacagcaccggcaaagagtcggcgttcggcggtgcgtacgaaggtgcgtcgcgactcaatcggcagaccgcgttgtggagcgcgccgtcgctgccggccgacatggagatttcgccggacaaggttcggctcgatgcgcgcactcgcgaactcattcgcaacgatggctacatccaaggtgctctcgacacgagttcggactccatcgtcggcggtcagtaccttctcaacgcgcgccccgattgggagacgctgggcctgagcgaagagtgggctgaagagttccagctcatcgccgagcgcaagttcatgctgtacgccgagtctccgatgaactggatcgacgcctcgcgcaagaacggtctgaccggcctcgtgcgcatggcgctcgcgcagtctttcatgtcgggcgaagcgctcgccgctgcggagtggctgtcgaaggcaggccgtccgtacaagaccgcgatcaacatgatcgaccccgaccgcctgagcaacccgaacgacaacagcgatacggcgtacatgcgtcgcggcgtcgaaatcgacaagttcggcgcggccgaggcgtaccacatccgcgacgcgcacccgatggagtcgtactacgaccgcttcggcgcgaagtggacgcgcgtgccggcgttcaagccgtggggccgtccgcagatcatccacatcgccgaagtgctgcgcccgggccagacgcgcggcgtatcgaagatggtcgcggtgctgaaagaaatgcgcatgacgaaggtctacaaggacatcgttctgcaaaacgccgtcgtcaatgcgaccttcgctgctgcaatcgaatcggagctgccgcgcgagctggtgttctcgcagctcggtgccggcgacatgggttggttgcagaagtacatgggcgcgctggctgagtatgtcggttcggccgacaatctcgccatcgacggcgtgcgcattccgcacctgtttccgggcacgaagctcaacctgcaaaacgccggccagcccggcggcgtcggcagcggcttcgaggactcgctgctgcgccacatctgcgctgcgctgggcctgtcgtacgagcagttctcgaaggactactcgaagacgaactactcgtctgctcgcgcgtcgatgatcgagacgtggaagtacatgcagacgcgcaagaagctcgtcaccgaccgcttcgcaacgctggtctacatgctgtggctggaagaggaaatcaaccgtccgaataccgacctgccgctgccgaagggcgcggcgcacttctacgaagggatcaaccgcgaggcgtactgccgctgcgactggatcggcgcttcgcgcggccagatcgacgagctgaaggaaacgcaggctgcggtgctgcgcatcgcgtcgggcctgtcgacctacgaggaagaactcggcaagctcggcaaggattaccgcgaagtgttcacgcagcgcgctcgcgaaatgaacctcatcgaaaagaagaaactcaacttcacgctcagcaccagcaagccgggcacgcagaaagaaaccgacagccgcgcatcgaacaacgaagacgcggacgccaccgacgataccgacacggagaacgacgatgaatgaactgctcgcgatgcgcatggcgctcatcgagggattcaacggccgcccggcgttgatcgaccctcgtgatgtcgagaaggtcgcaacgctgtgcatgacgatggcgcaggcatctttcccgccgaccgccgagcagcgcgcgcaggcggatgaaagcatcaccgccgctgtcgagaaggcgttcgacgtttccttcccgcgcgaccgtgccaagccgttccttttcagcaacggccttgccttcatcccgatgcgcggcacgctcgtacatcgcaacggcgacccgtggtacggcacgcgcggctacgacgacatccgccgcgagttcgacgccgcgatggccgacccggacgtggcgggcgtcgtgttcgacatccactccggcggcggcatggtctacggcaacttcgagctggccgagcacattcgcaagggtcgcgacacgaagccgtcgctgtctgtcgtcaacgcgggtgcgatgtcgggcgcgtattcgctcggcagttccgcgaagcgcatggtctcgacgccttcgggcgacagtggcagcattggcgtgctgaccatgcacgtcgacatgagcaaggcgctcgaaaagttcggcgtcgccatctccctcatccatgccggcgagcacaaggtcgacggcaatcccttcaacccgctgcccgacaacgtgcgtgccgacatgcaggcacgtctcgacggcatgtggcagaagttcatctccgtggttgctgttaatcgcgggatgtccgaacaagcgattcgcgacacgcaagcccgtgtgtatcaggcggacgatgcggtcaagatcggcttggtcgatgcggtgatgtctccgcaagacgccatcgctaccttccgggccgaagtcttcggctctaccaccaacgataggagtgcaaccatgagcgacacgaagaagaccgacgccaccgtcgagcagaagaaggacgacgcgcaggtcgagaacaagaccaccgacgccaccgtcgacgcgggcaagaagaaggacgagcaggtcgatgccggcgcggcgatgcaggcgcgttgcgccgccatcaccggctgcgaggaagccaagggccgcgaaggtctggcgaaccacatcgcgttcaagaccacgatgtcggtcgacgaagcgaagtcgatgctggccgcctcgccgaagcagtcggccgccaccggcaagtcgccgctcgattccgcgatggacaacagcggcggcggtgccgacatcgccaacaacggcggcgacgaagaagagcaggcgcgcggcaacgacgacggcggcctgctgggcgcgtacaccgctgccaccggcaacaaggccgtgctgaaggtcgtcaagtaaaccgaacaccgtcgccagcctagacggaaaaaaccggctaaaccgtcaatcacagaaggagtaacgaaatgaccaacttcggccccatcgctggctacgtggctcgtaccgacacgaacagcatccagctctacgccggggaagcggacatcgtgagcacgcagggcgcgctcgtcaccggcaccgcctacgtcggcggtcaggtgctcggccgcgtcaccgcttccggcctgttcgccaagcacgacccggccgcgaccgatggcagcgagaacgccatcgcgatcctcgcgtacgacgtggcgaccccgactgccgacaagaaggaagcgatctacgtcggcggcgtgttcaacatggaagcgctgaccttcaacgctgccaccaacaccgacgccctgaaggccgctgcgttcgatggcaccaacatcgtcgcgcagaagctctacggtgcgccgcccgccggctccggcccggtctaaccggcatcaccaacagcaagacgtttcgcaattcaactcagaaatagaaggagacaacgatggatttgttcagcactgcggaactgcgcaaggtgatcgtcgacagccggccccccgtgcagtatttcctcgaccgtctgtacaaggagcagatcaacttcacgaccgaagaaatcatgttcgacgagctgaagctcggccggcgcatggctccgttcgtggctccgaacgtgcagggtcgtgtcctgaagcgttccggcttctacaccaagtccttccgcccggcgtacgtcaagccgaaggacgcggtgactccgggccgcatgctgcgtcgcctcgcgggcgaagcactgaccggcgacatgacgcccggccagcgctggcgcgcagtggtcgccgcgtaccagctcgaccagcggaaccagattttccgccgctgggaatggctgggcgcgcaggctgcgctctacggtcaggtcacgatttcgggcgaggactacccgaccgtcaccatcgacttcggtcgcgccgccaaccacacggtcatcctgaccggcaccgcgctgtggaccgaccagaccaacagcgatcccgacgacgacctcgaagagtgggccgctcgtgtgcatgacgccgaaggtttcgtcgtcacccgcgtcacgatgggccgcctcgcgtggaaggcgttcaagaagcacccggtcatcaaggagctgctggaaacccggcgcggctcgaagtccgaagccgaaaccggcccgggcctcggcgagtcggtggagttcaagggccagatcggttcgttcaacatctacgtctacaacgacgtgtacgaggacgagaccggcacgatgcagccgatgatggacccgcgcgacgtgctgctcgaagccgaggctggcttcgacggcgtgcgggccttcggtgcgatcatggatgcggacgccgaccttcaggcgctcgacatcttcccgaagatgtggaagaacccggacccgtccgtgatctacctcatgtcgcagtcggctccgctcatgatcccgagccgtccgaactgcacgctgcgggcgcgcgtcgtcgcgtaagcgtcgtcgcacacggcaagcccggttcgccgggcttcgctgtggcaacacaactccccaaccgaaagaaggagcatcaagatggcgaagtacaagttcgtggcccgcgtggcgctgaagggcgatttcgacgccgaagacggtctcggcaccgcgttgcaggaagtgcaggcgggcaccaaggccggcaccgacgacaagaagctctacgactcgctgctggaacagggctacatcaagtccgcgaaggacgccgcgaaggaagaggacgaggctccggctgcgtcgtcgaacccgagcaccgcgccgaaggtcgagtcgaccgacgccggcaagtccagcggcggcaagcagggcgcgggcaagtaagcccggcgcgctgaagggagaacgaaatgggctggctcgaaaccaagcagaaggctcggcaaaccgtgcatagcacgtttggtctgccggcccaatttcgcccgaggtcgggcggtgctgtcgtcgacggcaccgctcggctgcactacaaggtccgcacgttcggcgacttggaccgcgaaggcttcgcgaccgtcaccgaggcagtggactacatcatcatcgacactcggattttcgtgggcgctgacgaaggcgaccgcgtgttcttcccgcaactcaaccgcgcgttcaagctcgatgtgcgcggcgaagcggaagacgacattttcatcaagtgggaagtgagcgaggtagcgccgtgacggtcgaggttggcttccgtggattggatgacgtgcgcaagcgcgtcgccggcataccggaaacggtagaccgggcatccgcgtttgcgatcaacgaagcggtcacgttcggtcaggccgagagcagccgccgcatccgcgagcaggttgcgttcaaggccagctacatcggcagctcggacgatccgaacgctcgcctgcgtgtgtcgaagaaggcgcgcgtcggcgacctcgaaggcgtcatcgccggccgcatgcgcccgacctcactcgcacagttcatgactggcgcgaagctcggcaaaggcggctacgctcgcgtcaaggtgtcggcgcacggtgcagcgcgtcgaatcccgaatgcgttcccgatgaagctgcgtcgcggtaccggcgtctacgacccggagaacgcgaacgtcggcctcgctgttcggttgcaggacgggaagctgccgggcggcatgaacaagaagcagatggtgcaggtcagcggcaatctctatctgctgtacggcccgtctgtcgatcaagtgtttcgcgatgttcgagtcgatgtgcaagcgccggtcggcgacgtgctcgaatcgagcttcctgcgcaatttcgggagattgaaccgtggctgatacgaagcgcctgctgctgctgaagagcctgtgcaactacctgctgaccgaaatcacgacggcgaacggctacaacttcgacctcgccgccgcgtatcgcggcaagaagaatttcggcaaggaagtgaagctgccggcaatcgtggtgttggagaacttcaacccggatcgtctgccggagaccatcggcggcgtcgtcggcaccaagcacaagtacgaccagatttacctcatcaacggatgggccgaaggcggcgatgtcgagcaggaagaggactcggctcatctactcatgggggacgtgaagcaagcgctcggcaagctgctggtgccgcgcaatcaaagcgggtttttcgatggtctcgcaaacacgctgtccatcgagcccggggttgttcgccctcccgacgagcaatccgagaaggcgtatttctggatgaggattcgtctggaagtcgtcgaaaaggtgggagacccgtactggattcgtgattaaccgttgtatcgacagaaggagaccgtaaatgggcagcgagaattacacccttggccgtggcgaactgcacttcgacaagttcgtcgccggcacgttcaacaagaccggcgagcgttacctcggtaacacgccggagttgaaccgcaccaccgagagcgaaaacctcgatcacttcaacagcgaccgtggtatccgcgtcaaggacaagagcatcgtgctcgaaaagaacgacagcggtacgttcatcgccgacgaaatcagcgacgagaacatcgccctgtggttcctcggcacgcagaacgtcgtggcgcagtcggcgtccgcgagcgtggtgcagaacatcccggccaaccgcgtcaagccgggcacctacatccagctcggcgagtcgaccgccaacccgaccggccatcgcaacgtgacgctgaccagcgtgaccagcgatccggttggcacgaccttcgacaacctgaccgactacacggtcgacgccgagctgggccgcctgcacatcgtgccgggcggggccatcgacgggaccgccccgctgatcgtgacctacgccacggcggcctcgacccgcacgcagatcgtggtcggcgagggcaccaccatcgagggcgcgctgcgcttcatctcgtacaacccgaccggcccgcgccgcgactactactggccctacgtgcagctccgggccgatggcgacttcgcgatgaagggcgacgaatggcagcagctttcgttcgcattcgacatcctgaagcgggacggctacgcttccgagtacatcgacggtcgtccgaccgtggcgtaaccggggtacgtcaaacgcggtcaaggccaacttagtcaagatcaagcgagccaagaccaacttcgacaggccgcctcggaacccccggggcggcctgtttcgcatcaccagccagaagaggaaagtccatgtcccttgccaacctgcaactccgcactgcaaccgttccgtatgtcggcgcgaacgatgagccgcacgacatcgtgctgcacggcctgagtgcgaacgccatcgccggtctcatcctgtcgcagctcaacaacatcgaagaaatcttcaacatcgtcgaggcggccggcgtcaagaagaccgaagacctcgcgaacgtcaacatcgccgaagtcggccagcggcttctcgtgcagctccccgacttcatcgcgcatgtcatcgcgtactccgcgcacgagcccgagcagtggagcaaggtcatgcacctgcctgcgcctgtgcaggtcgattgcctgaccaagctcgccaagctcacgttcaacgacgaggccggcttccgagaattcgtgggaaacgtggtcgcggcactgcgaagcgcaaaaggcgtagtgccgcagactctcaaccgaaatctcgccgccagcgtttcgctgagtggtggctcggaatccgcgcagccgtctctttcctgacggcggaaggtcactcgaacgctggcgaatatccgctcgggtatttgatcgtcgaatcggaaatcgcacgcgagcgggtgaacaacagaatcagaaccgagatgacgctgacgcagagtgcgattgcctcggcgctcagcaagaaagcagcatcggcattcaaagaaaacatcgaaggactataggcgatggccgctcagaacgaagttgaactgattgtacgtgcgaagaatctcagcacgcgaaccatcaaccagctcaacgacgagctgagcaagatcgcagataaccaagagcaagtcgccgatgcgaaccgactggcggagcggtcgttcgagagcctgaagtccgagcagcagcagttgctcgcgatcatgaagtctctcaatgaccgcgcttccaagctggacgcatactcgcgtcaagagcaacaggtgcgtagcctgcgcgacgagctgagtcgcgctcgcgacaacctcaacacgctcgcgcagcagttctacaacaccgagaagccgacgaaggaatttcagcagcagttgaagtcggctgcgagcgaagtcacccggctggaatcgtcgctgcgcaacaacgagcgccgactcgacaccaccggcaacaagctgcgcgacatgggcgtggatgtcacacgcttctcgcagtcgcagcaggaagtcaatcaggcgctcaacagctcggtggcgctgtacaagcgctcgaccgacaacgtggagcgctacgacgcggccatcaaggaagtgcgcacgacgcagcagcaggcccgtgaggccgagcgcgccgcagcgcaggaagccaaggactcggcggcgaagctggaacaggccgcccgcgagcgcgaagaccagatgcgccgcgaacagaaaatggccgagctgacggccaacgtctaccgcacgctggcccgggagaaggaaaaggcggctcgggccggagcggacttccgcgccaccggcacgcaggcgctcgccacggcccgcgcgaccgccggccctgccgtgggtagcgggtcgtctgccggcgcggctgctgcgggcgtacaggcgcttctcgacccggccaaggatgccgtcgcgacgctcgaccggctggaaaaggccgtcgaacagctcgacgaggaattcaaggcgctcacgccggacgctttgcaggccgccgatggcatggacaagctggccgaccaaagccgccggctgcgcgctgcgtcggatgcgctgaaggggcaggccgggctcgcggatgaattgaaccgccagaacaccgtgctgctcgccagccagcagcggttcgaggaagcgcggcaagaagtgatccagtacgcgcaggcggtcgagcgcgcggacaagccgaacgacgaactggcgcagtcgttgcagcgcgcgcagaacgagatgaagcaggcgcacggcgagctgacgcgccagaccgaagcgttcaatcgcgtgcagcagcgcgccgctgccgctggcatcacgctcaacaacctgaccggcatcgagcagcgtctcgctcaggccgccgggcgcgtgcgcaccgggcaggagcaagtcgcgaagacgatgacgcggttggagcagacgaccgcgaagaccaacacgcagttgaagctcttcaacgacgggcagcgcaccgcgctctcgctgtatcagcgcacccgtggtcaggtgctctcgctagtgtcggcgtacgtcggcgtgttcggcgcgatcaacctcgtcaacagcgcgatggacgcagcaatcgagaaagagcgcgtcatgtcgcgcctgctcatcgcgaacaagggaaaccagactgcggcggcggaagagtacgactacctgcgcaagaaggctgacgagctgggcgctgcgttcggccctctcgccgagtcgtactcgcgattcgctgtcgctgcacgcgacgcgggcatgagcaccgaggcgacgcgctacatcttcgaggcgttcaccgaggctgcgaccgcgatgcggttgagcggcgacgaaacggccggcgcgttccgtgcgttggaacaaatcttctcgaagggcttcatccaagcggaagagctgcgcggccagttgggcgaccgcatgaccggcgcgttcaatctgttcgcgaaggctatcggcgtcacgacgcaagaactgaacaacatgctcgaaaagggcggcgaagtgaaagcagagttcgtgctgctcgctgcgcagacggcccgtggtatctatggcccgcaagcgaaggctgcatcgaacagcctgctcggcgacctcaaccgcatgcagaacgcatggggcgacctgaagcgcgaaatcatcgacggcggtctcggtgatgcgctgcgccgcctgttcgtcgacttgacgaagtacctgaagagtgacgacggcaagaagttcgccgagaacttgacgaaggtgtttgtcgctgcggccgacgctggcggcgagctgctgaaggtgcttgctgagaacgatgaagtcatcaagctgctggcggacaccgttgcgttcctcatcaagaacttcaaggcgctgctcgcgatcatgctcgcgatccaaggcgcgcgcatcgcgctggtgttcacgcagctcgcaggcgaaattctgaaggcgcgtgcagcgacactcgcgttgaacactgcgctcggtgcaggcaccgccgcgtcggcgggccgtgccggtgctgcattgggcggcctcatctccgggccgattgccgcgatcctcgccatcgctgctgcgggcatcatcatcccgatctacttccagatgaagggcgagctggaatcgaacagggtcaaggtcgacgcgcagaagacgatcaacgacctcaaccggggcttcgaggtttcgcagcgcagcctcagcgacacgtcgaagaccaacgccgaacagctcgaacgtcaggtcacggccgcacagcggttgctcgacatctacgacaagcagaaggaatcgttgcaggcgcagattcgcgagaacactgctgtgcgccgcaaccaagtggcggtacgtgttgcgcagggcacgcgcgagcacgacatgaatttcccggccaagcagctcgccgccgttcgagaagtcgagaacgaaggcaaggcactggaagcgcagctcgccgcgctcgaacagcgtgccgcaccgctgcgccagcaggtcgccgccgccagtcgtcagatcggcgaagcgaaagcgcgcgaggcggctgcggagaacgatgcgctcgcagccgagtttaggcgcatccaagcagcggccgatgcggctgcggcgcgtgccggcaccgacgcaaaggcagcgaaggcggccgaggctgcacgcaagaaggcagaagccgaagagaagcgtctggccgcgctcgccgagcgccgcctgcgcctggaagaggacgtggcggaaaagctgcgcgacatcgacaacgacattgcggcgtcgcgcccggatacgctcgaagcgcgtctggccgtgatcgacaacaagatcgcggatcgcaaagccgaactggaacgcatgctgcgcgaagccgacaagctcggtcagtcggatgcagccaagggcgaaattcagcgcggcctcgacgcactgccggcgttgcagcaagcgcaggcgcaggcgaccacacaggagttctacgagcagcggattaatgacttgttgcagcagcgacaggcgtcgatggatgcgatcaacacgttgcaggaagccggcttgctgactagcagcgaagccgccgcgcgtatcgaggaagtcaacgctcgcctgctgccgcagctcgaagcgttgcgtgcgaaggcggccgagttcatggcgacgctgggcgatggtccgcaggcgcaggccgcgcgcgccagcctcgaaaacctcagcgcgcaaattcaggcgatgtcggtcgagctgtcggcacagaagcgtcaggtcatcgacgtgttcgtcaacggcttcggtcaggcgttcatggagaccgcgacgctcatctccgacacgctgaagggcgtgcaggatgccggtgacgcatggaaggcattcggcgacatcgtgctcaacaccatcgccgacatcctcatccagctcgcgcagatgattattcagcaggcgattttcaacgcgctgaaggcggcggccgagaacagcggcggcggctggggcgcgatcatctcgcaagtcgccgggtacctgcacgttggcggcgtcgtcggttccggcgctggccgtcgttcgtcggtgccgtcgtacgtgttcgatgcagcgccgcgctatcacaacggcggcatcgcgggcctcgccccggatgaagtgccgaccgtgctgaagcgcaacgaggaagtgctgaccgagaacgatccgcgccaccgcttcaacggcgggctggaaggcggggcgcaaccggcgatggacgtgtccatcatcaacaccatcgacagcgagagcgtggtcgctgccggcgcgaacacccgcgcaggacgccagtccatcttcaacgcaatcaaggctgaccgcagctcgtacaagaaacttctcgcataaggaatcaacatgggacacgcaattgcaactgtgactggcggtagcggcgacgaggcgcactacaaggtgctcgctgcgatcaagacgctcgccgaagcgaacgggtggacgacgctgcgctacgtcaacaccggcaccgttcgcgagttgatcctcaactccgctggcctgtcgggaaccgaggacatctacatcgggttccgtacctacagcagcgtgagcggcgactactacaacatgctcgtcggtacgttcaccggctacgtctccgcgaactcgttcgactcgcagcccggcgcgaagctgagcggcgtgccttgccacaacaacgcggtgacgtatttcatcactgcgaacgcgcagcgcatcgctggctgcttcaaggtcggaactccggtctacacccacttctacgcgggcaagatgttcccctactcgcgtccgggcgagttcccgtcgccgctggtgtgcgccggcatgttcgacggtgccgcgccgaagcgtttcagcgacaccgactatcgctttccgtaccacggtcgcgagtcgggctacacgggcggctcttcgtcgaacgtgcgcccgtcgtacctgtggctgcgcgatcaagccggcgcgtggcgtcggctctcgcacttcccgttctacaacggcccggccggcagcgattcgtcgagtgcctacaacgcgctcgaaaactggaattatttgaccggcggcgatcaatcgcgctcactcgttccggccggcacgaactatcagccgcagcctatcatcctgtacacgaccagcgcaccggccggcgtatggcaaggcgcggtgtacggcgagctggacggcgtgtacgcggtgtcgggcttcaacaacaacgtcgagaacgtgttgcaggtcggcggcacctacgtcgatccggcgggcctgagcgtcgtcgatcacgttgccgcgatcctcgctgccggcggtcgcgcgttcgtcgtgctgcaagacgtgaatcaaaccgactggcgcagctttatcgctttggagatgacctaatggcttactacaccggcaacttttcctcgttcgctacgctgaagaactcggtcgagaccgcgcttcaggcaaacggctgggggctcaacggcgacggcgtgctggaaaagaacggcatgtacctgcgcctcactgcgaccgctgcgcaactgctgttgcaggcaggcacgggcactgcgactggcgcgctgccgggcgcagctccgaacggcgtcaagatcatggacttcgagggctcgccgatgaatttcccggcgacttacgacctgcacgtcaacactggcccggacgaagtgttcctcgtcgtcaactacaacgccgacaagtaccagcagctctcgtggggcaagtcgaacatgcagcagatcggcggcaccggcatgtggttctcgggttcgttccacgagaacgctgcgtcgaatcagaaccatctcgtctacacgaacgccgatgcgagctacttcggcttcggttggtcgggcatgggctgcggcctgttcgccgagtattacacgcaggcgctcggctgctcctacgtccacacggggctcgactcgaccgcgtggcgtcgtgtgtacagcggcgacggcaacctcgtcggctcgggcgatcctgttgccggtctgctgcaagcgctgccgtcgatgttcaaccaaaacaccgtgctgctgccgctgctggtctcgcagcgtcgactctcgcagggccagaccatcgtcgtcgacatggcgaacgcgcgcctgtgccgcaacgacaaccacctgtccggcgaaatcgtcgagtacggcgcggacaagtggaaggtgtacccgttccaccgcaagaacgccgacgtgcgcaacggcgtctcgtggtcgacgggcgcaaaccactccggcactttcgcatacgccattcgctacacggggccgtaactcatggcaggcatcaccggacaattcggcagtgaggtcgagcgcggcatcgctaacgtgatgctgagcgaagacttggacgacaacaccgaagtcgtctcgcggttcgactcttacgaaatgcgcccgggccttcaaggcggctacgggcgctggcgcgtgcatgccgacaaccattgggcgatcaccggccagcgcaagtcgaccagcttcttcgacgactactacaaccgcatctacatcgtgccggccgcgctcgatgccggcaacctgctgtccacgcaggtgcgccacatcatcctgtggaacgcctacgtcacgccgcagacattggagaacgccgcgctcggcccgcagtccggcatctcgatgtcgttgccggtcggcgtcagcctgccgtacgagatggaaccgctgcgcgagctggacttcaccgtgcagatcgaactcagcggcccgccgactatcgacagctacgcaaacttcaccgttgaaggcgtcacctacaccgtgccgatcaccggccggcgcatcgtgctgttcccgttctcgccgaattggggctcgcctgttgacgagacggtcacgatgcgttcgtgggtgttggccgccgaggatggcagcgagcagaccggcagcgagtcaggcgaggttccgcgccgtacgctcgaatacaacatcaacctgcgcactgcgttgcaggcgcagcgctgcgagaatctgctgttcgcgtggcagtcgcgcttcttcggtgtgccgcattggggcgaggaagagcgcatcgcagccgacgtggcagcgggctcgctgacgattccgttcgacaccttcggcctgtctctcgaacccggctcgttggtggcgctctaccgcgacgacgagaagaacgagattcgcgaagtgcagtctgtcgctgtcgacggcgttacggtcacgaccgggttggagtacgactggccggaaggctcgcgcgtctacccgtgcttcgtcggcctcatgaacgatgcgatgagcggcacgcgcgaaacgtcgaaggtcggccgcatgcctatcgcgttcgactgcgagccgagcgtgaccccgggcaacgtagcgctcaacgcgccgccgctgacctaccggggcaaggagctgtttctcggccgtaccaactggcaatcggcgatgcccttcaccttcacgtcggatgtcaagcgcgtcgactcgaacaccggcaagttcgtcgcgttctcgtcggccgggttctcgaagatgtctcgccggcacaactggacgctgtacaaccgcgccgacattttcgagttccggcagttcctcggtcgccggcaaggcgtcgcgcgctcggtgttcatgccgagcggcacggtcgacttcaacatggccgcgccgatcctcgacaccgaagacatcctcgtggtcgagaacaacgagtacggcgcactggctggcgcacacccggcccgccgagacatcatcatcgagctggtcgacggcacgtacttctgccggcgcattgtcggcacgagcaacttcgacagcttcacccgactgcaactcgattcgtcgctgggcgtgtcgctcgacatcgacgacgttgcgcgtatcagcttcctcacgctgtaccgtttcgagtcgccgtcgaccaccatccgccacctgaccgactcgaaggctacggttgaagccatcatggtcgccaagaccaccgaggattgaaatgagcctgttgcaatacgagcaagacaaggaactcagctcccgtgtggagctgtacctgttcgagagcgacgacggccgctaccgctgggcctacaccaccgacgcgcgcgaaaaggtgctcggccccatcgtctacaagcccgagtcgatcaagcgcggcgagctgaagcagacggccggcgacgcgaacgtcgagaaccttcaggtcacgatgccgttcgataacccggtggcgctggcgcatgtgccgtacctgccggcgcggccgatcaagctgacgatctacgcctaccagcgcaacgatcctgctgcggaaatcgtgcaggcgttcaccggcttcatcaccagcttcaaccagaagggcgcggaagcgacgctcgaatgctcgcagatcatcgacaacctctcgcagacggtaccgtgggcggtgttcaagagcggctgcatttgggcgctgtatcaagtcggctgcggcgtcgacaagcagttgtggaagaacgacgcgctggtcacgaccgtcaacggctcggtgctgggctcgcctgagttctcggccaagccgaccggctggtacaccaacgggttcgcctacaacccgcagacgggcgagcagcgcttcatcgtcgcgcacgacgccgctgccggcacgatcacgctggtgtacccgttcctcgaaatcaacggaagccagatcatcgaggtctacgccggctgcgcgcgcacgaaggaagtgtgcgccgacaagttcaacaacaagctcaattatgtcgggttcgatcacttcccggcctacaacgtcttctcgcaggggatcacctaatggtttgggtagccatcgtagttgcgctcgtcatggcggtagttggcgagctgcttcggccgaagccgaaattcaacgacccgaagccttccgctgtcggcgatttttcgttcccgactgcggacgcatcgcgcgtcattccgatcttcttcggtacctgcaagatgcaaggcccgaacgtcgtgtggttcggcgacctgacgatcatcacgctgaagaagaaggtcaagaccggctggttctcgtcgaagcgcatcgtcaccggatacaactactacctcggcgtgcagctcgtgttcgcctacgggccgtgcgacgagttcatcgagctgcgtatcgacgacaaggttgcgccgatcaccagcaagaccttcactggcgacgtgtgctcgttcacgatcaacgcgccgacgattatcagcaacgacgacccgccgaacggcgtcaagggtccgtgcaagctgtatcgcggcactttcgagcagccgccgaatatgtacctcagcacacaatggaacgagccggagatgaccgcgttccgtccgttgctgcacatggtcatggagaagtgctacctcggcaacaccgacacgccgccgcccatctcgatcatcgcgcgccgctgcccgaaccagctcggcttgaccggcggccggcacaacgtcaacggcgactcgaatatcgcgtgcgcggtgtacgaggtcatgaccaacaatatgtggggcatgaaaatccctgaagacaagatcgacgtggactcgttcatcgcctgcggcaacacgctggccgacgagagcatcggcatctcgatgctggttcagaccgccatgctcggccgcgacctcgtggcggaaatgcttcggcacgctgacggcgtggtgtacgccgacccggttacgggtctgtacacgatgacgctggcgcgcgagattccgtccgacgagcaagacgagctgttgatcgtcgacgactcgaacatcctgcccgacaccttcgagttctcgcgttcgtcgtgggagatgacgaagaatacgatcatcgtgcagtacaccgaccgcactacgttcgagacgacgccggtccagtaccaagacctcgcgaacatcgacgtgcgcggcggcatgatcgactccgaggaattcagctatctcggcttcagcaattcgaccgccgcgatgaacaccgccgcgcgcgtgtcgaagatgaaagcgtcgccgctggtgtcggcgaagatgtcgctcaatcgcatcggctaccaactgcgcccgggctccgcgttctggctgcgcaagccgaaccgtggtctagcgaacgtgctcatgcgcgtcatcgaaatcaactacggcacgctggacgacccggccatcaagatcacggcgatggaagacatcttcgcggtcaacgccgtggcgtacgtgccgcccgacccgagcgactggacgccgccggtcagcgctgtcgtgccgttctcgcagcagcgtctcatcgaagcaccagccttcggtgccgaggatatgtcgcgccgctatgtcatcacgatgggcgtgccgtcgagcaacggcgtgatcgcgtacgacgtgtggacggataccagcggcggcacgaacttccagcagaccaactctatcgacgcgctcacgccttcgggcgtgttggtgtcgggtctgtcgcgtactggcccggaagtcgatgctgcgggcttcaccgtcacgtcggtcgtcggcgtcagcgacatcgaagccggcactgcgggctcgcgcgagtcgggcgaaaacctgctgctggtcggcaacgaactcatggcatggcagaacatcgtcaacaacggcaacggcacctacacgatcactggcgtgtatcgcggcgtgctcgacaccatgccgcaggatcacggctccggcgcgcgcgtctacttcatgtcggaaggcgcgggcacgaccaacgaggacggctatggcggcgacctgacgctcaacacgaagctgaccccgaagagcattgtcgacacggtgccgctggacaacgctgcggcgatgtcggtcacgaccaacgctcgtgcgctgcgtccgctgccgccgggccgcctgcgcatcaatggcgcggtcgtgggctccggcgcggcttactcgaacgacatgctgttctcgtgggcgcatcgcaatcgtctcgacgacagcatcgcatcgcaggccgacccgagccgcacgcccgaggaaggcacgacctacaacatccgggtctacaccagctcgaatgcgctgctggcgtctgcactggaagtgtcgagcgcggcgtcgaccggcaccatgcggttcgcggtgtcgggcgatatgcgcattgaaatcgaggcggttcgggacggctacgtgtcgtggacgaagctggtcggctacttcagctatactccggccgccggggctaccgccaacgaaatcatcgtcgacgaacccgagtacgttctggacgggggtggcgcgtaatggcacaggtagtcgttgcacaacgcatgtggcagcgccgcgacactgcggcgaattggtctgccaagaatccgatccttgcgggcggcgaaatcggcgtgcagctcggcgctacttcggacgagaccaagttcaagatcggcgacggtgtgaccccgtggaactcgctctcgttcttcgagggacgactcatcgaaatcggcacgggcggcggctacatccgctggcgctatgtcggcgacgagacgtggatcaatctggtttcgctcgaatcgctgcgcggccctgccggcgcgaacggtgcgcaagggccgcaagggttgagcgcatatcaggtcgcggtcgccaacggattcgccggcacgcaggccgaatggctcgcgtcgctgaagggcgagaagggcgaccaaggcgatcaagggccgcccggcattccgtcgcagcgtcgcattctgcgcatcgctaacaccgacaccggctccatcgtgtgcgactggaatgcctacgacgaaattcgcgtgacactgactgccgacacgctcgtcaacatgacgggcgcgctggacggtcaaggctgcgtgctgctgctgaagcagggcggcgtcggcggtcatggcgtttcgttcggcagcaacgtgcgcttcaacaacctcatcccgatctataacccgacaacgactgccggcaagtccgacaggcttggcttcgtctatgacgacgacgccggcttctacgacgtgcaggcaatcgtggatggaatctgacgatggcagacgactacatcccgccgttgtcgccgaacatcgtgtgggtcttcaagggcaatgactacacgcccccgttgaccccgaacatcgaatggatattcggtgcagatgatgaaggcggcggaaacgagcttcgcaaatccacctacatgctaatcctgacaatgtgaggtattgaaatgactgttcgcatctactcttcttccgacgctggcgctccggttcttcgcggcaacacgccgggcgacctcatcaacctgctcgaaaagtgcctcgtcaccggctacggctcgaaggccggtgcaggctggacgaagccgtacaccggcacgaacgtcgctgcgttccagcaaggcgcaggatcgaacggcatgttccttcgcatcgacgacaccagcaccgcgaccagctatcgctcggccaaggtgaagggctacgaagcgatgaccgatgtcaacaccggcaccccgaccccgttcccgactccggcgcaaaaagcggacggcgcgtattggttcacgcactacagcagcggctccgtcgcgaacccgcgcccgtggcgactcatcgcggacgagatgttcttctacttcatgctgtcgacttacccggaaaacaacgacagcggttactactacaacgagtgctatgcgttcggcgacatcatcccgtacaagccgggcgacacgacgcacaccgtactgctcggctcgtggcaggaaacgagtccgaacacttcggaaggctacccgtggtacggcgtcgacatcgcgagctacatgggctcgaatcgctacgtgcttttggctgcacgttcgttcactaacctcggcggcccgatctacctcggatggcatagcgaccacacgaaggggagttcgagctggggttctggcaggctctcgtacccgcatggcccggacggcggcctgtacctcgctccggtgtgggtgcatgaagcgcacgtctcgccgtacaacgtgcgcgggatcatgccgggcctgtgggtgccttgccacaactcgggcacgttcagtcaattccagacgttcaacggccaaggcgagttggcgggcaagcagttcatggcgcgcaggcactacgaccagaccgtgtgcttcgagatttccgacacttgggataggtaacgcgcgatggcgctcatcttcaacctgccgatgacggggccgaatggctccacgacaatcaccgacaccacggggaacttctcgtggtcggtgacaggcaatgcgcagattcaatcgaacgctctcgtccttgacgggagcggagattatgtgagcacgactgctgacgaccgcatgcggctcggagcgatcaacaatttccgcctcgctttcgacatgaagatggcgtcggcggacagcagcggctacaagatcgttttcgatcaactcaatactggcgtcagcgcatggacatggcaggtctacatctacaacggcgtgccgtatttcaacgtctaccatccgagcttcggcaacccgacagtcgtacaggggagcgcaagcatagcggacggcaactggcacacggtcgagttcatccgagctaacgggtcgatgcagttgtgggtcgacggcgttgtggtgtcgtcggctgcggataaccgcgactacatcatccaatcggcgttcggcatcggttctcgcatcggctacaacgcatcgtctgcttatgactacaaaggcgaactgcgcaatctcagtttggaaatcaccgagccggtagtgctgaccggacgcatcgctgcgtggatcaagcgcaacatcatcggctgggatcgagcgcgtactcgcagttatattcggcgcagcgtcttctacagcttcccgccgctcgaaacgaagatgcgctcgtacgtccgcatcacgcgcggcgtgccgccgtggtgggggccgagcggatcgaccacgcagctcccgacctacaagctacgcggccgggtgatgcagcgcgatcctgacggcgtgttgcccgacgccccggtacagtacgcgcgcgtcgtgctgttcttccggcgcttgcatacgctcgtagacatccagctctccgatgtcgacgggtacgtgcaattcgataacctcatgccgggcggtcaggcgtactacgcgattgcattcgacccggaaggcgcaccgttgcagaacgcggtgatttgggatcgactgtcacccgagcccggcccgtaaggagaagtgccgtgagccagaacaacacccacgagcggaacaggaaccgacgagtgacggacaaggcagggggacttttggacgccgcgcagcaggccatccggcttgaacgcatcgaaggcgatatgcgtctgctcacgcagcgcgtcagctccggcatggagaacgtcagcgccacgctcgcggctgtgcaggtcgaagtgcgcggttgctcgacgaacgtgtcagagctgcgcgggctgcaaggtgcgcacgactcgaacaaggtagcaatcgacaaggtggagaaatcagtgaccgacctcggtgcgcgcttggagtcgtggttcgatgagttcgaggcgaagcaagaacagcggtggcgcgactattcgagcaatcgcgatcaatggcggcgcgagcacgaggccgagaacgagaacgtcaagaaggacttggaaaaggaaatccgcagcgttcgcgaaaccgtcattcgcttcatcgggttcggttccgccatcggtgcgcttgcgggcgtgatcgtcggcggcttcctgtggaatatcaactaccgcttcaacgaccaaaaagaggacgtgacccgagtcgaacaaacgtcatcgcgcaaccgacaactcatcgaccagatgggtgtcgatcacggcaaagagctggccgacatcaagctctacctcgcgcgcggcgggcgaatccccgctgagccctatgtccctcaatcgcaaaggaaccacaatggaaacgaacaagactccggccaacccggaaagtgaaatgcccttccgccgccgcgcgtgggagttctggcggcgcaatcaaatcctgctgctgcaactgccgctcatgctggtcttcctcatcggcagctacgtcgtgctgaagtcggtcgactcgcgaatcggcgtcgagggtttcggcgacatcttcggctacgcgctcaacggcgtgcgcatcacgctcatcatcttcaccgcatggtggatcaagaagtggtgctggttcgacctgcacgacaagaccgagctggcgatgttcgaggcgatgaaggccggcgactggatggcgttctggatcgtggtgcgcgaccgggccgagtggctggcggcgctggcgttcgcgaccttctggtacacccgatgagcgcccgggtcgtagtcctcgctgcggccctcctgctgggcgcatgcgcccggccggcagcggtacccccggtcgaccagaccacgctcccgccggccgtggagagcctgcctgcggccacgccggagccggtcgtcgagcaggtcgtcgcggctcagcccctaccccgggccgagcaggctgtttcggagaccgtcacggagccgcttctggccgcgcaggcggcgctcgaagaccttaccccgctactacccccgccgccggcccgggacgcggcttgccggcgcgctgcggcggccctgacgctacgctgggaagtgaccagcccggccttctaccggaagcggctcgaactgccgatctggccgggcggggcgtccggggtgacgtgggggatcgggtacgacgggggccaccagacccgcaccgtgatcgtcgacgactggcacgaccacgggcaggtcgaccggctaggccagaccgccggcatcatcggccagcaggcccgggcggcgctgccgcgcttccgcgacatcccgaccggcttcgaccatgctagtcgcgtgttcgaggaacgcagcctcgtcgaatacgaacggcgaaccgagcgcgcgttccgcaacggcttcactgagctgcggccgaacgcatgcggtgcgcttatctcgctggtgtacaaccgtggcgcggcgatgaccggcgactcgcgacgggagatgcgcaacatccgcgacaactgcgtgccgaagcaggactacgcctgcatcgctgcggagattcgctcgatgaagcgcctgtggcgtggcacggtcaacgagaacggattgtctgcgcgccgcgaggccgaagcgatcctcactgaaaccccgtagggagaagagcatgtggacgaaagcaatcgcgtggctgttcggaacggcaatgggtcgcggtgtgctgcttggcggcagcatcgcgataggcatggcgctcggctggtatgcgttctcgacgcactactacaacgagggcgtcgcgtcgtgccaagctggccgcgccaccgatacgaacgcggccaacgtcgcgcaaggtgaaaagaacatcgccgacaaccagaccagctccgacatcggcaaggccgccgacgccgaagcagcgaaggtcgcagccgatgccgaagaagcgaagaacgactcgaaggagaccatccatgacgtgtacaagaagccccctgtcactgcgcctgttgctgttggttcttgcgtgcatcctctcgatgagcgggtgcaagaccggatcggcaaagcgcgagctgccgcagttgaagcaagaagccccgctcgttaactgcaagcagcctgcgtcgccggcagtgccgcgcgagccgaaggccgacgagtggatcgagtggaacccaccgcgtccgggcaagaccgaaggcgaggcccggctgagcgaacgtgcggtgaactggatcatcgacgtgctgggcgtggtgcgagtgagcgagggctaccgccgggtcgagcacggatgcctcgacgagctggaagcgaaagggctcatccggcagtagttgacaggcccgaggcgctgcattacggttggtctcgctggtggcacttcgcgttgcatcggcactcggcagagggacagcggcgcggagaatcggcgctccgcaccgcagggaacgaggaaccccggactaacactccggggtttcttttttgcgtcaagaccaagtgcgtcgtgaccaagttcgtcaagaccggaaaagagaaaagccccggtgctgaggccggggcttttcgggttgcgcgactcacgtcgggcggtgggtatcgaggcgggggttctgctgattccggtgtccgctctatgagcgctgcgccggctggaagggcatgtgtcgcgtcgatggatcgaacctaatgcggcacgccgcgcgtgtcaacaccttcgtcagtccttccacgtctcgacgagcttcagcatcttcttgcgcgccttctcgacgccggccgcccacttgtcccatgcgcgcgggtcgacgtgcgtcaggatttcgttgcgcgccatctcgctcagcacggtcggcggcagcgcgtccagctcccagctcttgtcgccgaagcgctggcggtatttcacgaagcgcgcgtcggtcgtcttggccgggttcggcggcggcttcagctcttcgatctggtcgaggttgagcgccatgcgcttcagcgtgaactcgccgttccaaccgaacagctcgaagcgctcttcgaggtcgcgcgtcatgtcgatgccgctcggatcgtggtctccgaagtgcaggatcacgacatccttgccgtcgctctgttcgatttcccgcttggcgaagtcgcgcacgacggaagcactcgggtagccgcgcgctgcgagcagcggcacatcgaactcgtggcatacacgctggaacacgccgaccagcgcttctttctcgacgacgaggaaaatgcgtgcgtcctgcgtcgcccacgggtcggtgtggtactgccgcgccgacgccgtgagaatgtcctgcggcttgttccaacggctgcgctgctcgaacgagcgcgtgcggtcctcgatggcgtcccaatcaatcaggccggcgatgcgcgcgtcgttgacgatgctcgtcgtctgcttgtaggacttctcgttgttcggaatgatgtcgcgcgcgacaagctggtagtagagctggcgcacggtcagcgtgtacccggcgtcgagatattcttcgatgatcgcgttgatcctgtcgatctgttgcagggtcttggtcttgaaggtgatttctttgtagcgttcgaggctcatggcagagggttcctgttatcggcgggtcttggtttgttcgagcagtcggtcaatcttgcgggtcagcctgtcgaactcttcgtcggttggcggcggcccgacatcggagcagtcgtagtgcgaatggtgcagtccgttgcgcgcctcgccgtcgagaatcggcttgcagcacaccgagcacgtatccgtgtcctcggcatgctcgatccgctcgcggcgctcatcgcggctgagccgccaaaattcaccggcagttagcggtttcatgcgcgcgggcaccgttcgggctgaccgtgtgctgcggcgtagcaaactccggcttcgtcgcagccaacacccatgtcgcagtgcgtgcttttagccttgccttccttctgtgcgcgaagttcttcgcggatttccatgagcagcaggccgagatggttctcgcccttgccgtcgcacacgccccaaaacttgtcgccccaccagttgccttcgaccagcttcgccttgccggttttcagcagcttcgacttcagcggatcggtgccgaacttctggcgaagcaggttgcgcatcacgtcgatcttgaccgcttcccaatcctcgcgcagcgtgacgtgcttgcctcggcgcttcgccccggcggcgtcaccttcgttgcggatgcgccgccgctcgtcctcgtcgaacgtcttggcggcttggaaggcgtgctcgaccgtgcggtacgagtggccctcgaaagcgatgcagcacgaccagaaattcgagaggaagcgatacggcccggaaaatgcagcgatggttttcatggtcatcccctagtggtacatcttcgccttgccgaacaactcgcgttgcttcgtcatgtcggtgcgggcgatctgctcttggatgggaacctgcacgttgcgattcatcatctggtgcaggtagcgcggctcgaccgcgtgcccggtcgcgaacttcgcaatcgccatgagaatttgcggcgagtgcagctcgaagaacgtgccggtcatcgcccaatggtgcgggcggatgtgcgcagcgatgtcgagcagttggcgctcgaccttgcgcacgttgatcggcggcgcgatgccttgcctctgcatcgagtgttcgacttcgctcgccgcacgatgcacgacgaggtactgcgcgcccgggaagcggagcagcagttggtcgaagaagaacagcgccgcgacatccgatacgaacacgcggcccggcggcagcttgtcgatcttctggcccagctcggcgatgctcgcgcattgctgcaacggattgtgcagcgacgcagcgcacagcggccgaaggaactcggccatccatgcgctgcggctgcgcggaagcgacagcatgaaggtcaagtgctcgtagctcatctcaatcctccaacgccacgagcagcaacgagcacttcagccccatgcactcgccgcagatgcacgccgtcttctcgtccgacagtgagcgcgcgaggtcgttgtccggccccatgacctgcgccagtgcagcgtgtccgccgagctgcaattcgagcccgtgctgctgcatgatcgcgttgtggtctaggccgaattgctcgaccttgacgcggtagaaaacgatgccgccagcggcgacaccacgttcgcacaggacgcacttcgagatgtccttgcgcttcagcccgggcctgtcagccatgtccgctctccttctgttcgcgcttcgcctgtgcggtctcgacgtagttgtcgagcaccttgacgaacgcatcgtggagcagcgacccggccggcacgtagatcaccacgccgccggtcaagtcgctgcggttgtatgtcgtcggcttggcgtcgagcagttgcccttggccttccggtgtcgcctgcatgcggtccggcgggcgcacgtcgaactcgcgcaccatgccgtccgccgggccgccgatgaagaacgccctcatcgcacttcaccgtcgccttgcagcgtgccgcgttccagccggccgttgagcttttcgcgattgccgaagagcaactgctcgtagccatcgtcgaagcccaccagaggcccggtacgctcggcgaactcgaccgacacgttgaccagcgcttgcaagtggaagcgcatctcgtcgagcttggcggcgcgcttgtcggcgttccacgttgcgccgtcgcgcatcatcttcttgacgacgcccagcacgtagcccgagtgcatgcacagcgctgattgcaggtcgtagccgctgatacgaacttcgcggtactcggcgtcggcgagacgctggaaagcgacctgcaccatcgcgtcgaatcgcggcagctccgggctctcggcgcacagccgcgcgatgtaccactgcacgtcgcccagctcgctccatccttttgcgtagcgttcggcacgcaggtcttcgcggacggcttcttggtcgaacagctcggccagctcgccgacttcgttcgcgatgccgatgctggtgtacagcatgccggcagtgacgttgccggcgagctgcgcgatgtcggtcgggtacttggccgtggtgatggtgaacgccgcatacgcttcggcgaagatgcgcgtgggctcgacgcgcgcggcacgcgactcgcgtgcggtatcgagggacaggatgctcatgcgcggcccccggcggcgagcgcgtcagcgaagtcgttgctgtagctggcctcgaacttcgtcgccatgtcgtgcaggacgagcgtggggccgccgtgcgctgccgggatcatggcgaagtcgacgccgcgcaccagcgggttgcgctcgccgtcctgaccgatggcatgcacgaccaacgcttcggggttctcgcgcgcggcgcggcgctcggccttcaggatgcgccgcatggtcttgccgccgaacgccttgcgcagcttttcctcgggcgagccgtggtcgcggatggcgagcacgccggcaatgccgcccttcgacgtgcgcacctgacgcttgttcttgcgctgctcgttttcgaggtcgcgctgctggacgaggaaggcgtagttctcgtcgacggcgagcatgcgcttacgccagtcgctcagggtcttgtccttctcggcattgtaggaacggaaaatgcgcttcaacaggttcatcgtgtggctccttcaggtgtgaaaaaagcggcccggccgatgtcgacagggccgcttcgatgtactacgtcaacgccaccggactcagcggccggcgacgaacttggtctgcttctgcacccggccgcgcttggtctcgcggaacagcacgatggtcgtgttgtcgtcggccatgatgctcgcgtcgtcgagcgcgttgctctcggtcgcgaacgggccgttcatggtgctggccttctgcgagccgtcttcctgcgcggtcagcagcaggtacgcgaactgcttcgcgcccttcttgccgcgacgcacgccgaccttgcgggcagcggtcttcttgccggccgggcgaccgcgcttcttggcgggcgcggcggcctcggtcttcttcgcagcgcgcttggccggagccttcttcgcggcggccttgcgtgcggtcttggcgggagccttcttggtggccttcttggcagcggcgcgcttcttcgcgaccttgccttcggtggcttcggcgttctcggacatctggtttctcctagcgttgttgtcgacaactcgcggaatgcgagcggggttcccttgcgggattcggttcagtccacgcagtacgcggggacttcggtgcggaacgtccggcactcggacggctgcgtgatgtacaggccggcgatggcggccagcagcaacacgccgtaggcgatcttctcgcggcggctcatcactcgcagcccacggtggcgttcgggcgggtcggatgcgcggcggtgtactggctgaagtcgcgccagccttccgagccgccgcacgcgaagccccagcggcgcacgatggagccggtcatgaagagcgtccagcacggctcgtcgttgttgccgaacagttcgagcaggtgcatgtggtcggcgctcaggcggcggaagtcgcccgtgtggaagtgctgcgtgtagtcgaacttgtgctggcccgggaacttgcccttgttgcgcaacacgctgccttcgacgaacgtgcggccgtcgttcggagtgaacagtcggtgcatgtacgagacgtgcgcgtccatgccttcagggctctcgtcgatggcgtgctcgtagcaccactcgctcgtgtgctcgatgtagcgaccgtcgaggatgagcgacgcactagcccacgggtgatcgtgcagtgcgcggtcgtcgtcgccatgcacgaacttgtgcaggtacaggttgaaccagcggttgcgcgggatgatgtgccagcgcgtcaggtacgggcggcgcgggccgccgtcgatgccgtcgagcatgatgaccttggacggcgagacgatgcgcgcgtacagcttgaacgcgccgacgaagagcgaccacaggccgatcatcgagagcacgttgtagaagcggcgggagacctcgggggcgttcatggcggggaacatcctcggtatggtggggtaattcatgcgtcgagcgtcgcgtcggcggtggccgggccatccgcgttggtcgtgtcgacctgcgggcgaacgagcgggagcggctgcgagccatcgagattcttgaactcgatgtagtagcgcgtgttgagcgtcttcagtccggtgtcgacacggttctggaagacggtcagcagttcggccttcgtcagctctccggcgtgcatgccgccttcggagacgacgcggaagttctcgatgtcgccgctcgtcagtacggcgaggttgtggcggtcgaggatgagcttgtccagcaagtcgcgaatgttcggcagttcggcgaagtcgattttcattgggttctctcggcgtgagatgaagagcggcgtatcgtgccgcaagccgccgggttgacccttcaagcgctggggagtgcgccatccagttgaccgggggtatcgcctcagcgaccccgtgcagttcggtgatttaccccgtagggggacgaagtaaattcgttactgcggggccactctagcgccagcttttcggcttgtcaacacccttccttgtgtccggcggccggctcagccgggccattttccgctcgccccggaagagcctgtcgcgcagcatcttctcgctgacgtgcgggcagtgccgcttgatctgctcgaaggtcatctcgtccccgtcgatggtgtacagccgcacgcgcgcaacctctttcactgcgtagtcctcgtcgtcgaatttctgcctgctcatagcgcccgcccgtgagtctggatgtagatgtcgtgcagcatctcgtgcgcgattgctttgcgaaacgcttcctgctgcacgagtgcatgtgcgaagtcgcgcgcgctcggttccttcatgccgagatgcgcggtcatgcgcagcgcctcgtcaatgatggcctgcggttcgccctcggcgtagccctcgtcggcgagcagcgcatggatggcttcgcggtacttcgcgtgtcgcgcgcgctgccgcagcatcgcgatgccagcgatgacgttggggccgatcaccagcagcaaccaatcgaaccagctcatacagacctcgcgtgtggacgctcttcgccttccttcggcgcgggaacgtggtggagtgtttcgagtcccttcttgatcttcgccgccatcgccttgccgaactccgacgcatcgccgtacatgaggtcgaggtcgggatcagcgcattcggcggcgacgttgcgcagcgtgtcgaccagcatcgggagttggtgctgcgcgctgtagttctggtggatcatcggccacgcgccctgcgccttccaccactgcttgcgctcgtgctcggtcagcgcgacgtactggtcgatcatcgccatcgcgaggaacggcgaccagaagcacgtatcgagcggcgtgatcggctcgcccagctcatcgagcgcgaagtacaccgcgaagacaggcgtggtgccgatgaggtagaccggctcatcgagcgggtctttgtaggtggcgatggtgcagccccggtacgcggccatgtgtgcgtagcggcgcttgctggcgtcagggagtggcatgcggaaactctcgttgaagtacgggtcaagggacgctgaggcgtacaagcacgcctgcttgggctcaggctgtgcagctctcatggcgacgaagctgcgctcgctcatgcgccgccggcatcgcgcacgagcacgacttcgccgccctcgccgtcaggcaggcatgcagccagtacgtcggccgcgccctgcgtgtcgccgagcacgagcagttggatcgcggcgcggatcgcggtctcggtctcgatggccttgcgctcagcggcgagcacgtagccagcaccgtcgcacagctcttcgagcagatgccgcaaccactgagcagtcgtgaggtctttgcggtcgagcgtcacgccgtacttcttcaggccggcgtcggcgcgctgacggatgatcgagatgaggtcgttcgtggtctgcatgtcgctcatgtcacagctccgaagttttcttgccggggttgcggcggtgccattccagtttcgcgttcgcttctatctgctggcgcgacaggcgggggctcttggctgcgagttcttcgcacagcgcatgaaaacccgggcggcggtcttcctgcatctgctggaactcggacagggtgttcttcttcagcatggctagaactccttgtggaaatctttctcggcccggatgagagccgaaaccttggggccgaactttttcggcgtgtcgagcaggatgtcggctgcgcccatcgcgatctgcggcgacacgaaatagccttggatcggatgcagcacttcgccgaagtcgtcgacgatgtagtacgcgagatggatgccgacgccatcgagcacgatgagcgggccgccgtcgctgcgcacgtcttcgctgtgcagctcggcgatgaacacgtcgcggtacggttggatgcgcttgaacttcatgcggctttgtccttcaggtggtcgagctgccagccggcttcgattgccgcgaacagccgcagctcgctcgcgtcttcggtgtcgagccgcaggaactcgatgaagctgtcgatcatctgcggcgtcatcgggcgcttgtcgtagaacctgcggtacgcgctttgcggaatcatgtcccacaccgggcacaggtcgacgatgcgcttgccttcctcgcgaagatggcgacgcatgatgtcgcgcaccgtcttcgggttcttcttgaccgtgatcttgcggccggtcgacggacggaaactcatagcccgatgtcctcgccagcctcgcgcttcagcaaccacatcggcttgcgcgaaagcatcggcagcgggccgatccatccgtcgacgagaccgtggtggcgattccagccgtagttgtcccaccagcgtccgcgcttctggcccagctcaggaacccacacagcaatctccatctccttgtgcgccggcagcgcggtcgggaacgggcggtgccagatggcgtagaagccgaattccggcgggtcttcgagcacttcgatgtcgttgtactgcatcggcccggcccagccgagcacgagcccgttgaagggcacgaacggcttttgcaggctcggtcgacgctcccaccacatgccgttcgcccagcgcatcaccgagtacatgcgcgggtcatgcacgatggtcgggttgcgcgtcagctcgacggcgtacagcccttcgactgtcgggtcgtcgagcacttcgagttgttcaatcttcatcgtgcggagcctcaacgtgcgcgcgtagtggccgcaggcgcggcagcgggccgatccagccgtggacttctcccctgaagtattggtcgctgttgagatagcaccagcggccgttgaaccacatgaggaagatgtcgacgacgagcccgcgaccgtgcgggtcgtctacgcggcaagcgtagacgcccgtgtcctgcggcagtccgatttcttcgtactgcaccttcacggcatgcacttctcggcgtaggtgcggcagtcgcgcatgaagtcgatgtagacctcgggcggcaggtcacgcatcgtcgtcacgccgaacgcctgcatgtgggccttcagcctgtcggtgccgtggatgatgcggaacagccgcgcgtactcgtacaccatctcgcgcatgcgatcctgctcggtacgaatgcgctccggtccccacgagccgccgcgttccttcttcagcgcgtcgacttcgcgcgtacgcgattcgagcgtggcggccaacttcttgttctgctcgcgcaggtcgtcgttctccttgcggccgtgcatgcgcaccagcgtgcggatagcacgaatcgcgaggtcggtctggttgagcgtgggtccgctggtcggctgcttgtcccagcccggcagacggcgatgcagttcatcgaacacgcgcacgaggtcgaacaccgctgcatcgtcgatggcctcgaacgcctcgtgcagcttgcgcccggcctcggccgccgctgcgctcgcttcactgacctgacgcatagcgtcgccagcgtcgacacgcagttcgacctcgacggtcttgcgtgcgttgccttcgtcgtctgccggccgccatgttgcgagccacgtcgcatggtcgcggtaggtgaacttggtgcggtggccgtcgccgtcgcgctccatcgtcacgtagtagtccgtgctgtcctgcttgcggcgcgcgtcgatcacggtgtaggtgccgcccgagatgacggagaagtagcgctcgccagcggccggcggttgctcgctgccgtcgaacggcacgttctcgatgaagtcgcggaacagcgattcgatgaggccgtagcccatgccgagttcgggcggcatgccgacgcgacgctcgcgcgcaggcttgaacgacacgtcatgcagctcggcggccatctgcgcatacggactgcccggcacagcgccggcagtcgtcggtgcgaacaggtcgttccacgcgctcgccgtggtgaacatccattcgtactcgccgccgcgcccgttgtcgacgcgcagcatgcgcacatgcgagtggccctcgcactcgtgcgtgctcacgaccatgaagaagcgcgccgggcggttgcgatcctgccagtaggtgccgaccttcggcgcgaactcgtagtccgggtggccgaccgtcactgcacgcgcttccttgcggtcgctcgcagcacccttggtcgtctgcgtgctgcccttcgagaagtcgcgacgcatgatgcgctcgatgaggctcggcgtgcccttcatcgcctcggcgatggcgtccgggctgaagtcgatggtgttgatgatgtggatttcgggcgcgctcgggttctcggcgaacgacggcgcaggcaccttgccgttgtgcgcattgaagaagaactcgtgctggccgacgaacgtgttgcgaatccagcggtgcatgcgctgcgcttccgcgcgctggatgtcgttctggccgacgatgccgccggcagcgtgcatgtcgcgcacgatgccgttgtcgtcgatgcacgcggcgaccgacacgatcatcggggtggtagcgtcgttggtgaactgcttttcggtatgacgagacattttcggcgtttcctcggttgggttaggtggtgctgacgtgaccggcggcctcgcggtcgagttgtaggtctgcgatgtcacgcagcgacgagggccagtcgtcgagcggcacgagtccttcctcgtgcatggtgatctggtcgggcgtcaggccgcacaggtaatacgccttcgcgagcgacatgccggcgatgagtcgatagcgcatagcggcgcggccatgcttgaaggattcgacttgtgcccgtgtcacttcgcccgtgcctcggcacagccggcacttcgtccccggcaagttgtcgtcgtgtcctgcgtcggggccgaacatctcgttgaactcgatcatgtcgtgccgcccttcgcagcgcgggcagacagtcttgtcacggagccaacgccacgccgcgcgcaccttcatccgcagggcggtacttactgcgcgaccgagcagggcggtagcggtgcgcagacgagacaaagggggtaccggagcattccgagaagccgcaagcctgcggcccaacattttcgcttcttcgatttcgcggcgtgtgtggcgcatggtgttggtcactccatccgggtgacagtgaggaaggcgaacatggcgtcgttgctggcgctcatgtaggtgccgcgttccatcttgaagcgcttgtgcttgtggtcgcccgctgcgcgcaccttcgcgatgccgccgctcaggatcgagttctgctgcttgaagtatttctgcgcctcgttgttgatcgcggcgatgttcccgttgtcgagcgggatgcgctggcagcgcgcgtgcgactcgccgatgtcgagcttgctgagctggtcgttgagcgagcccggcaggaagaccaaccggggcttctcgacgatgcgcacgcgcgggttggcgatgtcgctcttcttgatcttcgagcccgacttcttgcggctcttcttcgcaggcgcggcgctgctgttcgtggtggcggatgccattaggtgatgcctcctgttccggggaagtaagcggacaagaaacatactactgcgcgcacccggggtcgtgtcaacccgggcgttctcggtcgtgaccaactcgcgcgccgggccagcgccgcacaacgatccggctgggttgccgaagcgggcgcaatttcggaaccggctaggtcggcgaagcgagagcgcaaacggaaccggctggctttgcgaagcgggccgaattttggaacgggctgggtatccgaagcggggacgtttttggaattgctctcttacatgcacgcgcacacagatatgcacgcgggcacgtatgcgcgctcgcctgcgcacgcgctcgcgttctaagtcacgcgggcgcgcggcgcgtgcgggcgcgtcaaggttccgcgcgctgcgcgttgcgcgcggttccttcatccgggcgcgcttgccgccttccgcgcttcctgaatgcaaagtaaacggactactgcgcgcagtaaaaaacatcttgcgcagcgcgcgaaaccgtgtagcctacgcataccggcaacgtcgccggcatcgcaaagggtcgcaaacatggcacgcatgaaccgttccgaattttccgcccatgccgcgcttgccgcgtcgcgtggcgcgtccgctgcgcgcaaggtcgaaaccgcgcgcaaggtccagacgttgcgcgatttgctcgcgcgtcttcccttccttttcgccgtcgccgttgccgcctttgtcgcggtcgcggccgtcgccgtttccatcgtctaagggaatcacacaatgcgccgctatcttttcgtttcatccgctacgcttcccgtcgtcgcctacgcggaaagcaaagacgcgatgcgcgcatacgtgcgcgacctgctagggattccgtacggtttcccgctgccgcgtcatgccgtttgcagcatcgcttaacaattcactagacaaaggagattcaccatgcaacgcattagcctttcgcaagccttcgcacagtggcaagagctggccgcagacattccgcaagacgacgcgcccatgctggcggaatcgtggaacgattacacggattcgctttgcgaagatggcgcattgtgcgacctgcaataccactacgcgcccgcatacgatgaagagatgcccggcgacggttcgcgcttcgatccgctgagcgatgaccgcgaattcatcctagacgcaatgggcgtcaccatgcgcgcaacgcgcaaggatggaccgcgcgaaggatgggacgcgagcgcgtcacactggcgcgtcacgctgcgccgcgaccgcgcgagcatgacaacggattacagcatgggcgcggcgcatacgggctcgcctgagctggcggacgtgctgaattgcctaatgcgtgacgcggaatgcggcgcgcagtctttcgaggatttttgcgcggaccttggatacgacacggattcgcgcagcgcggaaaagacgtggcgcgcgtgcaaggtagcggccgtcgggctcgcgcggcttttcagcggtggcatgctgcgcgacctgcgcgaattgttcgaggatttttgaccatgagcgagctagacattagcgcggttgtcgccggcatgcgcgacccttggaattactcggcgagcgttgcggaacgcgggcaagatgccggccgcatgacgtgggaagccgcatgcgaggatgcgcgcggtttgttcggcgagcatttcgaccgcgccgcgttcgatgagtatttttcgcatttcggcgcatgggacgcggaagaattggccgcgcatacggatgaagaatgcgccgcgcttatgctgcaattcatcgccggcgacatgcgcgaggctgatttttccagctatgcggacatcgaaggcggcgcggaaccgttcacggatgaatggtggccgcagtatgaaaaagcgagcgaggccggaaccgtcgccggccgtttctttcgcgacgctggcggcgttttttactacctcggagaatgaccatgcaaagcaaatgggcaaagacaaccgcgcagcgcatcgcatccggcgagctggcggaatccatcatccgcaaggcgcgcgcgttgctgcgcgatgccgtgaacgctgaagagtatttcaagcgcgaaccgtcgccgtctgctaccgctgcggaagcgtgggagctggtggagatgattagcacgcatgcgccgcgcgtcacggatgcgcaagcgcgcaagggcgcggaatggctgcgccgccttgtctacacgtcgcgcggcacggtgcgccgcacggaagccgcgcagcaattcagcgatgcggacctgcgcgttttgcaggcttgcatcgcgcgcccggccttccgtctggtggagctggaaccgcacagcgacggccgatacctgcgcgaccttgcgcccgtctatcgctgcatcggcgacaacggcgaatccttcgattacacggcgagcgcgtggcagtctggcggcgcgttcgcaatcctgcgccacgcttaacccttcccatccgtgacaagcccggagaatctgaaaatgtacagcatcgcaaacaacgcaaagcccgccattctgacgcgcacggaatcgcgcatccaatcgcagcgcgacaagcgaacgcgcgacacggaagcgcgccgcgcaaagtatcggcgcaacgctgcgcgctatctggccgcgtctttctggcaagggtcgcgcgacatcgccgattttttcaagggtcgcggattcgatcatgcgacgttgcaggatgcggaaaacgattgcatggataacgtcgatttttcttatctgtattcccgcgactatgcgcgtgagctggaaaaggaatacggcgacgacgcgcgcgaattgttcgcgtacctttgcccggatgcgccgctgagcgtgtaccgtgagcaaatcgccgacgacatgacgcgcgcggttgcagactcgcgccgcgcggattatgcgttgcagtttttcgactggtgccgcgatgcggtcgaggatgcggccgattcttccgggcttgtctggtgctatctggacaaggccggcaagcctacggatcaggaatacgacgcgcacgcggtaggcttcgcatgctcgcgccgcatgtacctttcgcgcgacgcggaatggtggccggaaaaatggtgggcgaaaggcgaaacgacgtggaacgattacgcgagcaatcgcgaacgcatggacgcggccgacgacgtgctgagcgaatttctcggcgagcatctggaaagcgaaggcgcggaccctgaatcgttcgatgagcgcggttcgcgttatgcggacgatgattactggccggaatacttcagcgattacagcgaagcgcgcgaagaatgggaaggcgacaaagcaaagatgcgcgcgcgtctgcgcgagatgatcgcgaaccgtgcgccgctggaattgcgcgccgcgcttgtcgcgagcgtgtacggcgagcctgaccgcgcggccgatgaatccgaagattgaaagggagctaacgacatgacgacgattaccgcatacgcatacaatgccgcgcttcattgcccgcgctgcgccttccgttatttccgcgtcgatcctgcgaaggtgccgccgggcgcggatgcgctggacggttgcaaggatcgcgaagggaacgcgcccgcgccgctgttttcgacagacgcgaacgcggacggatattgcgacacttgcgacatggcatacggcgacgcggaaccgcgcgcgcacgtcctgagcgttgacgcatggcgcgacggcgaaggctggacatggaataactggcacaagcgcggcacggtgccggttgcatggtgcgacctgagcccgcgcgcgttgctgcggaacctgcgcgcgcacgggctcgacctgccgccgggcgcggtatgcgtcgaggatgacggatacaacgtcgagattcaggcgcgcggcacgcgggaaccgttgtatgccatcgcctacggcgaggcgcagcgatgagcgctaagcccggcctagcagaaaagcgcgaaattctgcgcgctggcattctggcggatcgcatcgaacgcggcgcgcgctggctttgtttcgctgccatcgtatgcgcgggcgcgttgccgctggcatggggagcgttccgggcgcatggcatcgttagcgggctcgccgtgctggcgctggtgctggcgctatgctggcacgtcaagccgcacgggcgcagcctagcggcgcaagcgcgcgagattgaagcccgattcaagccgcacgattaaaagcgcgctgcggcgcgttccctgcattgcctaccctgagcccggccgcgtgccgggctttttattgcctgcgcgcctaagcgcgttctagcggcttgccgggcgcacgtctgcccggccttccgtatcccttcgcttgagcccgtggccgcatcgcctgcggccgggctttttctttttcccgctgcccggccctgcccgggctcgcatgcgtgccggcctgcccgctgcccggccttgcatggtggcgggcttatccgctgcccggccttgcatgcgtgcggcatagctgcccggatgcggcaacgtggaattaatgcagcgctgcgccgcataggtgcgcgcgtgcggcctttccgaatttatttattgcatcgcatgcccgcatgcgtgcgcgccgcgctgcgcgcgttctagcgcggcaggaagggataaagggatagccgctaggcgagtaaaaaggtacttccggccttgctgcgagcgtcgcggggggcgctgacagatcggaataacgtcgggtaggtaaagagcgtagttat

SEQ ID NO: 2 - DNA, 55251 bp, unidentified
  source 1..55251: mol_type = genomic DNA
gctaacgacatgacgacgattaccgcatacgcatacaatgccgcgcttcattgcccgcgctgcgcgttccgatatttccgcgtcgatcctgcgaaggtgccgccgggcgcggatgcaatggaaggcgcacgcgaccgcgaagggaacgcgcccgcgccgctgttttcgacagacgcgaacgcggatggatattgcgacacttgcggcatggcgtacggcgacgctgagcccgtggcgcaattgctgagcgtggaagcatggcgcgagcccgaaggctggacgtggaataactggcacaagcgcggcatggtgccgcttgcatggtgcgacctgaagccgcgcgcgctgctgcgcaaactgcgcgagcatggcggcgcgtaccctgcgccgggcttgtgcgcggtcgaggatgacgggcataacgtcgttatcgtcatgcgtggtacgcgcgaacctatcgcggccattgcctacggcgaggcttgcgcatgacggaaccgacactaaacgaaaaggcgcaaatcctgcgcgctggcattctcgccgatagcgtgacgcgcgcggttcgctggtgctgtttcgctgccattgtttgcgcgggcgcgttgccgctggcatggggagcgttccgggcgcatggcatcgttagcgggctcgccgtgctggcgctggtgctggcgctatgctggcacgtcaagccgcacgggcgcagcctagcggcgcaagcgcgcgagattgaagcccggttcaagccgcacgattaaaaacgcgctaggcgcgttccctgcatcgcctaccctgagcccggccgcgtgccgggctttttattgcctgcgcgtctaggcgcgttctagtggcattgccgggcgcacgtctgcccggccttccgtatccctgccctgagcccgtgcccgcatcgcctgcgcccgggctttttctttttcccgctgcccggccttgcccgggctcgcatgcgtgccggcctgcccgctgcccggccttgcatggtggcgggcttatccgctgcccggccttgcatgcgtgcggcatggctgcccggatgcggcaacgtggaattaatgcagcgctgcgccgcataggtgcgcgcgtgcggcctttccgaatttatttattgcatcgcatgcccgcatgcgtgcgcgccgcgctgcgcgcgttgtggcgcggcaggaagggataaagggatagcggctaggcgagtaaaaaggtacttccggccctgctgcgagcgtcgcggggggcgctgacctcggtgctcgcgcatttttcggaattttcgcggtttcgtctcctttggacccccgggcggccccgaatttccgaatttattccccgaataaacgcgaatttcctgtgacagtagtgacagtgacgtttttgggtactgtcacaaattcggccccccaagaaatccgctcaaatcaacgatttacgggcgcgaatttactgcgagtttaggctcagtgacactgtgacagtgacttccaatcctttacggcggaaagaaaagttctgcctgccaagaaaaaattctcgcgtatgagagaaggtactgtcactactgtcactactgtcacaagatagggaaaaaggtatgtagatcaagcacttgaatttgtgacagtaccttgtgacagtgaccgatttgcgcctcggagagcatggaaaaccgggtactgtcacaagaatcggcctttttccgaatttccgcccatacggttgcaattttttccgtatgtgacagtgaaaagaattcggaattaatttaatcggagccgctgcggggcgtcgtgcggaaattcggaaattccgggcaataaaaagccccgggggatgagcccggggccggcactgcggaaattccgccgaattaaatcgcgctcttcggcgctccatcgcctacacgcacgtcctcgacgttcgagccgttgtcgcccgcgcccggcggaagcggatcgctctcgtagcggttcgcgtcggtgttgttttcgtcgacggtcgcgttcggcaccatgccctgcggcttcgacgcgccgaagaagtcgccggtctcgcgcgctgtgacctgcaagtcaccgtgcatcgtgatttcgaccgagcggccgggtgcatcgagcactgcatgcaccacgccgttgccgtcgaccaactcgaccgccttgttgccgttgacgtgcgtgaacttcacggtagtcgtcatgtcgtttctcctgtgctcgggattgagcgtcttcgatcatacgctcgcaggcatgaaaaagcccggttgcccgggcttcttcgatcacaccttcagcgacgtgatttctatgtagtcgtcgatccacgcttgaaggttcggccgcaccaccacgtcaggcgagcgtgaccaataccgggcctgctttccgttcgcgccgcgcgcgcggcccacgtacacgaagcccttcgaggtcaggaagttcgacagcttcggcccgtacggcacaccgacgctgttgtccatcgccatgtcgcgcagcttgccgacgttgagcagcaggtggctcacttccgggtcgcgcgactccgcgatcatctcttcgatttcgtcttcgtcgtcgccgcgcgcgaggtcgatcatgcgcgacttcgcatcggtcatgggcgcatggccgtccgggtcgaactcgggatgcagcgggtagtcttccagccactcgcggatcgcacccgggtgataggcgattgcgttgaagatgtcgtcgtagtgatccgggtggcgctcgcggaacttctcgatcatctgcttcgtctggaagtgcgtcgagatgacgaagtagcggcggtcagcgtcgtagaccggcagcgcgtcgctgtggttggtcaggatgatggtcgaggtcacattcggcacgttgtacgagtcgcggtgcatgcggcgaatcgaaaccacgtcgttcgtgatgaagggcttcagcttatccatcaccgcgtagcgcgacgtgccgtggatgcgcgcttcttccagcaccacgaccttgcgcgactcgaagaacgacgtgtacttctcttcgagcgcctgtgcgttcacggtctcgacgttgttgcgcgacatgatcgccatgagcatttcgccgacgaagcccttgcctgcgccgtccacgccctgcatcacgaccgcccaacggattttcctgtccatgcgcttgatcgtgtacgccagccacgacagcaggatttcgcgctcgcgttcgaccgggtacgaaatctcgaagtggcgcttcaccgcctcgaccgcgcgccgggccttgctggtcaacttgtccggcaccggcacgatgtcctcggcgttgaacttgttcgcgtgcttctggccgtcccactcgacgatgcggtctgcgcccggcaggtagacgtagccgctgacgacgggaatctggtacacgttcaacgcgagcgcggcggcctgctgctcaggcacggcttccatgttcgcgcggtccttcttcgtcagcaggaagcggttgttgcgtgcgttgaatgcgcgctcgctcagtgcgagacggctgtccatgtagtagaactcttcctcggcgtcgacgtacaccacgtcgttgcaccaatgcggcagctccttgtagttgaagtcggaattgcggaagccttcgttgatcgccttgcggatcatcgcgatgggaaccttcttccccagctccgcaacgcgctccttgatcgcgccggccaacagctcgacttggaactcgttctccaacatgcggccccacttcgccgcgagcgggccaagcagctccatctccgaagtcgtctcggcgaccttgcgcttgatcttctcgaactgctcctgcgagtgctcctgccgatgctccttcgccatcttgataagcgaggcggcggtcgtcaggttgcgacccatgtcgtcgtggaacgagttccacttgaactccaactcgtccgggtcgtagttgtgcgcgggctcggaccactcgtgccaaagctgcaagccttcttcgttgccgtcgaattggtgatgcagcgccatgccgaccttcaaccactgctcgtagtcgtcggcacccggcacccattgcagcacttcgcggagctggtcttcggtcaggttttccagcgggcgcttgtattccagcagcgcgttgtcgttctcgtcgtcgctgctgcgcgattcggtcggcgcgttgtgcttcttcaacgtccagccgcgacgctgcgcttcgagcttgaacaccgagaacagttcgtcgatgtgctcggtcgtgatttccggcagcatgtcggccggcacgctcagcgggttcagctccttgcccgaagtccacttgtacggcttcttggtgtcggggtggatgccgatgccgacgaactgttggccgtccgcgagcacttcgatggcctgctcatgaccttcggtgtcgaggaacgtgatcttgcgcttctggaacggaatgtcggtgcgatatacgagcaacgtcttcggcgcacggccgactcgcgtcatcgtcttgccgatgatttcttccgtgtgctcagccatgagcgcggccatttcgtcatcggtgatgtcgatgtcgaccgcaggcgtgtgcttcgtgtggaagccgatgttgccctgcttgtagttgccattcgcccacttgcgaatctgcttctcgtccgcgcggattttctgccactgcggttcgattgggcctttccttcctgccgggatcggcaagatggagtacccgttttccagcaattgcgcgccgtacttacggagcacgctggtgatcggtcgtccagcagccataggtcactccgcgatgtcgtcgctaacaaggtcttcgaggttgaagccgatcttgcggttgaaatccttgtgcaagatggtcgccttgtcgcgcggcacaccgccgaggcgctgccaacgcgagacagtggtctcgtgccagttgtacttctcgcaaattgcgttgagccgaccgtacggcgggtcgagcatgagggcgatgcgccgaagcagatagcgcactcgcgcgtctgcgctgtccagtgaatcaagagtagggtctcggcgcatgaattcctcgcagacgttgggatttaaggggtctgctaagtcggtgagcacgcctattgacttagcatcgggacaggcgcatagtgcgctcgccgggcaggaattgcaatccacccgtcactcccgaaaccaacctagctaggagatacaaccgatgtcgaagatcaacgcgaagaagctcgccgaagccatcaccctcatcatcgaagcagtcggcggcggtgccgccaacgagtccgaggatgcgggcggcgaagaggaagcgccgaagaagggtcgcggccgtccggccggcagcaccaacaaggccaaggccgagaccaagcccgccgccaagggcaaggccaaggcgaaggacgaggacgaggacgaggacgacggtctcggcgacgacgacgatgccggcgacgacgatgacgacctcggtctcggcggcgacgacgaagaagtgacgcaggaagatgtcgtcaatgcgttcaaggcgctgaaggcgagcaagggcatcgacaagtgccgcgaagtgctcgccaagctggacgagagcaacgtgctcaacatcccgccgaagaagtacgccgaggcgctgaaggaaatcaaccgcgccgcgtcgaagaagtaactcggcctgcacgtcacacgaaacgcccgggttcgctcgggcgtttctttcggagaggaacacatgcccggttcgcacgcccgcttcgcaccatcgtcggcgcatcgcatctacgattgcccggcgagcctgttgctcaacgagaacgagcccgaccgcgaaatctacgaagcggccgagggcaccgttgcacaccacatcgcggaaatctgcgcacgcgcgcgccgcgagccggaagagtttctaggaatgacgttcgacagcggcgacctcgacgccgactacgacgaagagcagcattcctcgaaaggcttcgcaatcaccgtcgacgacgagatggtgcagggagtcggggcgtacctcgaccgcatcatgggcctgccgggcgaccactacgtcgagacgcgcgtcaacatctccccgtggtgcccgatccccgatcaattcggcacctgcgaccacgcagccgcgtcgcacaagaagctcatcatcaccgacctgaagtacggccgcgtgcaggtcgatgcgccgcagaacaagcagctcgtgatgtacgcgctcggcttcatcaacgagtacgactggctgtacgacttcgatgaggtcatcatccgcattgcgcaaccgcgcctcgatcacttcgacgtgtggatcaccagcaaggccgaactgctcgctatcggcgagaagatcaaagagcgcttcgcgcttgcgttgaagccgaatccgccgttcggcccgagcgagaaggcgtgccgcttctgcaaggtcaacttcaagtgccgcgcgaaccacgacttcctgtaccacgagcgcatcatgctgctcgatgacgacgacgagttcgtcgagcctgacctcatgctcatgagcgacgacgaaatcgctgcgctgtggctgcgcaagggcatgtacgagaaccgcatgcgcgcggtcgaagactacctgcacaagaaggtcgcggacggcgacttcgtgccgggcctgaagaccgtggcgggccgcagctcgcgctacttcaccagcgaaatcgacgccgagctgctgctgctggaagccggcgtgcccgagtctaagctgtactccaaacccgaattcgtgtcgcctgcgcaggctgaaaagctggtgcgcggcgaggcgaagaagaaattgcaggacttcatcaagtcgaagcccggcaaaccctgtctggtctcttccgacgacaaacggaaagacctgaccgtccagtcgctcgaactgctcgacgactgacgcaaccgttgtacgaatgcgcgaaagcgaactacgaacgtcgaatgacgaaggagaaatcgaaatggcgaagaagaaagttggtgatctggtcgacaagggcaatgggcgttttctgctgaagaacgtgcgcctgagcttcccgtacttgttcgagcccgacgagcaggaagacgacaacggcaacaagaagaagtcgtaccgcgtcaccctgctgctcccgaaggcgacgcacaagcccgtcgcgcagaagctctcccgtctcatctccgagatgtgcgaggaagagtacggcaacccgaagctggcggccgaccgcaagttcctgcgcgatggtgacgagtcggatgtcgaagatcatcacggctgctggacggtgacggttcgcgagacccggaagccgatcctcgtcgaccgtgatcgtcagcccaccgaggaagacgacgagctgctgtacagcggcgcgtgggccaacgtggtgatccgcccgtgggctcagaacggcaagtccatgaagaagaagaacaagtacggcaagcgcatcaatgccggcttcgacatcgtgcagttcgtcgaccacgacgacaacctcgcgggcaacgctcgcccggatgtcgacgaggttctggatgagctggacgacgacttcgcggatgacgacgacaacagcaccagccgcagcaagtccaagagcaagtcgaagggtcgttctcgcgacgaggacgatgacgacgacgggctcggcgacgacgatgacgacgaccgcagctcgcgccgcagccgtccgtcgaagagcaagaccagcagcaagagccgtcgctcgcgcgacgacgatgacgatgacggcgacgaggacgatgacgacctcggcatctaaaatcgggcatcggtaagcggtacctacggtcgcccgggcactccccgggcggctgtttttcagggatacggtatggacaagctgcatcacgacttcgagaccttcagcaagtgcgacctgaagaagcacggcttggcgcgctatgctcgcgacaagtcgaccgaagtgctgttcctgtggtacgcattcaacgacgaggaacccgaagtgtggttccccgcgacggagccgatgccgaagcgcctgcgccgcgcgctcaaagacccgaacgtgcagaagtgcgcgcacaacgctcagttcgagcgcgcgatttggctgcacgtcctcggcatcgacatcccggtcgagcagttctattgctcgatggcgcacgcattctggctctcgctgcccggcaacctcgacgaactctcgggcgtgcttcgcctcggcgagaacgcgaagatgaaggaaggcaagtcgctcgtgaagttcttctgcgggccgcgcaagccgacgaagaccaagcagtacacgcgcaacaccgcgcagaccgatccggcgaagtggaagacgttcgtcgagtacggccgccgcgacgtgatcgccgagcgcgcggcaggtcgcaagctctcgctcttcccgatgagcgatttcgagcgcaacctgtggtacatcgaccagcacatcaacgaacgcggcattccgttcgacaaggaattcgtcgagaccgcgctgcgcgtcatcgcgaaggagaagaagcgcctgctgggcgagatgagccgcatcaccggcctgagcaatcccggcagcggcgcacagttgctcccgtggctgcgcgagcgcggctacccgttcaccaacctcaaatccgcctcgatcaagaaggcacgcgaggattgggactggaacatgaccgatgaggcgaacgcggttctcgccttgcacgcggaagcggcgcgttcgtctgtcacgaagttgcagaagatgctcgacatcgaagtcgacggagtgctgtgctacacgatgcagttcgcaggcgcggggcgcacggcgcgctgggccggtcgcgcagtgcaggtgcaaaatttgccccgccccctccgcgaactagaagagcaaggggcactgctcatggcgcgcgatgcgatcatgcgcgaagacatcgagttccttcgcctgctggtgtcgtcgccgatgggcgcgattgcatcgtgcatccgcaccgcgatcaaagcgccgcccggctacgagtatgcaacgtgcgacttggcctcgattgagtccgtcgtcattgcatggctgtcgggctgcgacaagttgatcgaggtctttcagaagaacctcgacgtgtacaaggtgttcgcgtcgaagatgtacaaggtcgactacgagcaggtcgagaagtggatgcgtcaacacgcgaagcccggcgtgctcggcgcaggcttccgcctcagcggcggcatggagttgggcgagtacccggaagtcatcaagaccggcctgtggggctacgcggagaacatgggcatcgagatgtcgcagaaggatgctgcggccgtcgtgaaattcttccgcgaggaatacaccgaaatcgtcgagctgtggtacgagctggaacgcgccgtcgcgaaggtgatgaacacgaaggagccggtgcgcgttggtccgatcctcatggacgtgaagggaccgttcctgcgcatgcgtctgccgtccggtcgctacctgcactacctgcggccgaagatgatctggaagaagatcaaggtcggcatcgacaagaagaccggcaagccgaaatacaagtcgaagaagggcttcacctacgaaggctacaacacgaagaagaagtggacgcgcatcgactcgcacggcggcaagatcgtcgagaacttggtgcaggcaatcgcacgcgagctgctggccgccggtctgctgcgcgcttggaaggccgggctcgatgtgcgcatgcacgttcacgacgaaatcgttgcgctggtcaagcgcaagctgtcggacatctcggccgcgacgctcgaagagcagatggtcaagaagccgaagtggtggggcgaagacgttccgatccgtgcgaaggctgacgtagtggagtgctatcagaaatgagctggctgaccgattggcgcaacgtaatcaacggcaagccgccgcgcggcgacatcctgccgaccgacaagcatcgcgtcgaaaaggacgtggagcagaagtggtgcgccgttgcgaagcggcacggatggaaggcatacaagttctcgtcgcccggcaacagcagcgttcccgaccgcatgttcatccgcaacggcttcgtcttcttcatcgagttcaagcgccccggcggcaaggcaaccgacaatcaactcgaagagcacaaggagctgcggcgcaagggcatgatcgtgtgggtcatcgactacttcgataaagaattcgccgagtggatttttgagtgaaacaactactgaagcgctccgacctcgacgagtttcaaatcgctgccggcctgttcctcgaacgggtcggcagttgcgcgttgtggatcgacatgggcctcggcaagaccgtggtcgtgctcacgcatgtttcggacaaggtgttctccggcgagtggagccgcgtgctggtcgtaggcccgccgctggtcatctccgatacgtggtcgaccgaggtcaagaattgggagcacacccgcttcctcgactatcaggaactcgacggcgacagcgagcacatgcgcatgcagttgcagcggccgtgcgaggtcgacggcatctcggtgcataaactcgggcgtctcgcggcgctgttcaagcgaggcgacacggtgccgtgggacgcggttgtgttcgacgagtcgagcatgttccgcaacaagtcgtcgaagcgctggaagtacggcgtgcgcctgacgtggggccagccgaacgacgtgatcgagctgacaggtacgccgagcccgaacggcctgcatcaagtctggtcgcagattgcgatgatcgacggcggcgagcggctgggcttgacgtacaagaagttcctgtcccgctggttcaagcaggagttcatgggccgcaaagtgattccgaagtcgcacgcgatggcgtcgatcacgaagaagctgagcgacatcgtgtacaccttgcgcgaagaggattacgtcaagttgccgccgctccgctctacgcctgtgccgatcatcctgccgccggatgtgatggctcgctatcaggaattcgagcgcacgtctgtgctgaagtggggcgaagagcaagacccggcagtgcgtgctctatcggaaggcgcgctgtacggaaagctgttgcaatttgcgtgcggtcgcatctatacggattcagagacgaaagagttcgtcgacatacacgacaagaagatcgagcgcctgaaggaaatcgtcgagttcagcgacggctcgccgatcctcgtggcacgtacgtggcagcactcgcgtgatcggctgcgcgatgagttcccgggcatccgctcgttgaagacgaagcgcgacctcgacgcatggaacgcgggcgacatcgagatagccgagacacaccctgcgagcatcggtcacggcacgaacatccagaagggcggcaacaacctcatctggtacgaccacacgcccgacctcgaactctacatgcagttgcgcaaacgactgcaccgacgcggccagacccgaagccacgtcaacatgatgcacctgacagcagtaggcactatcgaagaggatttgacacgcgagctggtcaagaaagaaattacccaagacgccctgagagaacccatgcggcgacgagtcgcagacgtacagagagaactagccaatggccgcacctaagatcgactacgaagaagagtttttcgacggcatgaccgtgccgcgtctggcgcagttgttccgcctcgaccgccgcactgttaccgagaagctgcgtccgctgcgaccgaccggcgaccggcgcggcgcaccgacgtatcacatcgtcgacgctgcaccgtacctcgtggagcccatcgtcgacatcgccaagtacctcgcggaagtcggccccggcgacctgcccgcaccgctgcaagcgcagtattggaacgcgcagaacagcaagttgaagtacaaggaacagtcgggcgacttgtggcgcacgcaacaggtgctcgaagtgctgaccggcgtgttccgctcgctcacgcaatcgcttcgcctgctggccgaccgcatcgaagcgcagaccgggctcacgccggagcagcgcgcgatcatcgagcgcgaagtgtcagacaaggccatcgacatgctgcgcaagcgccttgtcgaagacttcgagatttacgtcggcatcaaggacaaggaacagctcgccgacatcaagctcgacgacatcggcctcgacgaagaggacgaagaagatgtctgacggcagctttttcaacgacctcggcgagctggtcacgttcgttgccgatagcgttctggttccgccggagcgcttgaccgtttctcaggccgcagcaaagtaccgctacctcgacaacgaaggctcgttcgtcggcgagtgggacaacaacgaaacgccgtacctcgtcgagccgatggacgtgctcacgagtcgcgagttcgagtcgtgcatcttcatcggcccggcgcagggcggcaagaccgaaatcatcctcaattggatcgcatacaccgcgaagtgcgacccggccgacttcttcctcatccagaccgcgcgcgacaccgcacgcgacttctcgtatcgccgcatcgacaagatgcaccgcgacagcaaggagctgggcgcgatgctgcgtccgggcagcgacaacgacaacatcttcgacaagttctaccgcaacggcatgatgctgacgctgggctggccgacgatcaaccagctctcaggcaagccggtgccgcgcgtcgcgctgaccgactatgaccgcatgccgcaggacgtggagaagaacggcccgccgttcccgctcgctcgtaagcgtacgacgaccttcggctcgttcggcatgacgctggccgagtcgtcgccgtcgttcgacgtgaaagacccgaaatggaaggcaccgcacccggactcgcatatgttcccgccgtgcgatgggatcggcggcctgtacaacgaaggcgaccgccgttgcttctactggcagtgccctcactgcggcgagtggtttgagccgaagttctcgctgctgaagtgggacatcaagaaccccgacccgttcgaggctgcgatgtcgacgatgatggcgtgcccgcgtaacggttgcgtcatcgagccgaagcacaagtacgagatgaatcgacgcggcgtgtggctgcgagaaggccagcgtattgatcgcgacggcaacaagctcggcgtcggcgttcgctcacgtagcgcatcgttctggctgaaaggcccggcggcgcgcttcattacatggcagaccctcgtcgagcgattcctgcttgcgcaccagacgctcgaacgcacgggcgaaaccaaggcgctgaaggccacgatcaacaccgatcaaggcgaagcgttctggccgctcaacgcgaaggactcgaaccgcctgccggaagacctgcaatcgaaggcgatccagtgggccgacaagaaggtgccgtacggcgtgcgcttcctgctcgggactgtcgacgtgcagaagagccgcttcgtcgtgcaggtcttcggcgtcggcccgagcgataacggcgtcaacttcgacctgtacctaatcgaccgattcgacattcagaagtcgaagcgcaaggacgaggctggcgacacactatgggtcaagccgtatgccgtgcaggaagattgggacttgattaccgagcaggtcgtcgagaaggaatacgagctggaagacggcagtggcttcatgtcgatcaagatgaccggcatcgactccggcggtaagtcaggctcgacgacgcgcgcatacaactactggcgctcgatgcgcgacaacggcaacggcggtcgcgtgctgctcatcaagggcgagccgaagctcggtgcgccgcgtgccgaaatcgacttccccgactcggatcgcaaggatcgttcggccggtgcgcgcggtgaaatcccggtgctgttcctcaactcgaacgtgctgaaggacatgctgctcggcatggtcgactacgacgagaagacgacgctcggcggcaggcacttcacgaacaagtggacgccggaagttgtgtacgccgaactcactgtcgagttccgcgacgaccgtggtcgttggcagaatccggctaagcgacgcaacgaagcgtgggacttgggctactactgcctcggcctgtgcgtgatcttgaaggtcgaaggattcgattgggacgcgcctgagtcgtggttcgcggagtggagtaacaactctcttgtgcgccgtgtggatcaggaaaaacggtttgcgtcaagccccactacggattatggtttcgccaagttcgggaaatccttgggatgacaaatggcgaccctagagcagttgcaagcatggctggcggaagcgcaaaccgcctaccatagcgtcatgatcggcggcggcgtgaccgtcgtcgtcgaccagaacggggagcgggtcgagtacagccgggccaacgcaaccggcctcgccaaatacatagccactttgcaagcgcagatcaattccctattgggggtcgcagtaaccggcggcccccttcgtccgttcttctgagggtaaaacgacatggcaaaagcactcactgtcgtgcgctctcccgagggcgacgaagcgttcaacagcaccggcaaagagtcggcgttcggcggtgcgtacgaaggtgcgtcgcgactcaatcggcagaccgcgttgtggagcgcgccgtcgctgccggccgacatggagatttcgccggacaaggttcggctcgatgcgcgcactcgcgaactcattcgcaacgatggctacatccaaggtgctctcgacacgagttcggactccatcgtcggcggtcagtaccttctcaacgcgcgccccgattgggagacgctgggcctgagcgaagagtgggctgaagagttccagctcatcgccgagcgcaagttcatgctgtacgccgagtctccgatgaactggatcgacgcctcgcgcaagaacggtctgaccggcctcgtgcgcatggcgctcgcgcagtctttcatgtcgggcgaagcgctcgccgctgcggagtggctgtcgaaggcaggccgtccgtacaagaccgcgatcaacatgatcgaccccgaccgcctgagcaacccgaacgacaacagcgatacggcgtacatgcgtcgcggcgtcgaaatcgacaagttcggcgcggccgaggcgtaccacatccgcgacgcgcacccgatggagtcgtactacgaccgcttcggcgcgaagtggacgcgcgtgccggcgttcaagccgtggggccgtccgcagatcatccacatcgccgaagtgctgcgcccgggccagacgcgcggcgtatcgaagatggtcgcggtgctgaaagaaatgcgcatgacgaaggtctacaaggacatcgttctgcaaaacgccgtcgtcaatgcgaccttcgctgctgcaatcgaatcggagctgccgcgcgagctggtgttctcgcagctcggtgccggcgacatgggttggttgcagaagtacatgggcgcgctggctgagtatgtcggttcggccgacaatctcgccatcgacggcgtgcgcattccgcacctgtttccgggcacgaagctcaacctgcaaaacgccggccagcccggcggcgtcggcagcggcttcgaggactcgctgctgcgccacatctgcgctgcgctgggcctgtcgtacgagcagttctcgaaggactactcgaagacgaactactcgtctgctcgcgcgtcgatgatcgagacgtggaagtacatgcagacgcgcaagaagctcgtcaccgaccgcttcgcaacgctggtctacatgctgtggctggaagaggaaatcaaccgtccgaataccgacctgccgctgccgaagggcgcggcgcacttctacgaagggatcaaccgcgaggcgtactgccgctgcgactggatcggcgcttcgcgcggccagatcgacgagctgaaggaaacgcaggctgcggtgctgcgcatcgcgtcgggcctgtcgacctacgaggaagaactcggcaagctcggcaaggattaccgcgaagtgttcacgcagcgcgctcgcgaaatgaacctcatcgaaaagaagaaactcaacttcacgctcagcaccagcaagccgggcacgcagaaagaaaccgacagccgcgcatcgaacaacgaagacgcggacgccaccgacgataccgacacggagaacgacgatgaatgaactgctcgcgatgcgcatggcgctcatcgagggattcaacggccgcccggcgttgatcgaccctcgtgatgtcgagaaggtcgcaacgctgtgcatgacgatggcgcaggcatctttcccgccgaccgccgagcagcgcgcgcaggcggatgaaagcatcaccgccgctgtcgagaaggcgttcgacgtttccttcccgcgcgaccgtgccaagccgttccttttcagcaacggccttgccttcatcccgatgcgcggcacgctcgtacatcgcaacggcgacccgtggtacggcacgcgcggctacgacgacatccgccgcgagttcgacgccgcgatggccgacccggacgtggcgggcgtcgtgttcgacatccactccggcggcggcatggtctacggcaacttcgagctggccgagcacattcgcaagggtcgcgacacgaagccgtcgctgtctgtcgtcaacgcgggtgcgatgtcgggcgcgtattcgctcggcagttccgcgaagcgcatggtctcgacgccttcgggcgacagtggcagcattggcgtgctgaccatgcacgtcgacatgagcaaggcgctcgaaaagttcggcgtcgccatctccctcatccatgccggcgagcacaaggtcgacggcaatcccttcaacccgctgcccgacaacgtgcgtgccgacatgcaggcacgtctcgacggcatgtggcagaagttcatctccgtggttgctgttaatcgcgggatgtccgaacaagcgattcgcgacacgcaagcccgtgtgtatcaggcggacgatgcggtcaagatcggcttggtcgatgcggtgatgtctccgcaagacgccatcgctaccttccgggccgaagtcttcggctctaccaccaacgataggagtgcaaccatgagcgacacgaagaagaccgacgccaccgtcgagcagaagaaggacgacgcgcaggtcgagaacaagaccgccgacaccaccgtcgacgcgggcaacaagaacgagcaggtcgatgccggcgcggcgatgcaggcgcgttgcgccgccatcaccggctgcgaggaagccaagggccgcgaaggtctggcgaaccacatcgcgttcaagaccacgatgtcggtcgacgaagcgaagtcgatgctggccgcctcgccgaagcagtcggccgccaccggcaagtcgccgctcgattccgcgatggacaacagcggcggcggtgccgacatcgccaacaacggcggcgacgaagaagagcaggcgcgcggcaacgacgacggcggcctgctgggcgcgtacaccgctgccaccggcaacaaggccgtgctgaaggtcgtcaagtaaaccgaacaccgtcgccagcctagacggaaaaaaccggctaaaccgtcaatcacagaaggagtaacgaaatgaccaacttcggccccatcgctggctacgtggctcgtaccgacacgaacagcatccagctctacgccggggaagcggacatcgtgagcacgcagggcgcgctcgtcaccggcaccgcctacgtcggcggtcaggtgctcggccgcgtcaccgcttccggcctgttcgccaagcacgacccggccgcgaccgatggcagcgagaacgccatcgcgatcctcgcgtacgacgtggcgaccccgactgccgacaagaaggaagcgatctacgtcggcggcgtgttcaacatggaagcgctgaccttcaacgctgccaccaacaccgacgccctgaaggccgctgcgttcgatggcaccaacatcgtcgcgcagaagctctacggtgcgccgcccgccggctccggcccggtctaaccggcatcaccaacagcaagacgtttcgcaattcaactcagaaatagaaggagacaacgatggatttgttcagcactgcggaactgcgcaaggtgatcgtcgacagccggccccccgtgcagtatttcctcgaccgtctgtacaaggagcagatcaacttcacgaccgaagaaatcatgttcgacgagctgaagctcggccggcgcatggctccgttcgtggctccgaacgtgcagggtcgtgtcctgaagcgttccggcttctacaccaagtccttccgcccggcgtacgtcaagccgaaggacgcggtgactccgggccgcatgctgcgtcgcctcgcgggcgaagcactgaccggcgacatgacgcccggccagcgctggcgcgcagtggtcgccgcgtaccagctcgaccagcggaaccagattttccgccgctgggaatggctgggcgcgcaggctgcgctctacggtcaggtcacgatttcgggcgaggactacccgaccgtcaccatcgacttcggtcgcgccgccaaccacacggtcatcctgaccggcaccgcgcggtggaccgaccagaccaacagcgatcccgacgacgacctcgaagagtgggccgctcgtgtgcatgacgccgaaggtttcgtcgtcacccgcgtcacgatgggccgcctcgcgtggaaggcgttcaagaagcacccggtcatcaaggagctgctggaaacccggcgcggctcgaagtccgaagccgaaaccggcccgggcctcggcgagtcggtggagttcaagggccagatcggttcgttcaacatctacgtctacaacgacgtgtacgaggacgagaccggcacgatgcagccgatgatggacccgcgcgacgtgctgctcgaagccgaggctggcttcgacggcgtgcgggccttcggtgcgatcatggatgcggacgccgaccttcaggcgctcgacatcttcccgaagatgtggaagaacccggacccgtccgtgatctacctcatgtcgcagtcggctccgctcatgatcccgagccgtccgaactgcacgctgcgggcgcgcgtcgtcgcgtaagcgtcgtcgcacacggcaagcccggttcgccgggcttcgctgtggcaacacaactccccaaccgaaagaaggagcatcaagatggcgaagtacaagttcgtggcccgcgtggcgctgaagggcgatttcgacgccgaagacggtctcggcaccgcgttgcaggaagtgcaggcgggcaccaaggccggcaccgacgacaagaagctctacgactcgctgctggaacagggctacatcaagtccgcgaaggacgccgcgaaggaagaggacgaggctccggctgcgtcgtcgaacccgagcaccgcgccgaaggtcgagtcgaccgacgccggcaagtccagcggcggcaagcagggcgcgggcaagtaagcccggcgcgctgaagggagaacgaaatgggctggctcgaaaccaagcagaaggctcggcaaaccgtgcatagcacgtttggtctgccggcccaatttcgcccgaggtcgggcggtgctgtcgtcgacggcaccgctcggctgcactacaaggtccgcacgttcggcgacttggaccgcgaaggcttcgcgaccgtcaccgaggcagtggactacatcatcatcgacactcggattttcgtgggcgctgacgaaggcgaccgcgtgttcttcccgcaactcaaccgcgcgttcaagctcgatgtgcgcggcgaagcggaagacgacattttcatcaagtgggaagtgagcgaggtagcgccgtgacggtcgaggttggcttccgtggattggatgacgtgcgcaagcgcgtcgccggcataccggaaacggtagaccgggcatccgcgtttgcgatcaacgaagcggtcacgttcggtcaggccgagagcagccgccgcatccgcgagcaggttgcgttcaaggccagctacatcggcagctcggacgatccgaacgctcgcctgcgtgtgtcgaagaaggcgcgcgtcggcgacctcgaaggcgtcatcgccggccgcatgcgcccgacctcactcgcacagttcatgactggcgcgaagctcggcaaaggcggctacgctcgcgtcaaggtgtcggcgcacggtgcagcgcgtcgaatcccgaatgcgttcccgatgaagctgcgtcgcggtaccggcgtctacgacccggagaacgcgaacgtcggcctcgctgttcggttgcaggacgggaagctgccgggcggcatgaacaagaagcagatggtgcaggtcagcggcaatctctatctgctgtacggcccgtctgtcgatcaagtgtttcgcgatgttcgagtcgatgtgcaagcgccggtcggcgacgtgctcgaatcgagcttcctgcgcaatttcgggagattgaaccgtggctgatacgaagcgcctgctgctgctgaagagcctgtgcaactacctgctgaccgaaatcacgacggcgaacggctacaacttcgacctcgccgccgcgtatcgcggcaagaagaatttcggcaaggaagtgaagctgccggcaatcgtggtgttggagaacttcaacccggatcgtctgccggagaccatcggcggcgtcgtcggcaccaagcacaagtacgaccagatttacctcatcaacggatgggccgaaggcggcgatgtcgagcaggaagaggactcggctcatctactcatgggggacgtgaagcaagcgctcggcaagctgctggtgccgcgcaatcaaagcgggtttttcgatggtctcgcaaacacgctgtccatcgagcccggggttgttcgccctcccgacgagcaatccgagaaggcgtatttctggatgaggattcgtctggaagtcgtcgaaaaggtgggagacccgtactggattcgtgattaaccgttgtatcgacagaaggagaccgtaaatgggcagcgagaattacacccttggccgtggcgaactgcacttcgacaagttcgtcgccggcacgttcaacaagaccggcgagcgttacctcggtaacacgccggagttgaaccgcaccaccgagagcgaaaacctcgatcacttcaacagcgaccgtggtatccgcgtcaaggacaagagcatcgtgctcgaaaagaacgacagcggtacgttcatcgccgacgaaatcagcgacgagaacatcgccctgtggttcctcggcacgcagaacgtcgtggcgcagtcggcgtccgcgagcgtggtgcagaacatcccggccaaccgcgtcaagccgggcacctacatccagctcggcgagtcgaccgccaacccgaccggccatcgcaacgtgacgctgaccagcgtgaccagcgatccggttggcacgaccttcgacaacctgaccgactacacggtcgacgccgagctgggccgcctgtacatcgtgccgggcggggccatcgacgggaccgccccgctgatcgtgacctacgccacggcggcctcgacccgcacgcagatcgtggtcggcgagggcaccaccatcgagggcgcgctgcgcttcatctcgtacaacccgaccggcccgcgccgcgactactactggccctacgtgcagctccgggccgatggcgacttcgcgatgaagggcgacgaatggcagcagctttcgttcgcattcgacatcctgaagcgggacggctacgcttccgagtacatcgacggtcgtccgaccgtggcgtaaccggggtacgtcaaacgcggtcaaggccaacttagtcaagatcaagcgagccaagaccaacttcgacaggccgcctcggaacccccggggcggcctgtttcgcatcaccagccagaagaggaaagtccatgtcccttgccaacctgcaactccgcaccgcaaccgttccgtatgtcggcgcgaacgacgagtcgcacgacatcgtgctgcacggtctgagtgcgaacgccatcgccggcctcatcctgtcgcagctcagcaacatcgaagaaatcttcaacatcgtcgaggcggccggcgtcaagaagaccgaagacctcgccaacgtcaacatcgccgaagtcggccaacggcttctcgtgcagctccccgacttcatcgcgcacgtcatcgcgtactccgcacacgagcccgagcagtggagcaaggtcatgcacctgccggcacccgtgcaggtcgagtgcctgacgaaactcgcgaagctcacgttcaacgacgaagccggcttccgagaattcgtgggaaacgtggtcgcggcgctgcgaagcgcaaaaggcgtagtgccgcagactctcaaccgaaatcccgccgtcaacgcttcgccgaatggtggcttggcatccgagcagccgtctctttcctgacggctgaaggtcactcgaacgctggcgaatatccgctgggatatttgatcgtcgaatcggaaatcgcacgcgagcgggtgaacaacagaatcagaaccgaaatgacgctgacgcagagtgcaatcgcttcggcgctcagcaagaaagcagcatcggcattcaaagaaaacatcgaaggactataggcgatggccgctcagaacgaagttgaactgattgtacgtgcgaagaacctcagcacgcgaaccatcaaccagctcaacgacgagctgagcaagatcgcagataaccaagagcaagtcgccgatgcgaaccgcttggcggagcggtcgttcgagagcctgaagtctgagcagcagcagttgctcgcgatcatgaagtctctcaacgaccgcgcttccaagctggacgcatactcgcgtcaagagcaacaggtgcgcagtctgcgcgacgagctgagtcgcgcccgcgacaacctcaacacgctcgcgcagcagttctacaacaccgaaaagccgacgaaggaattccagcagcagttgaagtcggctgcgagcgaagtcacgcggctggaatcgtcgctgcgcaataacgagcgccggctcgacacgaccggcaacaagctgcgcgacatgggcgtggatgtcacccgcttctcgcagtcgcagcaggaagtcaatcaggcgctcaacagctcggtggcgctgtacaagcgctcgaccgacaacgtggagcgctacgacgcggccgtcaaggaagtgcgcacgacgcagcagcaggctcgcgaggccgagcgcgccgcagcgcaggaagccaaggactcggcggcgaagctggaacaggccgcccgcgagcgcgaagaccagatgcgccgcgaacagaaaatggccgaactgacggccaacgtctaccgcacgctggcccgggagaaggaaaaggcggcccgggcgggggtggacttccgcgccaccggcacgcaggcgctcgccacggcccgcgcgaccgctgcccctgccgtgggtagcgggtcgtctgccggcgcggctgcggcgggcgtacaggcgcttctcgacccggccaaggatgccgtcgcgacgctcgaccggctggaaaaggccgtcgaacagctcgacgaggaattcaaggcgctcacgccggacgctttgcaggccgccgatggcatggacaagctggccgatcaaagccgccggctgcgcgctgcgtcggatgcgctgaaggggcaggccgggctcgcggacgaattgaaccgccagaacaccgcgctgctcgccagccagcagcggttcgaggaagcgcggcaagaagtgatccagtacgcgcaggcggtcgagcgtgcagacaagccgaacgacgagctggcgcagtcgttgcagcgcgcgcagaacgagatgaagcaggcgcacggcgagctgacgcgccagaccgaggcgttcaaccgcgtgcagcagcgcgccgctgccgccggcatcacgctcaacaacctgaccggcatcgagcagcgtctcgctcaggccgccgcgcgcgtgcgcaccgggcaggagcaggttgcgcagacgatgacgcggttggagcagacgaccgcgaagaccaacacgcagttgaagctcttcaacgacggacagcgcaccgcgctctcgttgtatcagcgcacccgtggtcaggtgctctcgctggtgtcggcgtacgtcggcgtgttcggtgcgatcaacctcgtcaacagcgcgatggacgcagcaatcgagaaagagcgcgtcatgtcgcgcctgctcattgcgaataaggggaaccagactgcggcagcggaagagtacgactacctgcgcaagaaggctgacgagctaggcgctgcattcggcccgctcgccgagtcgtactcgcgcttcgccgttgctgcacgcgatgcggggatgagcaccgaggcgacgcgctacatcttcgaggcgttcaccgaggctgcgaccgcaatgcggttgagcggcgacgagacggccggcgcgttccgtgcgctggaacagattttctcgaagggcttcatccaagcggaagaactgcgcggccagttgggcgaccgcatgaccggcgcgttcaatctgttcgcgaaggctatcggcgccacgacgcaagagctgaacgacatgctcgaaaagggcggcgaagtgaaagcagagttcgtgctgctcgctgcgcagacggcccggggcatctatggcccgcaagcgaaggctgcatcgaacagcctgctcggcgacctcaaccgcatgcagaacgcatggggcgacctgaagcgcgaaatcatcgacggcggtctcggtgatgcgctgcgccgcctgttcgtcgacttgacgaagtacctgaagagtgacgacggccagaagttcgccgagaacttgacgaaggtgtttgtcgctgcggccgacgctggcggcgagctgctgaaggtgcttgctgagaacgatgaaatcatcaagctactggcggacaccgttgcgttcctcatcaagaacttcaaggcgctgctcgcgattatgctcgcgatccaaggtgcgcgcatcgcgttggtgttcacgcagcttgcaggcgaaatcctgaaggcgcgtgcggcaacgctcgcgttgaacactgcgcttggtgccggcaccgccgcgtcggcgggccgtgccggtgctgccttgggcggcctcatctccgggccgattgccgcgatcctcgccatcgctgctgcgggcatcgtcatcccgatctacttccagattaagggcgagctggaatcgaacaaggtcaaggtcgacgcgcagaagacgatcaacgacctcaaccggggcttcgaggtttcgcagcgcagcctcagcgacacgtcgaagaccaacgccgaacagctcgaacgtcaggtcacggccgcacagcggttgctcgacatctacgacaagcagaaggagtcgttgcaggcgcagattcgcgagaacactgctgtgcgccgcaaccaagtggcggtacgtgttgcgcagggcacgcgcgagcacgacatgaatttcccggccaagcagctcgccgccgttcgagaagtcgagaacgaaggcaaggcgctggaagcgcagctcgccgcactcgaacagcgtgccgcaccgttgcgccagcaggtcgccgccgccggtcgccagatcggtgaagtgaaagcgcgcgaggcggctgcggagaacgacgcgctcgcggccgagttcaggcgcatccaagctgcggccgatgcggctgcggcgcgtgccggtaccgacgccaaggcggcgaaggcggccgaggctgcacgcaagaaggcggaagccgaagagaagcgtctggccgcgctcgccgagcgccgcctgcgtctggaagaggacgtggcggaaaagctgcgcgacatcgacaacgacattgcggcgtcgcgcccggatacgctcgaagcgcgtctggccgtgatcgacaacaagatcgcggatcgcaaagccgaactggaacgcatgctgcgtgaagtcgacaagctcggtcagtcggatgcagccaagggcgaaattcagcgcggcctcgacgcactgccggcgttgcagcaagcgcaggcgcaggcgaccacacaggagttctacgagcagcggattaatgacttgttgcagcagcgacaggcgtcgatggatgcgatcaacacgttgcaggaagccggtttgctgactagcagcgaagccgccgcgcgtatcgaggaagtcaacgctcgcctgctgccgcagctcgaagcgttgcgtgcgaaggcggctgagttcatggcgacgctgggcgatggtccgcaggcgcaggccgcgcgcgccagcctcgaaaacctcagcgcgcagattcaggcgatgtcggtcgagctgtcggcgcagaagcgtcaggtcatcgacgtgttcgtcaacggcttcggtcaggcgttcatggagaccgcaacgctcatctccgacacgttgaagggcgtgcaggatgccggcgacgcatggaaggcattcggcgacatcgtgctcaacaccatcgccgacatcctcatccagctcgcgcagatgattattcagcaggcgattttcaacgcgctgaaggcggcggccgagaacagcggtggcggttggggccagattatcagcgcggtcgcgagctacctgcacgttggcggcgtggcgggctccggttctggccgtcgttcgtcggtgccggcgtacgtgttcgaggcagcgccgcgctaccacacgggcggcgtcgcgggcctcgcgccggacgaagtgccggcggtgctgaagcgcaacgaggaagtgctgaccgaagatgatccgcgtcaccgcttcaacggcggcatggcgggcggcgctcagcctgcgatggacgtgtccatcatcaacaccatcgacagcgagagcgtggtcgctgccggcgcgaacacccgcgcaggacgccagtccatctttaacgcaatcaaggctgaccgcagctcgtacaagaaacttctcgcataaggaatcgacatgggacacgcaattgcaactgtgactggcggtagcggcgacgaggcacactacaaggtgcttgctgcaatcaagacgctcgctgaagcgaacggctggacgacgctgcgctacgtcaacaccggaaccgtgcgcgagttgatcctcaactccgccggcctgtcgggcaccgaggacatctatatcgggttccgtacctacagcagcgtgagcggcgactactacaacatgctcgtcggtacgttcaccggctacgtctccgcgaactcgttcgactcgcagcccggcgcgaagctgagcggcgtgccttgccacaacaacgcggtgacgtatttcatcactgcgaacgcgcagcgcatcgccggctgcttcaaggtcggcactccggtctacacccacttctacgcgggcaagatgttcccgtattcgcgcccgggcgagttcccgtcgccgctggtgtgcgccggcatgttcgatggtgctgcaccgaagcgtttcagcgacaccgactaccgcttcccgtatcacggccgcgagtcgggctacacgggcggctcgtcgtcgaatgtccgaccgtcgtacctgtggctgcgcgatcaagccggtacgtggcgtcgactctcgcatttcccgttctacaacggccccgccggcagcgatgcgtcgagcgcttacaacgcactcgaaaactggaactacctgactggcggcgaccaatcgcgctcgcttgttccggcgggcacgaattaccagccgcagccgatcatcctgtacacgaccagcgcgccggctggtgcgtgggaaggtgcggtgtacggcgagctggatggcgtgtatgcggtgtcgggcttcaacaacaacgtcgagaacgtgttgcaggtcggcggcacctacgtcgacccggcgggcctgagcatcgtcgatcacgtcgctgcgatcctcgccgctggcggccgtgcattcgtcgtgctgcaagacgtgaatcaaaccgactggcgcagctttatcgctttggagatgacctaatggcttattacaccggcaacttttcctcgttcgctacgctgaagaactcggtcgagaccgcgcttcaggcaaacggctgggggctcaacggcgacggcgtgctggaaaagaacggcatgtatctgcgcctcactgcgacggctgcgcaactgttgttgcaggccggcacgggcagcgcgaccggcgcgcttccgggcgcagctccgaacggcgtcaagatcatggacttcgagggctcgccgatgaatttcccggcgacctacgacctgcacgtcaacactggcccggacgaagtgttcctcgtcgtcaactacaacgccgacaagtaccagcagctctcgtggggcaagtcgaacgtgcagcagatcggcggcaccggcatgtggttctcgggttcattccacgagaacgctgcgtcgaatcagaaccatctcgtctacacgtcggcggatgcgagctacttcggcttcggttggtcgggcatgggctgcggtctgttcgccgagtattacacgcaggcgctcggctgctcctacgtccacacggggctcgacacgaccgcgtggcggcgcgtgtacagcggcgacggcaacctcattggctcgggcgatcctgtcgccggcctgctgcaagcgctgccttcgatgttcaaccaaaacaccgtgctgctgccgctgctggtctcgcagcgtcgactctcgcagggccagaccatcgtcgtcgacatggcgaacgcgcgactgtgccgcaacgataatcacctgtccggcgaaatcgtcgagtacggcgaggacaagtggaaggtttatccgttccaccgcaagaacgccgatgtgcgcaacggcgtctcgtggtcgacgggcgcgaaccactccggcaccttcgcatacgccatccgctacacggggccgtaactcatggcaggcatcaccggacaattcggcagtgaggttgagcgcggcatcgccaacgtgatgctgagcgaagacttggacgacaacaccgaagtcgtctcgcagttcgactcttacgaaatgcgcccgggccttcaaggcggctacgggcgctggcgcgtgcatgccgacaatcattgggcgatcaccggccagcgcaagtcgaccagcttcttcgacgattactacaaccgcatctatatcgtgccggccgcgctcgacgccggcaatttgctgtccacgcaggtgcgccacatcatcctgtggaacgcctacgtcacgccgcagacgttggagaatgccgcgctcggcccgcagtccggcatctcgatgtcgctgcctgtcggcgtgagcctgccgtacgagatggagccgctgcgcgagctggacttcacagtgcagatcgaactcagcggcccgccaaccatcgacagctatgcgaacttcaccgttgaaggcgtcacctacaccgtgccgatcaccggccgacgcatcgtgctgttcccgttctcgccgaattggggctcgcctgtcgacgaaacggtcacgatgcgttcgtgggtgctggccgccgaggatggcagcgagcagaccggcagcgagtcgggcgaggttccgcgtcgtacgctcgaatacaacatcaacctgcgcaccgcgttgcaagcgcaacgctgcgagaatctgctgttcgcgtggcagtcgcgcttcttcggcgtgccgcattggggcgaggaagaacgcatcgctgccgacgtggcggcgggctcgctgacgattccgttcaacaccttcggtctgtcgctcgaacccggctcgctggtggcgctctaccgcgacgacgagaagaacgaaatccgcgaagtgcaggctgtcgccgtcgactgcgttacggtcacgaccgggttggagtacgactggccggaaggctcgcgcgtctacccgtgcttcgtcggcctcatgaacgatgcgatgagcggcacgcgcgaaacgtcgacggtcggccgcatgcctatcgcgttcgactgcgagccgagcgtgaccccgggcaacgtggcgctcaatgcgccgccgctgacctaccgaggcaaggagctgtttctcggccgcaccaactggcagtcggcaatgccttttaccttcacgtcggatgtcaagcgcgtcgactcgaacaccggcaagtttgtcgcgttctcgtcggccggcttctcgaagatggctcgccggcacaactggacgttgtacgaccgcgccgacatcttcgcgttccgtcagttcctcggccgccggcagggcgtcgcgcgctcggtgttcatgccgagcggtacggtcgacttcaacatggctgcgccgatcctcgacactgaagacatcctcgttgtcgagaacaacgagtacggcgcgctggccggcgcacacccggctcgccgcgacatcatcatcgagctggtcgacggcacgtacttctgccggcgcattgtcggcacgagcgacttcgacagcttcacccgtctgcaactcgattcgtcgctgggcgtgtcgctcgacatcgacgacgttgcgcgtatcagcttcctcacgctgtaccgcttcgagtcgccgtcgaccaccatccgccacctgaccgactcgaaggctacggttgaagccatcatggtcgccaagaccaccgaggattgaaatgagcctgctgcaatacgaacaagacaaggaactcagctcccgcgtggagctgtacctgttcgagagcgatgacggccgctaccgctgggcctacacaactgacgcgcgcgaaaaggtgctcggccctatcgtctacaagcccgagtcgatcaagcgcggcgagctgaagcagacggccggcgacgcgaacgtcgagaaccttcaggtcacgatgccgttcgataacccggtggcgctggcgcatgtgccgtacctgccggcgcggccgatcaagctgacgatctacgcctaccagcgcaacgatcctgctgcggaaatcgtgcaggcgttcaccggcttcatcaccagcttcaaccagaagggcgcggaagcgacgctcgaatgctcgcagatcatcgacaacctctcgcagacggtgccgtgggcggtgttcaagagcggctgcatttgggcgctgtatcaggtcggttgcggcgtcgacaagcagttgtggaagaacgatgcgctggtcacgaccgtcaacggctcggtgctgggctcgcctgagttttcggccaagccgaccggctggtacaccaacggattcgcctacaacccgcagacgggcgagcagcgattcatcgtcgcgcacgatgccgctgccggcacgatcacgctggtatacccgttcctcgaaatcaacggaagccagaccatcgaggtctacgcgggctgcgcgcgcacgaaggaagtgtgcgctgacaagttcaacaacaagctcaattacgtcgggttcgaccacttcccggcctacaacgtcttctcgcaggggatcacctaatggtttgggtagccatcgtagttgcgctcgtcatggcagtagttggcgagctgcttcggccgaagccgaaattcaacgacccgaagccttccgctgtcggcgatttttcgttcccgactgcggacgcatcgcgcgtcattccgatcttcttcggtacctgcaagatgcaaggcccgaacgtcgtgtggttcggcgacctgacgatcatcacgctgaagaagaaggtcaagaccggctggttctcgtcgaagcgcatcgtcaccgggtacaactactacctcggtgtgcagctcgtgttcgcctacgggccgtgcgacgagttcatcgagctgcgtatcgacgacaaggttgcgccgatcaccagcaagaccttcaccggcgacgtgtgctcgttcacgatcaacgcgccgacgattatcagcaacgacgacccgccgaatggcgtcaaagggccgtgcaagctgtatcgcggcactttcgagcagccgccgaatatgtacctcagcgcacaatggaacgagccggagatgaccgcgttccgtccgctgctgcacatggtcatggagaagtgctacctcggcaacaccgacacgccgccgcccatctcgatcatcgcgcgccgctgcccgaaccagctcggtttgaccggcggccggcacaacgtcaacggcgactcgaatatcgcgtgcgcggtgtacgaggtcatgaccaacaatatgtggggcatgaaaatccccgaagacaagatcgacgtggactcgttcatcgcctgcggcaacacgctggctgacgagagcatcggcatctcgatgctggttcagaccgccatgctcggccgcgacctcgtggcggaaatgctgcggcacgctgacggtgtggtgtacgccgacccggtgacgggcctgtacacgatgacgctggcgcgcgagattccgtccgacgagcaagacgagctgttgatcgtcgacgactcgaacatcctgcccgacactttcgagttctcgcgttcgtcgtgggagatgacgaagaacacgatcatcgtgcagtacaccgaccgcaccacgttcgagacgacgccggttcagtaccaagacctcgcgaacatcgacgtgcgcggcggcatggtggattccgaagaattcagctacctcggcttcagcaactcgaccgccgcgatgaacaccgccgcgcgcgtgtcgaagatgaaggcgtcgccgttggtgtcggcgaagatgtcgctcaaccgcatcggctaccaactgcgtccgggctccgcgttctggctgcgcaagccgaaccgtggtctggcgaacgtgctcatgcgcgtcatcgaaatcaactacggcacgctggacgacccggctatcaaaatcacggcaatggaagacatcttcgcggtcaacgccgtggcctatgtgccgcccgatccgagcgactggacgccgccggtcggtgccgtcgtgccgttctcgcagcagcgcctcatcgaagcgccggccttcggtgccgaggatatgtcgcgccgctacgtcatcacgatgggagtgccgtcgagtaacggcgtgatcgcgtacgacgtgtggacggataccagcggcggcaccaacttccagcagaccaactccatcgacgcgctcacgccttcgggcgtgctggtgtcgggtctgtcgcgcactggcccggaagtcgatgttgcgggcttcaccgtcacgtcggtcgtcggcgtcagcgacatcgaatccggcactacgggctcgcgcgagtcgggcgaaaacctgctgctggtcggcaacgaactcatggcatggcaaaacatcgtcgacaacggcaacggcacctacacggtcactggcgtgtatcgcggcgtgctcgacacgatgccgcaagaccacggctccggcgcgcgcgtttacttcatgtcggaaggtgcgggcacgaccaacgaagacggctacggcggcgacctgacgctcaacacgaagctgacgccgaagagcatcgtcgacacggtgccgctggacaacgctgcggcgatgtcggtcacgaccaacgctcgtgcgctgcgtccgctgccgccgggtcgtctgcgcatcgacggtgcagtcgtcggctccggcgcaacctacgacggcgacatgctgttctcgtgggcgcaccgcaaccgcctcgacgacagcatcgcatcgcaggccgatccgagccgtacgcccgaggaaggcacgacctacaacatccgggtctacaccagctcgaacgcgctgctggcatctgcgctggaagtgtcgagcgccgcgtcgaccggcaccatgcggttcgcggtgtcaggcgatatgcgcattgaaatcgaggcggttcgggacggctatgtgtcgtggacgaaactggtcggctacttcagctatactccggcctcgggggctaccgccaacgaaatcatcgtcgacgagcctgagtacgtcttggacgggggtggcgcgtaatggcacaggtagtcgttgcacaacgcatgtggcagcgccgcgacactgcggcgaattgggctgcgaagaatccgatcctcgcgggcggcgaaatcggcgtgcagctcggcgctacttcggacgagaccaagttcaagatcggcgacggcgtgaccccgtggaactcgttgtctttcttcgagggccggctcatcgaaatcggcacgggcggcggctacatccgctggcgctacgtcggtgacgagacgtggatcaatctggtctcgcttgaatcgctgcgcggcccgcagggtgcgcaaggcaacccgggcgcgaacggcctgagcgcgtatcaggtcgcggtcgccaacgggttcgccggcacgcaggccgaatggctcgcatcgctgaaaggcgagaagggcgatcaaggcgaccaagggccgcccggtattccgtcgcagcgtcgcatcctgcgtatcacgaacaccgacagcggctccatcgtgtgcgactggaatgcctacgacgaaattcgcgtgacgctgactgccgacacgctcgtaaacatgacgggcgcgctggacggtcaaggctgcgtgctgctgctgaagcaaggcggcgttggcggtcacggcgtttcgttcggcagcaacgtgcgcttcaacaacctaatcccgatttacaacccgacaacgactgccggcaagtccgacaggctcggtttcgtttatgacgacgacgccggcttctacgacgtgcaggcaatcgtggatggaatctaacgatggcagacgactacatcccgccgttgtcgccgaacatcgtgtgggtcttcaagggcaacgactacacgcccccgctgaccccgaacatcgaatggatattcggtgcagatgatgaaggcggcggaaacgagcttcgcaaatccacctacatgctaatcctgacaatgtgaggtattgaaatgactgttcgcacctactcttcttccgacgctggcgctccggttctgcgcggtaacacgccgggcgacctcatcaacctgctcgaaaagtgcctcgtcaccggctacgggtcgaaggccggcgcaggttggacgaagccgtacgccggcacgaacgtcgccgcgtttcagcagggcgcaggctcgaacggcatgttcctgcgtgtcgacgacacgagcactgcgaccagctatcgcgcagcgcgcatcgttggctatgagtcgatgagcggtgtcaacaccggcacaccgacttcgttcccgacgccgacgcagcgcagcggtggcgcagcatggttcacgcactacagcagcggctcggttgcgaacccgcgcccgtggaaaatcatcgctgacgaaatgttcttctggttcttcctgtcgacctacccggaaaacaacgacagcggcttttactacaacgagagctatgcgttcggcgacatcattccgtttaagccgggcgacacgacgcataccgttttgctcgccagctactcggtcgactcgccgaattcctcggagccttacccgtgggatggcgtcagcatttcgagcgcgatgggaagcaatcgctacggcctgtgggcggcgcgttcgtacacgaacctcggcggcccgatctggctcggctggcacgccgatcacgtcaaggcttcttcgagctggggccaagggttcctgtcgtatccgcacggcccggacggcggcctttacctatcgcctgtgtgggttcacgagtaccacgtctcgccgtacaacgtgcgcgggatcatgccgggcctgtgggtgccgtgtcattaccaaggaatcctgagtcagtatcaggagttcgacggacagggcgagctggcaggcaggcggttcatggcgcgccgccactatgagcgcacggtctgcatcgaaatctcgaatacttgggataggtaacgcgcgatggcgctcatcttcaacctgccgatgacggggccgaacggctccacgacgatcaccgacaccacggggaatttctcgtggtcggtgacaggcaacgcgcagattcaatccaacgctctcgtccttgacgggagcggtgactacgtgagcaccactgctgacgttcgattgaacttcgggccgatcaacgatttccgtatcgcgttcgacatgaagatggcggctgcggacaagggcggctataaaatcatcttcgaccagctcaacacgggtgcgtcgaatacgtggacgtggcagctctacacctatgaaggtgtgccgtacttcaacgtctataacaattactacggcaatccgacgccggttcaaggcacgaccgatcttgctgacggcaactggcacacggttgaagtcattcgcactggcggcgctctctcgatgtgggttgacggcgtgcaggttgcaactgctaccgacaatcgcgactacgtgttccagccgcctttcggtatcggttcgcgtatcggctacaacgcatcgtcggcctacgactacaagggcgagctgcgcaacctgtccatctcgatcacgacgccggtcatcctgacgaatcgcatcgcgtcttggactcggcacagcgacatcggctggaaccgtggccgccgcagcagcttcattcggcgcatggcgttctacccggtgcagccggtcacgaccaagaaggtgcagacggtcaaggtgacgcgcggcgtaccgccgtggtgggggccaagcgggtcgaccacgcagctcccgacctacaagctgcgcggccgggtgatgcagcgcgatcctgacggcgtgttgcccgacgccccggtacagtacgcgcgcgtcgtgctgttcttccggcgcttgcatacgctcgtagacatccagctctccgatgtcgacgggtacgtgcaattcgataacctcatgccgggcggtcaggcgtactacgcgattgcattcgacccggaaggcgcaccgttgcagaacgcggtgatttgggatcggctgtcacccgagcccggcccgtaaggagaagtgccgtgagccagaacaacacccacgagcggaacaggaaccgacgagtgacggacaaggcagggggacttttggacgccgcgcagcaggccatccggcttgaacgcatcgaaggcgatatgcgtctgctcacgcagcgcgtcagctccggcatggagaacgtcagcgccacgctcgcggctgtacaggtcgaagtgcgtggctgctcgacgaacgtgtccgagctgcgcggcctgcaaggtgcgcacgactcgaacaaggtggcaatcgacaaggtggagaaatcagtgaccgacctcggtgcgcgcttggagtcgtggttcgatgagttcgaggcaaagcaggaacagcggtggcgcgactatcaagccaaccgcgaccaatggcgacgcgagcacgaggccgagaacgagaacgtcaagaaggacttggaaaaggaaatccgcagcgttcgcgagaccgtcatccgcttcatcggtttcggttccgccataggcgcactcgcgggcgtcatcgttgctggatttttgtggaatatcaactaccgcttcaccgacaacaaagaggacaccgaccgcgtagaaaaatcgtcggcctacaaccgccagctcatcgacgcgatgggcgtggagcacggcagggagttgtccgacatcaagctgtacctcgcccgtggtgggcgaatccccgaagagccctacgttccgcaatcacagaggaaggaaaatggacacgaacaatccgcagcaagcagccaacccgcaaagtgaagtgccgatgcgcacgcgactgtgggagttctggcggcgcaaccaaatcatcctgttccagctcccggtcatgctggtgttcctcatcggcagctacatcgtgctgaagtcggtcgactcgcgcatcggcgtggaaggcttcggcgacatcttcggctacgcgctcaacgcggtgcgcatcacactcatcatcttcaccgcatggtggatgaagaagtggtgctggttcgacctgcacgaccgcaccgaactcgaactgttcgacctgcgcaagcaaggcaaccgcgacgcgcactggatcgtgtggaccgaccgcatcgagtggatgctggcgctcgcgctcgcgaccttctggtacacgcgatgaggggccgggtcgtagttctcgctgcggccctgctgctggccgggtgcgcccggcctgcggccgtgccggcggtcgaccagaccgtgctcccggcggccgtcgacgagctgccggcggccaccccggagcccgtggtcgaacaggtcgtttcggagcaaccgctgccgaccgccgtcgaggcggcttcaggcaccgtcgcggagccgcttctggctgcgcaggcggcgctcgaagacctgaccccgctactacccccgccgccggcccgggacgcggcttgccggcgcgctgcggcggccctgacgctacgctgggaagtgaccagcccggccttctaccggaagcggctcgaactgccgatctggccgggcggggcgtccggggtgacgtgggggatcgggtacgacggcggccaccagacccgcaccgtgattgtcgacgactggcatgaccacgggcaggtcgaccggctgggccagaccgccggcatcctcggccagcaggcccgggcggcgctgccgcgcttccgcgacatcccgaccggcttcgaccatgccagtcgcgtgttcgaggaacgcagcctcgtcgagtacgaacggcgcaccgagcgcgcgttccgcaacggcttcaccgagctgcgaccgaacgcatgcggtgcgctcatctcgctggtgtacaaccgtggcgcggcgatgaccggcgactcgcgacgggagatgcgcaacatccgcgacaactgcgtgccgaagcaggactacgcctgcatcgctgcggagattcgctcgatgaagcgcctgtggcgtggcacggtcaacgagaacggattgtctgcgcgccgcgaggccgaagcgatcctcactgaaaccccgtagggagaagagcatgtggacgaaagcaatcgcgtggctgttcggaacggcaatgggtcgcggtgtgctgctgggcggcagcatcgcgataggcatggcgctcggctggtatgcgttctcgacgcactactacaacgagggcgtcgcgtcgtgccaagctggccgcgccaccgatacgaacgcggccaacgtcgcgcaaggtgaaaagaacatcgccgacaaccagaccagctccgacatcggcaaggccgccgacgccgaagcagcgaaggtcgcagccgatgccgaagaagcgaagaacgactcgaaggagaccatccatgacgtgtacaagaagccccctgtcactgcgcctgttgctgttggttcttgcgtgcatcctctcgatgagcgggtgcaagaccggatcggcaaagcgcgagctgccgcagttgaagcaagaagccccgctcgttaactgcaagcagcctgcgtcgccggcagtgccgcgcgagccgaaggccgacgagtggatcgagtggaacccgccgcgcccgggcaagaccgaaggcgaagcgcggctcagcgagcgtgcggtgaactggatcatcgacgtgctgggcgtggtgcgagtgggcgagggctatcgccgcgtcgagcacaagtgcctcgacgagctggaagcgaaagggctcatccggcagtagttgacaggcccgaggcgctgcattacggttgatcccgctggcggcacttcgcgttgcatcggcactcggcagagggacagcggcgcggagaatcggcgctccgcaccgcagggaacgaggaaccccggactaacactccggggtttctttttgcgtcaagaccaagtgcgtcgtgaccaagttcgtcaagaccggaaaagagaaaagccccggtgctgaggccggggcttttcgggttgcgcgactcacgtcgggcggtgggtatcgaggcggtggttctgctgattccggtgtccgctctatgagcgctgcgccggctggaagggcatgtgtcgcgtcgatggatcgaacctaatgcggcacgcggcgcgtgtcaacaccctcgtcagtccttccactgctcgaccagcttcagcatcttcttgcgcgccttctcgacgccgctcgcccacttgtcccacgcacgcgcgtcgacgtgcgtcaggatttcgttgcgcgccatctcgctcagcacggtcggcggcagcgcgtccagctcccagctcttgtcgccgaagcgctggcggtatttcacgaagcgcgcgtcggtcgtcttggccgggttcggcggcggcttcagctcttcgatctggtcgaggttgagtgccatgcgcttcagcgtgaactcgccgttccagccgaacagctcgaagcgctcttcgaggtcgcgcgtcatgtcgatgccgctcgggtcgtgatccccgaagtgcaggatcaccacatccttgccgtcgctctcttcgatttcccgcttggcgaaatcgcgcacgaccgatgcgctcgggtagccgcgcgctgcgagcagcggcacgtcgaactcatggcacacgcgcgaaaacacgccgaccagcgcttccttctcgacgacgaggaacaggcgcttctcctgcgtcgcccacgggtcggtgtggtactgccgcgccgacgccgtgagaatgtcctgcgggcgcgaccagcggctccgctgctcgaacgagcgcgtgcggtcttcgatggcgtcccaatcaatcaggcccgcgatgcgtgcgtcgttgacgatgctcgtggtctgcttgtacgacttctcgttgttcggaatgatgtcgcgcgcaacgagctggtagtagagctggcgcacggtcagcgtgtaccccgcatcgagatattcttcgatgatcgcgttgatcctgtcgatctgttgcagggtcttcgtcttgaaggtgatttctttgtagcgttcgagactcatggcactcggctcctgttagcggctggcgggctgttcggcggcccggatgtcagtggcgcggatggattcgatttcaggcggcagctcgatgcgctcgaccgcgtagccaacatcgcggccgtagtacacgccgcgcacgtcgggcaccgggtagacgtggtagctgccggcgtgcatgtgcagcgcgtggtggatgcgctgctcgatctgcgggtaggtgtacgggttgtccgggctcggctgcacagtgcgcacgccgatgccgacgtagccgctgcgcgccagcgtctcgcggaacagcgcggtgtgtcccgcatgccacggctgatagcggccgatcatcgtgccctgcggcgtcaggtagcgcaggcacgcagcgatgcgttcgagcgtgggctgcatcacttcggccgtgacctgcaccgcgacttgctgcgggcgctcgaacatttcgtcggtgtccgggtagcggctcttctgcaccgtgtccatgaagacgatgaggtcaggcgcgaacgcctcgcgcgtctcttcggtcgggcacacgaacgacgcgacgacgatgccgtcgtggctgtccgcgacctcacgcatgagctgcgcttggcggatgcggcccggcgtactgaagtcccaatcgccgtgctcttcgcgcactgcgtcgccgtcgatgtgcgttgccggcaacacgcgcgcgagtgctgcgccgagcgtggtcttgccgctgcccggcagaccgcagatgagaattcgcttagccattgttcgattccttctgtgcgcgaagttcttcgcggatttccatgagcagcaggccgagatgattctcgcccttgccgtcgcacacgccccaaaaacggtcgccccaccaattcccttcgacgagcttcgacttcccggtcttcagcaggcgcgaccgaagcgggtcggtgccgaacttctggcgcagcaggtcgcgcatgacgccgaccttgatctgctcccaatcctcgcgcagcgttgcgtgcttgccgcgctgcttcgcgccagcggcactcggctcgttacgaatgcgacggcgctcgtcctcgtcgagcgtcttggctgcttggaaggcgtgctccacggtgcggtacgagtgcccctcgaaggcgatgcagcatgaccagaaattagagaggaagcggtacgggccgttgaagctgtcgatggtcttcatagtgtcccctagtggaagtcgatcttcgccttgctgaagagctggcgctgcttctgcatgtcggtgcgagtgatctggtcttggatgggaacctgcacgttgcgattcatcatctggtgcaggtagcgcggctcgaccgcgtgcccggttgcgaacttcgcaatcgccatgagaatttgcggcgagtgcagctcgaagaacgtgccggtcatcgaccacggttgcggtcgaatgtgcgccgcgatgtcgagcagttgccgctcggccttgcgcacgttgagcggcggctggatgccttgcttcttcatcgagtgctcgacctcgctggccgcgcgatgcacgacgaggtactgcgcgcccgggaaccggacgagcagttggtcgaagaagaacagcgcggccacgtccgacacgaacacgcggccgggcggctgcgcgtcgatcttctggcccagctcggcgatgctcgcgcactgctgaagcgggttgtgcatcgacgagacgcacagcggccgaaggaactcggccatccatgcgctgcggctgcgcggcaggctgagcatgatcgtcaggtgctcgtacgccatgtcagccctccttctgctcgcgcgcgttctttgcgttgtcagcgtacgtgtcgagcacgcgaacgaacgcatcgtgcagcagcgtgccggcgggcacgtagatcaccgtgccgccggtcaggtcgttgcgggtgtagatggtcggagccgcgcccgggatgagctggccttgaccttctggcgtcgcctgcatgcgatccggtgggcgcgagtcgaactcgcgcaccagaccgtccgcagggccaccgacgaagaagccacggacggacgtgttcatcgcacgtctccgtcgccctgcaacgtgccacgctccttgcggccgttgagcttttcgcggttgtcgaacagcagcttttcgtagccgccctcgcaaccgaccagcggccccgtgcgctcggcgtactcgactgagaccgcgatgacggaagccagcgcgccgcgcagctcggcgatcttctccgcacgcttctcgccgctccacgtcgcgccgtcgcgcatcatcttcttgatgacgcccagcacgcggcccgcgtgcgcgcacagcgccgattgcaggtcgtagccgctgatacgaacctcgcggtactcggcgtcggcaaggcgctgcatgccttcctgcaccagcacgtcgaagcgcggcagctccggcgtctcggcgcacaggcgcgcggcgtaccactgcacgtcgcccagctcgtgccacgccttctggtagcgctcgacacgaaactcttccttgacggcttcttggtcgaacagttcggccagctcgccgacttcgttcgccagaccgatgccggtgtacagcatgcccgcgctcacgttgccggcgagctgcacgatgtcggtcgggtacttggccgtggtgacggtgaaggcgttgtacgcctcggcgaagatgcgcgtgggctcgacgcgcgcggcacgcgactcgcgtgcggtatcgagggacaggatgctcatgcgcggcccccggcggcgagcgcgtcagcgaagtcgttgctgtagctggcctcgaacttcgtcgccatgtcgtgcaggacgagcgtggggccgccgtgcgctgccggggtcatggcgaagtcgacgccgcgcaccagcgggttgcgctcgccgtcctgaccgatggcatgcacgaccaacgcttcggggttctcgcgcgcggcgcggcgctcggccttcaggatgcgccgcatggtcttgccgccgaacgccttgcgcagcttttcctcgggcgagccgtggtcgcggatggcgagcacgccggcaatgccgcccttcgacgtgcgcacctgacgcttgttcttgcgctgctcgttttcgaggtcgcgctgctggacgaggaaggcgtagttctcgtcgacggcgagcatgcgcttgcgccagtcgctcagggtcttgcccttctcggcattgtaggaacggaaaatgcgcttcaacaggttcatcgtgtggctccttcaggtgtgaaaaaaaagcggcccggccgatgtcgacggggccgcttcgatgtactacttcaacgccaccgggctcagcggccggcgacgaacttggtctgcttctgcacccggccgcgcttggtctcgcggaacagcacgatggtcgtgttgtcgtcggccatgatgctcgcgtcgtcgagcgcgttgctctcggtcgcgaacgggccgttcatggtgctggccttctgcgaaccgtcttcctgcgcggtcagcagcaggtacgcgaactgcttcgcgcccttcttgccgcgacgcacgccgaccttgcgggcggcggtcttcttgccagcgggacggccgcgcttcttggcgggcgcggcggcctcggtcttcttcgcagcgcgcttggccggagccttcttcgcggcggccttgcgtgcggtcttggcgggagccttcttggtggccttcttggcagcggcgcgcttcttcgcgaccttgccttcggtggcttcggcgttctcggacatctggtttctcctagcgttgttgtcgacaactcgcggaatgcgagcggggttccctcgcgggattcggttcagtccacgcagtacgcggggacttcggtgcggaacgtccggcactcggacggctgcgtgatgtacaggccggcgatggcggccagcagcaacacgccgtagacgatcttctcgcggcggctcatcactcgcagcccacggtggcgttcgggcgggtcggatgcgcggcggtgtactggctgaagtcgcgccagccttccgagccgccgcacgcgaagccccagcggcgcacgatggagccggtcatgaagagcgtccagcacggctcgtcgttgttgccgaacagttcgagcaggtgcatgtggtcggcgctcaggcggcggaagtcgcccgtgtggaagtgctgcgtgtagtcgaacttgtgctggcccgggaacttgcccttgttgcgcaacacgctgccttcgacgaacgtgcggccatcgttcggagtgaacagtcggtgcatgtacgagacgtgcgcgtccatgccttcggggctctcgtcgatggcgtgctcgtagcaccactcgctcgtgtgctcgatgtagcgaccgtcgaggatgagcgacgcactagcccacgggtgatcgtgcagtgcgcggtcgtcgtcgccatgcacgaacttgtgcaggtacaggttgaaccagcggttgcgcgggatgatgtgccagcgcgtcaggtacgggcggcgcgggccgccgtcgatgccgtcgagcatgatgaccttggacggcgagacgatgcgcgcgtacagcttgaacgcaccgacgaagagcggccacaggccgatcatcgagagcgcgttgtagaagcggcgggagaccttgggggcggtcatggcggggaacatcctcggtatggtggggtagttcatgcgtcgagcgtcgcgtcggcggtggccgggccatccgcgttggtcgtgtcgacctgcgggcgaacgagcgggagcggctgcgagccatcgagattcttgaactcgatgtagtagcgcgtgttgagcgtcttcagtccggtgtcgacacggttctggaagacggtcagcagttcggccttcgtcagctctccggcgtgcatgccgccttcggagacgacgcggaagttctcggtgtcgccgctcgtgagcacggcgaggttgtggcggtcgaggatgagtttgtcgagcaagtcgcggatattcggcagttcggcgaagtcgattttcatgttgtctctcggcgtgagatgaagagcggcgtatcgtgccgcaagccgccgggttgacccttcaagcgctggggagtgcgccatccagttgaccgggggtatcgcctcggcgaccccgtgcagttcgtgatttaccccgtagggggacgaagtaaattcgttactgcggggcaactctagcgccagcttttcggcttgtcaacacccttcctcgtgtcgggcgggcggctcagccgggccatcttccgctcgccccggaacagcctgtcgcgcagcatcttctcgctgacgtgcgggcagtggcgcttgatctgctcgaacgtcatctcgtccccgtcgatggtgtacagccgcacacgcgcaacctctttcactgcgtagtcctcgtcgtcgaatttctgcttgctcatagcgcccgtccgtgcgtctcgatgtagatgtcgtgcagcatctcatgcgcgaccgccttacggaacgcgggctgctgcacgagtgcgtgtgcgaagtcgcgcgctgtcggctccttcatgccgagatgcgcggtcatgcgcagcgcttcgtcgatgatggcctgcggctcgccctcggcgtaaccgtcgtccgcaagcagcgcatggatggcctcgcgatacttcgcgtgtcgcgcgcgctgccgcagcatcgcgatgccggcgatgacattggggccaatgactagaagcaaccagtcgaaccagctcatacagacctcgcatacggacgctcttcgccttccttgggcttcggaacgtcatggagagtggacagtcctttcttgatcttggcggccatcgccttgccgaacttcgacgcatcgccgtacatgaggtcgaggtcgggatcggcgcactcggcagcgacgttgcgcagcgtgtcgagcaacatcgggagctggtgctgcgcgctgtagttctcgtggatcatcgtccacgcgccctgcgccttccaccactgcttgcgctcgtgctcgttgagcgcgacgtattggtcgatcatcgccatcgcaaggaacggcgaccagaagcacgtatcgaccggcgtgatcgagtcgcccagctcgtcgagcgcgaagtacaccgcgaacacgggcgtggtgccgatgaggtagaccggctcgtcgagcgggtctttgtaggtggcgatggtgcagccccggtacgcggccatgtgtgcgtagcggcgcttgctggcgtcagggagcggcatgcggaaactctcgttgaagtacgggtcaagggacgctgaggcgtacaagcacgcctgtttgggctcaggttgtgcagctctcatggcagtgaagttgcgctcactcatgcgccgccggcatcgcgcacgagcacgacttcgccgtcctcgccgtcaggcagacatgcagccagtacgtcggccgcgccctgcgtgtcgccgagcacgagcaactggatggcggcgcggatcgcggtctcggtctcgatggccttgcgctcggcggcgagcacgtagccagcaccgtcgcacagctcttcgagcagatgccgcaaccactgtgcagtcgtgaggtctttgcggtcgagcgtcacgccgtacttcttcaggccggcgtcggcgcgctgacggatgatcgagatgaggtcgttcgtggtctgcatgtcgctcatggtgttctccttaccagcggcgggccggggtttcttcgacgcacatgatcgtgtctgccgggaacgaatgcgtcttgccgtactcgtcggtaacggcgatccagccctcggagcgttcgcagtgcttgtagtggttgaacgtcatcgtctggccgtcgcgaaacttgatcgtgcatgtcgccatgtcagaactccttgtggaaatctttctcggcccggatgagagccgaaaccttggggccgaactttttcggcgtgtcgagcaggatgtcggctgcgcccatcgcgatctgcggcgacacgaaatagccttggatcggatgcagcacttcgccgaagtcgtcgacgatgtagtacgcgagatggatgccgacgccatcgagcacgattagcgggccgccgtcgctgcgcacgtcttcgctgtgcagctcggcgatgaacacgtcgcggtacggttggatgcgcttgaacttcatgcggttttgtccttcaggtggtcgagctgccagccggcttcgattgcagcgaacagccgcagctcgctcgcgtcttcggtgtcgagccgcaggaactcgatgaaactgtcgatcatctgcggcgtcatcggtcgcttgtcgtagaacctgcggtacgcgctttgcggaatcatgtcccacaccgggcacaggtcgacgatgcgcttgccttcctcgcgaagatggcggcgcatgatgtcgcgcaccgtcttcgggttcttcttgaccgtgatctttcggccggtcgacggacggaaactcatagcccgatgtcctccgcttcttccttctcgtgcatgcgcagccacggcagctcgacgcgcagcatcgggaacggcccgatccagccgagcacgttgccgtactgttgcgcccagccgtattggtcgtaccacgcgccgcgccgccagatgcacacgcgcatctccttgaagtgcggcgactggcccggccacggttgcagccacaccgcgtagtagccgacctgcgtcggatcgtcgagcgattccatgtcggcgagcgcgagagggccgtgccagccgtacacgatcatctcctttcgcgcagggtggcgctgctcgtgccattgcgccttgtcgtcgaggcggaagagctggtacgcgcgcctgtccgcgttcgccgccgggtactcgcacacttcgacgacgtagaagcccggctcgacgggatcgtcgagcacttcgagttggatggtcattcttccggtgcctcgacgttcgagcgcaaggggcgcaggcgcggcagcgggccgatccagccgtggacttctcccctgaagtattggtcgctgttgaggtagcaccagcggccgttgaaccacatgaggaagatgtcgacgaccagcccgcgaccgtgcgggtcgtctacgcgacatgcgtagacgcccgtgtcctgcggcagtccgatttcttcgtattgaaccttcatccgaacagcagccttgcgacaccgatcactgcgccgatggcgagcagcgctgcgcatgtccagatgacgacgatgacgaccgtcaggaaccgcttcatcggctcagccctcttcgttggcggagtgagcctcgcacttcgtcacgagcagcatgaagtgctcctgcgggagcccgagcaggttgtgcgaatcgagcgtggcgagcagttccttcagcttggccttgccgtggtgccgggcgaacagcagcgtgtagtggcgcagcagctcgcgcatggtgtcctgctcgcgacgcacgcgcgccgcgtcccacgcaccgccgcgttcctgcttcagcgcgtcgacctcgcgtgtgcgcacgcctagcagcgacgacagctcgcggttcttgtccgacagcttcgagacttcggtcgtcgcggtattggcgatctgctggtagttcagcatgtgcttgttgatcgagcggatcgcacgcagcgcgaggcccacgtcgtcgatgtgctcgtagtgcgcgcccatgttgcgccagccgggcaccttgcgatccagctcgcggtagatgacgttgagctgccgctcggcgttggcttcgcggaaatccatcatcgcctcggccgcagcgtgcgcctgctcgccgacactacgcagcgcctcgctcgcgtccttcgtgtccagccgcagctcgacctcgacggtcttgcgcgcattgccttcgtcgtctgccggccgccacgttgcgagccacgtcgcatggtcgcggtaggtgaacttggtgcggtggccgtcgccgtcgcgctccatcgtcacgtagtagtccgtgctgtcctgcttgcggcgcgcgtcgatcacggtgtaggtgccgcccgagatgacggagaagtagcgctcgccagcggccggcggctgctcactgccgtcgaacggcacgttctcgatgaagtcgcggaacagcgattcgatgaggccgtagcccatgccgagttcgggcggcatgccgacgcgacgctcgcgcgcaggcttgaacgacacgtcatgcagctcggcggccatctgcgcatacggactgcccggcacagcgccggcagtcgtcggtgcgaacaggtcgttccacgcgctcgccgtggtgaacatccattcgtactcgccgccgcgcccgttgtcgacgcgcagcatgcgcacatgcgagtggccctcgcactcgtgcgtgctcacgaccatgaagaagcgcgccgggcggttgcgatcctgccagtaggtgccgaccttcggcgcgaactcgtagtccgggtggccgaccgtcactgcacgcgcttccttgcggtcgctcgcagcgcccttggtcgtctgcgtgctgcccttcgagaagtcgcgacgcatgatgcgctcgatgaggctcggcgtgcccttcattgcctcggcgatggcgtccgggctgaagtcgatggtgttgatgatgtggatttcgggcgcgctcgggctctcggcgaacgacggcgcaggcaccttgccgttgtgcgcattgaagaagaactcgtgctggccgacgaacgtgttgcgaatccagcggtgcatgcgctgcgcttccgcgcgctggatgtcgttctggccgacgatgccgccggtagcgtgcatgtcgcgcactatgccgttgtcgtcgatgcacgcggcgaccgacacgatcatcggggtggtagcgtcgttggtgaactgcttttcggtacgacgagacattttcggcgtttcctcggttgggttaggtggtgctgacgtgaccggcggcctcgcggtcaagttgtaggtctgcgatgtcacgcagcgacgagggccagtcgtcgagcggcacgagtccttcctcgtgcatgatgatctggtcgggcgtcaggccgcacaggtagtacgccttcgcgagcgacatgccggcgatgagccggtagcgcatagcagcgcggccgtgcttgaaggattcgacttgcgcccgcgtcacttcgcctgtgcctcggcacaaccggcacttcgtccccggcaagttgtcgtcgtgtcctgcgtcggggccgaacatctcgttgaactcgatcatgtcgtgccgcccttcgcagcgcgggcagacggtcttgtcgcggagccaacgccacgccgcgcgcaccttcatccgcagggcggtacttactgcgcgaccgagcagggcggtagcggtgcgcagacgagacaaagggggtaccggagcattccgagaagccgcaagcctgcggcccaacattttcgcttcttcgatttcgcggcgcgtgtgtcgcatggcgtcggtcactccatccgggtgacagtgagaaacgcgaacatggcgtcgttgctggcgctcatgtaggtgccgcgctccatcttgaaccgcttcgacttgtgctcggccacaccgcgcaccttggcgatgccgccgctcaggatcgagttctgctgcttgaagtatttctgcgcctcgttgttgatcgcggcgatgttgccgttgtcgagcgggatgcgctggcagcgcgcgtgcgactcgccgatgtcgagcttgctgagctggtcgttgagcgagcccggcaggaagaccaaccgaggcttctcggcgatgcgcacgcgcgggttggcgatgtcgctcttcttgatcttcgagcccgacttcttgcggctcttcttcgcaggcgcggcgctgctgttcgtggtggcggatgccattaggtgatgcctcctgttccggggaagtaagcggacaagaaacatactactgcgcgcacccggggtcgtgtcaacccgggcgttctcggtcatgaccagctcgcgcgccgggccagcgccgcacaacgatccggctgggttgccgaagcgggcgcaatttcggaaccggctaggtcggcgaagcgagagcgcaaacggaaccggctggctttgcgaagcgggccgaattttggaacgggctgggtatccgaagcggggacgtttttggaattgcacccttacatgcacgcgcacacagatatgcacgcgggcacgtatgcgcgctcgcctgcgaacgcgctcgcgttctaagtcacgcgggcgcgcggcgcgtgcgggcgcgtcaaggttccgcgcgctgcgcgttgcgcgcggttccttcatccgggcgcgcttgccgccttccgcgcttcctgaatgcaaagtaaacggactactgcgcgcagtaaaaaacatcttgcgcggcgcgcgaaaccgtgtagcctacgcataccggcaacgtcgccggcatcgcaaagggtcgcaaacatggcacgcatgaaccgttccgaattttccgcccatgccgcgcttgccgcgtcgcgtggcgcgtccgctgcgcgcaaggtcgaaaccgcgcgcaaggtccagacgttgcacgatttgctcgcgcgtcttcccttccttttcgccgtcgccgttgccgcctttgtcgcggtcgcggccgtcgccgtttccatcgtctaagggaatcacacaatgcgccgctatcttttcgtttcatccgctacgcttcccgtcgtcgcctacgcggaaagcaaagacgcgatgcgcgcatacgtgcgcgacctgctagggattccgtacggtttcccgctgccgcgccatgccgtttgcagcatcgcttaacaattcactagacaaaggagattcaccatgcaacgcattagcctttcgcaagccttcgcacagtggcaagagctggccgcagacattccgcaagacgatgcgcccatgctggcggaatcgtggaacgattacacggattcgctttgcaaggatggcgcattgtgcgacctgcaataccactacgcgcccgcatacgatgaagagatgcccggcgacggttcgcgcttcgacccgctgagcgatgatcgcgaattcatcctagacgcgctaggcgtcaccatgcgcgcaacgcgcaaggatggaccgcgcgaaggatgggacgcgagcgcgtcacactggcgcgtcacgctgcgccgcgaccgcgcgagcatgacaacggattacagcatgggcgcggcgcatacgggctcgcctgagctggcggacgtgctgaattgtctaatgcgcgatgcggaatgcggcgcgcagtctttcgaggatttttgcgcggaccttggatatgacacggattcgcgcagcgcggaaaagacgtggcgcgcgtgcaaggtgacggccgtcgggctcgcgcggcttttcagcgatggcatgctgcgcgacctgcgcgaattgttcgaggatttttgaccatgagcgagctagacattagcgcggttgtcgccggcatgcgcgacccttggaattactcggcgagcgttgcggaacgcgggcaggatgccggccgcatgacgtgggaagccgcatgcgaggatgcgcgcggcttgttcggcgagcatttcgaccgcgccgcgttcgatgagtatttttcgcatttcggcgcgtgggatgatgaagagctggccgcgcatacggatgaagaatgcgccgcgcttatgctgcaattcatcgccggcgacatgcgcgaggctgatttttccagctatgcggacatcgaaggcggcgcggaaccgttcacggatgaatggtggccgcagtatgaaaaagcgagcgaggccggaaccgtcgccggccgtttctttcgcgacgctggcggcgttttttactacattggagaatgaaacatgcaaagcaaatgggcaaagacaaccgcgcagcgcatcgcatccggcgagctggcggaatccatcatccgcaaggcgcgcgcgttgctgcgcgatgccgtgaatgctgaagagtatttcaagcgcgaaccgtcgccgtctgctaccgctgcggaagcgtgggagctggtggagatgattagcacgcatgcgccgcgcgtcacggatgcgcaagcgcgcaagggcgcggaatggctgcgccgccttgtctacacgtcgcgcggcacggtgcgccgcacggaagccgcgcagcaattcagcgatgcggacctgcgcgttttgcaggcttgcatcgcgcgcccggccttccgtctggtggagctggaaccgcacagcgacggccgatacctgcgcgaccttgcgcccgtctatcgctgcatcggcgacaacggcgaatccttcgattacacggcgagcgcgtggcagtctggcggcgcgttcgcaatcctgcgccacgcttaacccttcccatccgtgacaagcccggagaatctgaaaatgtacagcatcgcaaacaacgcaaagcccgccattctgacgcgcacggaatcgcgcatccaatcgcagcgcgacaagcgaacgcgcgacacggaagcgcgccgcgcaaagtatcggcgcaacgctgcgcgctatctggccgcgtctttctggcgcggctcgcgcgacatcgccgatttttttaagggtcgcggattcgaccatgcgacgttgcaggatgcggaaaacgattgcatggataacgtcgatttttcttatctgtattcccgcgactatgcgcgcgagctggaaaaggaatacggcgacgacgcgcgcgaattgttcgcgtacctttgcccggatgcgccgctgagcgtgtaccgtgagcaaatcgccgacgacgtgacgcgcgcggtcgcagactcgcggcgcgcggattatgcgttgcagtttttcgactggtgccgcgatgcggtcgaggatgcggccgattcttccgggcttgtctggtgctggctggacaaggccggcaagcctacggatcaggaatacgatgcgcacgcggtaggcttcgcatgctcgcgccgcatgtacctttcgcgcaatgcggaatggtggccggaaaaatggtgggcgaaaggtgaaagcgtttggagcgattacgcgagcaatcgcgaacgcatggacgcggccgatgacgtgctgaacgaatttctcggtgagcatctggaaagcgaaggcgcggaccttgaatcgttcgatgagcgcggttcgcgctatgcggatgatgattattggccggaatacttcagcgactacagcgaagcgcgcgagcaatgggaaaacgacaaagcaaagatgcgcgcgcgtctgcgcgagatgatcgcgaaccgtgcgccgctggaattgcgcgccgcgcttgtcgcgagcgtgtacggcgagcccggccgcgcggccgatgaatccgaagattgaaaggga

SEQ ID NO: 3 - DNA, 55335 bp, unidentified
  source 1..55335: mol_type = genomic DNA
gggggcgctgacctcggtgctcgcgcatttttcggaattttcgcggtttcgtctcctttggacccccgggcggccccgaatttccgaatttattccccgaataaacgcgaatttcctgtgacagtagtgacagtgacgtttttgggtactgtcacaaattcggccccccaagaaatccgctcaaatcaacgatttacgggcgcgaatttactgcgagtttaggctcagtgacactgtgacagtgacttccaatcctttacggcggaaagaaaagttctgcctgccaagaaaaaattctcgcgtatgagagaaggtactgtcactactgtcactactgtcacaagatagggaaaaaggtatgtagatcaagcacttgaatttgtgacagtaccttgtgacagtgaccgatttgcgcctcggagagcatggaaaaccgggtactgtcacaagaatcggcctttttccgaatttccgcccatacggttgcaattttttccgtatgtgacagtgaaaagaattcggaattaatttaatcggagccgctgcggggcgtcgtgcggaaattcggaaattccgggcaataaaaagccccgggggatgagcccggggccggcactgcggaaattccgccgaattaaatcgcgctcttcggcgctccatcgcctacacgcacgtcctcgacgttcgagccgttgtcgcccgcgcccggcggaagcggatcgctctcgtagcggttcgcgtcggtgttgttttcgtcgacggtcgcgttcggcaccatgccctgcggcttcgacgcgccgaagaagtcgccggtctcgcgcgctgtgacctgcaagtcaccgtgcatcgtgatttcgaccgagcggccgggtgcatcgagcactgcatgcaccacgccgttgccgtcgaccaactcgaccgccttgttgccgttgacgtgcgtgaacttcacggtagtcgtcatgtcgtttctcctgtgctcgggattgagcgtcttcgatcatacgctcgcaggcatgaaaaagcccggttgcccgggcttcttcgatcacaccttcagcgacgtgatttctatgtagtcgtcgatccacgcttgaaggttcggccgcaccaccacgtcaggcgagcgtgaccaataccgggcctgctttccgttcgcgccgcgcgcgcggcccacgtacacgaagcccttcgaggtcaggaagttcgacagcttcggcccgtacggcacaccgacgctgttgtccatcgccatgtcgcgcagcttgccgacgttgagcagcaggtggctcacttccgggtcgcgcgactccgcgatcatctcttcgatttcgtcttcgtcgtcgccgcgcgcgaggtcgatcatgcgcgacttcgcatcggtcatgggcgcatggccgtccgggtcgaactcgggatgcagcgggtagtcttccagccactcgcggatcgcacccgggtgataggcgattgcgttgaagatgtcgtcgtagtgatccgggtggcgctcgcggaacttctcgatcatctgcttcgtctggaagtgcgtcgagatgacgaagtagcggcggtcagcgtcgtagaccggcagcgcgtcgctgtggttggtcaggatgatggtcgaggtcacattcggcacgttgtacgagtcgcggtgcatgcggcgaatcgaaaccacgtcgttcgtgatgaagggcttcagcttatccatcaccgcgtagcgcgacgtgccgtggatgcgcgcttcttccagcaccacgaccttgcgcgactcgaagaacgacgtgtacttctcttcgagcgcctgtgcgttcacggtctcgacgttgttgcgcgacatgatcgccatgagcatttcgccgacgaagcccttgcctgcgccgtccacgccctgcatcacgaccgcccaacggattttcctgtccatgcgcttgatcgtgtacgccagccacgacagcaggatttcgcgctcgcgttcgaccgggtacgaaatctcgaagtggcgcttcaccgcctcgaccgcgcgccgggccttgctggtcaacttgtccggcaccggcacgatgtcctcggcgttgaacttgttcgcgtgcttctggccgtcccactcgacgatgcggtctgcgcccggcaggtagacgtagccgctgacgacgggaatctggtacacgttcaacgcgagcgcggcggcctgctgctcaggcacggcttccatgttcgcgcggtccttcttcgtcagcaggaagcggttgttgcgtgcgttgaatgcgcgctcgctcagtgcgagacggctgtccatgtagtagaactcttcctcggcgtcgacgtacaccacgtcgttgcaccaatgcggcagctccttgtagttgaagtcggaattgcggaagccttcgttgatcgccttgcggatcatcgcgatgggaaccttcttccccagctccgcaacgcgctccttgatcgcgccggccaacagctcgacttggaactcgttctccaacatgcggccccacttcgccgcgagcgggccaagcagctccatctccgaagtcgtctcggcgaccttgcgcttgatcttctcgaactgctcctgcgagtgctcctgccgatgctccttcgccatcttgataagcgaggcggcggtcgtcaggttgcgacccatgtcgtcgtggaacgagttccacttgaactccaactcgtccgggtcgtagttgtgcgcgggctcggaccactcgtgccaaagctgcaagccttcttcgttgccgtcgaattggtgatgcagcgccatgccgaccttcaaccactgctcgtagtcgtcggcacccggcacccattgcagcacttcgcggagctggtcttcggtcaggttttccagcgggcgcttgtattccagcagcgcgttgtcgttctcgtcgtcgctgctgcgcgattcggtcggcgcgttgtgcttcttcaacgtccagccgcgacgctgcgcttcgagcttgaacaccgagaacagttcgtcgatgtgctcggtcgtgatttccggcagcatgtcggccggcacgctcagcgggtttagctccttgcccgaagtccacttgtacggcttcttggtgtcggggtggatgccgatgccgacgaactgttggccgtccgcgagcacttcgatggcctgctcatgaccttcggtgtcgaggaacgtgatcttacgcttctggaacggaatgtcggtgcgatatacgagcaacgtcttcggcgcacggccgactcgcgtcatcgtcttgccgatgatttcttccgtgtgctcagccatgagcgcggccatttcgtcatcggtgatgtcgatgtcgaccgcaggcgtgtgcttcgtgtggaagccgatgttgccctgcttgtagttgccattcgcccacttgcgaatctgcttctcgtccgcgcggattttctgccactgcggttcgattgggcctttccttcctgccgggatcggcaagatggagtacccgttttccagcaattgcgcgccgtacttacggagcacgctggtgatcggtcgtccagcagccataggtcactccgcgatgtcgtcgctaacaaggtcttcgaggttgaagccgatcttgcggttgaaatccttgtgcaagatggtcgccttgtcgcgcggcacaccgccgaggcgctgccaacgcgagacagtggtctcgtgccagttgtacttctcgcaaattgcgttgagccgaccgtacggcgggtcgagcatgagggcgatgcgccgaagcagatagcgcactcgcgcgtctgcgctgtccagtgaatcaagagtagggtctcggcgcatgaattcctcgcagacgttgggatttaaggggtctgctaagtcggtgagcatgcctattgacttagcatcgggacaggcgcatagtgcgctcgccgggcaggaattgcaatccacccgtcactcccgaaaccaacctagctaggagatacaaccgatgtcgaagatcaacgcgaagaagctcgccgaagccatcaccctcatcatcgaagcagtcggcggcggtgccgccaacgagtccgaggatgcgggcggcgaagaggaagcgccgaagaagggtcgcggccgtccggccggcagcaccaacaaggccaaggccgagaccaagcccgccgccaagggcaaggccaaggcgaaggacgaggacgaggacgaggacgacggtctcggcgacgacgacgatgccggcgacgacgatgacgacctcggtctcggcggcgacgacgaagaagtgacgcaggaagatgtcgtcaatgcgttcaaggcgctgaaggcgagcaagggcatcgacaagtgccgcgaagtgctcgccaagctggacgagagcaacgtgctcaacatcccgccgaagaagtacgccgaggcgctgaaggaaatcaaccgcgccgcgtcgaagaagtaactcggcctgcacgtcacacgaaacgcccgggttcgctcgggcgtttctttcggagaggaacacatgcccggttcgcacgcccgcttcgcaccatcgtcggcgcatcgcatctacgattgcccggcgagcctgttgctcaacgagaacgagcccgaccgcgaaatctacgaagcggccgagggcaccgttgcacaccacatcgcggaaatctgcgcacgcgcgcgccgcgagccggaagagtttctaggaatgacgttcgacagcggcgacctcgacgccgactacgacgaagagcagcattcctcgaaaggcttcgcaatcaccgtcgacgacgagatggtgcagggagtcggggcgtacctcgaccgcatcatgggcctgccgggcgaccactacgtcgagacgcgcgtcaacatctccccgtggtgcccgatccccgatcaattcggcacctgcgaccacgcagccgcgtcgcacaagaagctcatcatcaccgacctgaagtacggccgcgtgcaggtcgatgcgccgcagaacaagcagctcgtgatgtacgcgctcggcttcatcaacgagtacgactggctgtacgacttcgatgaggtcatcatccgcattgcgcaaccgcgcctcgatcacttcgacgtgtggatcaccagcaaggccgaactgctcgctatcggcgagaagatcaaagagcgcttcgcgcttgcgttgaagccgaatccgccgttcggcccgagcgagaaggcgtgccgcttctgcaaggtcaacttcaagtgccgcgcgaaccacgacttcctgtaccacgagcgcatcatgctgctcgatgacgacgacgagttcgtcgagcctgacctcatgctcatgagcgacgacgaaatcgctgcgctgtggctgcgcaagggcatgtacgagaaccgcatgcgcgcggtcgaagactacctgcacaagaaggtcgcggacggcgacttcgtgccgggcctgaagaccgtggcgggccgcagctcgcgctacttcaccagcgaaatcgacgccgagctgctgctgctggaagccggcgtgcccgagtctaagctgtactccaaacccgaattcgtgtcgcctgcgcaggctgaaaagctggtgcgcggcgaggcgaagaagaaattgcaggacttcatcaagtcgaagcccggcaaaccctgtctggtctcttccgacgacaaacggaaagacctgaccgtccagtcgctcgaactgctcgacgactgacgcaaccgttgtacgaatgcgcgaaagcgaactacgaacgtcgaatgacgaaggagaaatcgaaatggcgaagaagaaagttggtgatctggtcgacaagggcaatgggcgttttctgctgaagaacgtgcgcctgagcttcccgtacttgttcgagcccgacgagcaggaagacgacaacggcaacaagaagaagtcgtaccgcgtcaccctgctgctcccgaaggcgacgcacaagcccgtcgcgcagaagctctcccgtctcatctccgagatgtgcgaggaagagtacggcagcccgaagctggcggccgaccgcaagttcctgcgcgatggtgacgagtcggatgtcgaagatcatcacggctgctggacggtgacggttcgcgagacccggaagccgatcctcgtcgaccgtgatcgtcagcccaccgaggaagacgacgagctgctgtacagcggcgcgtgggccaacgtggtgatccgcccgtgggctcagaacggcaagtccatgaagaagaagaacaagtacggcaagcgcatcaatgccggcttcgacatcgtgcagttcgtcgaccacgacgacaacctcgcgggcaacgctcgcccggatgtcgacgaggttctggatgagctggacgacgacttcgcggatgacgacgacaacagcaccagccgcagcaagtccaagagcaagtcgaagggtcgttctcgcgacgaggacgatgacgacgacgggctcggcgacgacgatgacgacgaccgcagctcgcgccgcagccgtccgtcgaagagcaagaccagcagcaagagccgtcgctcgcgcgacgacgatgacgatgacggcgacgaggacgatgacgacctcggcatctaaaatcgggcatcggtaagcggtacctacggtcgcccgggcactccccgggcggctgtttttcagggatacggtatggacaagctgcatcacgacttcgagaccttcagcaagtgcgacctgaagaagcacggcttggcgcgctatgctcgcgacaagtcgaccgaagtgctgttcctgtggtacgcattcaacgacgaggaacccgaagtgtggttccccgcgacggagccgatgccgaagcgcctgcgccgcgcgctcaaagacccgaacgtgcagaagtgcgcgcacaacgctcagttcgagcgcgcgatttggctgcacgtcctcggcatcgacatcccggtcgagcagttctattgctcgatggcgcacgcattctggctctcgctgcccggcaacctcgacgaactctcgggcgtgcttcgcctcggcgagaacgcgaagatgaaggaaggcaagtcgctcgtgaagttcttctgcgggccgcgcaagccgacgaagaccaagcagtacacgcgcaacaccgcgcagaccgatccggcgaagtggaagacgttcgtcgagtacggccgccgcgacgtgatcgccgagcgcgcggcaggtcgcaagctctcgctcttcccgatgagcgatttcgagcgcaacctgtggtacatcgaccagcacatcaacgaacgcggcattccgttcgacaaggaattcgtcgagaccgcgctgcgcgtcatcgcgaaggagaagaagcgcctgctgggcgagatgagccgcatcaccggcctgagcaatcccggcagcggcgcacagttgctcccgtggctgcgcgagcgcggctacccgttcaccaacctcaaatccgcctcgatcaagaaggcacgcgaggattgggactggaacatgaccgatgaggcgaacgcggttctcgccttgcacgcggaagcggcgcgttcgtctgtcacgaagttgcagaagatgctcgacatcgaagtcgacggagtgctgtgctacacgatgcagttcgcaggcgcggggcgcacggcgcgctgggccggtcgcgcagtgcaggtgcaaaatttgccccgccccctccgcgaactagaagagcaaggggcactgctcatggcgcgcgatgcgatcatgcgcgaagacatcgagttccttcgcctgctggtgtcgtcgccgatgggcgcgattgcatcgtgcatccgcaccgcgatcaaagcgccgcccggctacgagtatgcaacgtgcgacttggcctcgattgagtccgtcgtcattgcatggctgtcgggctgcgacaagttgatcgaggtctttcagaagaacctcgacgtgtacaaggtgttcgcgtcgaagatgtacaaggtcgactacgagcaggtcgagaagtggatgcgtcaacacgcgaagcccggcgtgctcggcgcaggcttccgcctcagcggcggcatggagttgggcgagtacccggaagtcatcaagaccggcctgtggggctacgcggagaacatgggcatcgagatgtcgcagaaggatgctgcggccgtcgtgaaattcttccgcgaggaatacaccgaaatcgtcgagctgtggtacgagctggaacgcgccgtcgcgaaggtgatgaacacgaaggagccggtgcgcgttggtccgatcctcatggacgtgaagggaccgttcctgcgcatgcgtctgccgtccggtcgctacctgcactacctgcggccgaagatgatctggaagaagatcaaggtcggcatcgacaagaagaccggcaagccgaaatacaagtcgaagaagggcttcacctacgaaggctacaacacgaagaagaagtggacgcgcatcgactcgcacggcggcaagatcgtcgagaacttggtgcaggcaatcgcacgcgagctgctggccgccggtctgctgcgcgcttggaaggccgggctcgatgtgcgcatgcacgttcacgacgaaatcgttgcgctggtcaagcgcaagctgtcggacatctcggccgcgacgctcgaagagcagatggtcaagaagccgaagtggtggggcgaagacgttccgatccgtgcgaaggctgacgtagtggagtgctatcagaaatgagctggctgaccgattggcgcaacgtaatcaacggcaagccgccgcgcggcgacatcctgccgaccgacaagcatcgcgtcgaaaaggacgtggagcagaagtggtgcgccgttgcgaagcggcacggatggaaggcatacaagttctcgtcgcccggcaacagcagcgttcccgaccgcatgttcatccgcaacggcttcgtcttcttcatcgagttcaagcgccccggcagcaaggcaaccgacaatcaactcgaagagcacaaggagctgcggcgcaagggcatgatcgtgtgggtcatcgactacttcgataaagaattcgccgagtggatttttgaatgaaacaactactgaagcgctccgacctcgacgagtttcaaatcgctgccggcctgttcctcgaacgggtcggcagttgcgcgttgtggatcgacatgggcctcggcaagaccgtggtcgtgctcacgcatgtttcggacaaggtgttctccggcgagtggagccgcgtgctggtcgtaggcccgccgctggtcatctccgatacgtggtcgaccgaggtcaagaattgggagcacacccgcttcctcgactatcaggaactcgacggcgacagcgagcacatgcgcatgcagttgcagcggccgtgcgaggtcgacggcatctcggtgcataaactcgggcgtctcgcggcgctgttcaagcgaggcgacacggtgccgtgggacgcggttgtgttcgacgagtcgagcatgttccgcaacaagtcgtcgaagcgctggaagtacggcgtgcgcctgacgtggggccagccgaacgacgtgatcgagctgacaggtacgccgagcccgaacggcctgcatcaagtctggtcgcagattgcgatgatcgacggcggcgagcggctgggcttgacgtacaagaagttcctgttccgctggttcaagcaggagttcatgggccgcaaagtgattccgaagtcgcacgcgatggcgtcgatcacgaagaagctgagcgacatcgtgtacaccttgcgcgaagaggattacgtcaagttgccgccgctccgctctacgcctgtgccgatcatcctgccgccggatgtgatggctcgctatcaggaattcgagcgcacgtctgtgctgaagtggggcgaagagcaagacccggcagtgcgtgctctatcggaaggcgcgctgtacggaaagctgttgcaatttgcgtgcggtcgcatctatacggattcagagacgaaagagttcgtcgacatacacgacaagaagatcgagcgcctgaaggaaatcgtcgagttcagcgacggctcgccgatcctcgtggcacgtacgtggcagcactcgcgtgatcggctgcgcgatgagttcccgggcatccgctcgttgaagacgaagcgcgacctcgacgcatggaacgcgggcgacatcgagatagccgagacacaccctgcgagcatcggtcacggcacgaacatccagaagggcggcaacaacctcatctggtacgaccacacgcccgacctcgaactctacatgcagttgcgcaaacgactgcaccgacgcggccagacccgaagccacgtcaacatgatgcacctgacagcagtaggcactatcgaagaggatttgacacgcgagctggtcaagaaagaaattacccaagacgccctgagagaacccatgcggcgacgagtcgcagacgtacagagagaactagccaatggccgcacctaagatcgactacgaagaagagtttttcgacggcatgaccgtgccgcgtctggcgcagttgttccgcctcgaccgccgcactgttaccgagaagctgcgtccgctgcgaccgaccggcgaccggcgcggcgcaccgacgtatcacatcgtcgacgctgcaccgtacctcgtggagcccatcgtcgacatcgccaagtacctcgcggaagtcggccccggcgacctgcccgcaccgctgcaagcgcagtattggaacgcgcagaacagcaagttgaagtacaaggaacagtcgggcgacttgtggcgcacgcaacaggtgctcgaagtgctgaccggcgtgttccgctcgctcacgcaatcgcttcgcctgctggccgaccgcatcgaagcgcagaccgggctcacgccggagcagcgcgcgatcatcgagcgcgaagtgtcagacaaggccatcgacatgctgcgcaagcgccttgtcgaagacttcgagatttacgtcggcatcaaggacaaggaacagctcgccgacatcaagctcgacgacatcggcctcgacgaagaggacgaagaagatgtctgacggcagctttttcaacgacctcggcgagctggtcacgttcgttgccgatagcgttctggttccgccggagcgcttgaccgtttctcaggccgcagcaaagtaccgctacctcgacaacgaaggctcgttcgtcggcgagtgggacaacaacgaaacgccgtacctcgtcgagccgatggacgtgctcacgagtcgcgagttcgagtcgtgcatcttcatcggcccggcgcagggcggcaagaccgaaatcatcctcaattggatcgcatacaccgcgaagtgcgacccggccgacttcttcctcatccagaccgcgcgcgacaccgcacgcgacttctcgtatcgccgcatcgacaagatgcaccgcgacagcaaggagctgggcgcgatgctgcgtccgggcagcgacaacgacaacatcttcgacaagttctaccgcaacggcatgatgctgacgctgggctggccgacgatcaaccagctctcaggcaagccggtgccgcgcgtcgcgctgaccgactatgaccgcatgccgcaggacgtggagaagaacggcccgccgttcccgctcgctcgtaagcgtacgacgaccttcggctcgttcggcatgacgctggccgagtcgtcgccgtcgttcgacgtgaaagacccgaaatggaaggcaccgcacccggactcgcatatgttcccgccgtgcgatgggatcggcggcctgtacaacgaaggcgaccgccgttgcttctactggcagtgccctcactgcggcgagtggtttgagccgaagttctcgctgctgaagtgggacatcaagaaccccgacccgttcgaggctgcgatgtcgacgatgatggcgtgcccgcgtaacggttgcgtcatcgagccgaagcacaagtacgagatgaatcgacgcggcgtgtggctgcgagaaggccagcgtattgatcgcgacggcaacaagctcggcgtcggcgttcgctcacgtagcgcatcgttctggctgaaaggcccggcggcgcgcttcattacatggcagaccctcgtcgagcgattcctgcttgcgcaccagacgctcgaacgcacgggcgaaaccaaggcgctgaaggccacgatcaacaccgatcaaggcgaagcgttctggccgctcaacgcgaaggactcgaaccgcctgccggaagacctgcaatcgaaggcgatccagtgggccgacaagaaggtgccgtacggcgtgcgcttcctgctcgggactgtcgacgtgcagaagagccgcttcgtcgtgcaggtcttcggcgtcggcccgagcgataacggcgtcaacttcgacctgtacctaatcgaccgattcgacattcagaagtcgaagcgcaaggacgaggctggcgacacactatgggtcaagccgtatgccgtgcaggaagattgggacttgattaccgagcaggtcgtcgagaaggaatacgagctggaagacggcagtggcttcatgtcgatcaagatgaccggcatcgactccggcggtaagtcaggctcgacgacgcgcgcatacaactactggcgctcgatgcgcgacaacggcaacggcggtcgcgtgctgctcatcaagggcgagccgaagctcggtgcgccgcgtgccgaaatcgacttccccgactcggatcgcaaggatcgttcggccggtgcgcgcggtgaaatcccggtgctgttcctcaactcgaacgtgctgaaggacatgctgctcggcatggtcgactacgacgagaagacgacgctcggcggcaggcacttcacgaacaagtggacgccggaagttgtgtacgccgaactcactgtcgagttccgcgacgaccgtggtcgttggcagaatccggctaagcgacgcaacgaagcgtgggacttgggctactactgcctcggcctgtgcgtgatcttgaaggtcgaaggattcgattgggacgcgcctgagtcgtggttcgcggagtggagtaacaactctcttgtgcgccgtgtggatcaggaaaaacggtttgcgtcaagccccactacggattatggtttcgccaagttcgggaaatccttgggatgacaaatggcgaccctagagcagttgcaagcatggctggcggaagcgcaaaccgcctaccatagcgtcatgatcggcggcggcgtgaccgtcgtcgtcgaccagaacggggagcgggtcgagtacagccgggccaacgcaaccggcctcgccaaatacatagccactttgcaagcgcagatcaattccctattgggggtcgcagtaaccggcggcccccttcgtccgttcttctgagggtaaaacgacatggcaaaagcactcactgtcgtgcgctctcccgagggcgacgaagcgttcaacagcaccggcaaagagtcggcgttcggcggtgcgtacgaaggtgcgtcgcgactcaatcggcagaccgcgttgtggagcgcgccgtcgctgccggccgacatggagatttcgccggacaaggttcggctcgatgcgcgcactcgcgaactcattcgcaacgatggctacatccaaggtgctctcgacacgagttcggactccatcgtcggcggtcagtaccttctcaacgcgcgccccgattgggagacgctgggcctgagcgaagagtgggctgaagagttccagctcatcgccgagcgcaagttcatgctgtacgccgagtctccgatgaactggatcgacgcctcgcgcaagaacggtctgaccggcctcgtgcgcatggcgctcgcgcagtctttcatgtcgggcgaagcgctcgccgctgcggagtggctgtcgaaggcaggccgtccgtacaagaccgcgatcaacatgatcgaccccgaccgcctgagcaacccgaacgacaacagcgatacggcgtacatgcgtcgcggcgtcgaaatcgacaagttcggcgcggccgaggcgtaccacatccgcgacgcgcacccgatggagtcgtactacgaccgcttcggcgcgaagtggacgcgcgtgccggcgttcaagccgtggggccgtccgcagatcatccacatcgccgaagtgctgcgcccgggccagacgcgcggcgtatcgaagatggtcgcggtgctgaaagaaatgcgcatgacgaaggtctacaaggacatcgttctgcaaaacgccgtcgtcaatgcgaccttcgctgctgcaatcgaatcggagctgccgcgcgagctggtgttctcgcagctcggtgccggcgacatgggttggttgcagaagtacatgggcgcgctggctgagtatgtcggttcggccgacaatctcgccatcgacggcgtgcgcattccgcacctgtttccgggcacgaagctcaacctgcaaaacgccggccagcccggcggcgtcggcagcggcttcgaggactcgctgctgcgccacatctgcgctgcgctgggcctgtcgtacgagcagttctcgaaggactactcgaagacgaactactcgtctgctcgcgcgtcgatgatcgagacgtggaagtacatgcagacgcgcaagaagctcgtcaccgaccgcttcgcaacgctggtctacatgctgtggctggaagaggaaatcaaccgtccgaataccgacctgccgctgccgaagggcgcggcgcacttctacgaagggatcaaccgcgaggcgtactgccgctgcgactggatcggcgcttcgcgcggccagatcgacgagctgaaggaaacgcaggctgcggtgctgcgcatcgcgtcgggcctgtcgacctacgaggaagaactcggcaagctcggcaaggattaccgcgaagtgttcacgcagcgcgctcgcgaaatgaacctcatcgaaaagaagaaactcaacttcacgctcagcaccagcaagccgggcacgcagaaagaaaccgacagccgcgcatcgaacaacgaagacgcggacgccaccgacgataccgacacggagaacgacgatgaatgaactgctcgcgatgcgcatggcgctcatcgagggattcaacggccgcccggcgttgatcgaccctcgtgatgtcgagaaggtcgcaacgctgtgcatgacgatggcgcaggcatctttcccgccgaccgccgagcagcgcgcgcaggcggatgaaagcatcaccgccgctgtcgagaaggcgttcgacgtttccttcccgcgcgaccgtgccaagccgttccttttcagcaacggccttgccttcatcccgatgcgcggcacgctcgtacatcgcaacggcgacccgtggtacggcacgcgcggctacgacgacatccgccgcgagttcgacgccgcgatggccgacccggacgtggcgggcgtcgtgttcgacatccactccggcggcggcatggtctacggcaacttcgagctggccgagcacattcgcaagggtcgcgacacgaagccgtcgctgtctgtcgtcaacgcgggtgcgatgtcgggcgcgtattcgctcggcagttccgcgaagcgcatggtctcgacgccttcgggcgacagtggcagcattggcgtgctgaccatgcacgtcgacatgagcaaggcgctcgaaaagttcggcgtcgccatctccctcatccatgccggcgagcacaaggtcgacggcaatcccttcaacccgctgcccgacaacgtgcgtgccgacatgcaggcacgtctcgacggcatgtggcagaagttcatctccgtggttgctgttaatcgcgggatgtccgaacaagcgattcgcgacacgcaagcccgtgtgtatcaggcggacgatgcggtcaagatcggcttggtcgatgcggtgatgtctccgcaagacgccatcgctaccttccgggccgaagtcttcggctctaccaccaacgataggagtgcaaccatgagcgacacgaagaagaccgacgccaccgtcgagcagaagaaggacgacgcgcaggtcgagaacaagaccgccgacaccaccgtcgacgcgggcaacaagaacgagcaggtcgatgccggcgcggcgatgcaggcgcgttgcgccgccatcaccggctgcgaggaagccaagggccgcgaaggtctggcgaaccacatcgcgttcaagaccacgatgtcggtcgacgaagcgaagtcgatgctggccgcctcgccgaagcagtcggccgccaccggcaagtcgccgctcgattccgcgatggacaacagcggcggcggtgccgacatcgccaacaacggcggcgacgaagaagagcaggcgcgcggcaacgacgacggcggcctgctgggcgcgtacaccgctgccaccggcaacaaggccgtgctgaaggtcgtcaagtaaaccgaacaccgtcgccagcctagacggaaaaaaaccggctaaaccgtcaatcacagaaggagtaacgaaatgaccaacttcggccccatcgctggctacgtggctcgtaccgacacgaacagcatccagctctacgccggggaagcggacatcgtgagcacgcagggcgcgctcgtcaccggcaccgcctacgtcggcggtcaggtgctcggccgcgtcaccgcttccggcctgttcgccaagcacgacccggccgcgaccgatggcagcgagaacgccatcgcgatcctcgcgtacgacgtggcgaccccgactgccgacaagaaggaagcgatctacgtcggcggcgtgttcaacatggaagcgctgaccttcaacgctgccaccaacaccgacgccctgaaggccgctgcgttcgatggcaccaacatcgtcgcgcagaagctctacggtgcgccgcccgccggctccggcccggtctaaccggcatcaccaacagcaagacgtttcgcaattcaactcagaaatagaaggagacaacgatggatttgttcagcactgcggaactgcgcaaggtgatcgtcgacagccggccccccgtgcagtatttcctcgaccgtctgtacaaggagcagatcaacttcacgaccgaagaaatcatgttcgacgagctgaagctcggccggcgcatggctccgttcgtggctccgaacgtgcagggtcgtgtcctgaagcgttccggcttctacaccaagtccttccgcccggcgtacgtcaagccgaaggacgcggtgactccgggccgcatgctgcgtcgcctcgcgggcgaagcactgaccggcgacatgacgcccggccagcgctggcgcgcagtggtcgccgcgtaccagctcgaccagcggaaccagattttccgccgctgggaatggctgggcgcgcaggctgcgctctacggtcaggtcacgatttcgggcgaggactacccgaccgtcaccatcgacttcggtcgcgccgccaaccacacggtcatcctgaccggcaccgcgctgtggaccgaccagaccaacagcgatcccgacgacgacctcgaagagtgggccgctcgtgtgcatgacgccgaaggtttcgtcgtcacccgcgtcacgatgggccgcctcgcgtggaaggcgttcaagaagcacccggtcatcaaggagctgctggaaacccggcgcggctcgaagtccgaagccgaaaccggcccgggcctcggcgagtcggtggagttcaagggccagatcggttcgttcaacatctacgtctacaacgacgtgtacgaggacgagaccggcacgatgcagccgatgatggacccgcgcgacgtgctgctcgaagccgaggctggcttcgacggcgtgcgggccttcggtgcgatcatggatgcggacgccgaccttcaggcgctcgacatcttcccgaagatgtggaagaacccggacccgtccgtgatctacctcatgtcgcagtcggctccgctcatgatcccgagccgtccgaactgcacgctgcgggcgcgcgtcgtcgcgtaagcgtcgtcgcacacggcaagcccggttcgccgggcttcgctgtggcaacacaactccccaaccgaaagaaggagcatcaagatggcgaagtacaagttcgtggcccgcgtggcgctgaagggcgatttcgacgccgaagacggtctcggcaccgcgttgcaggaagtgcaggcgggcaccaaggccggcaccgacgacaagaagctctacgactcgctgctggaacagggctacatcaagtccgcgaaggacgccgcgaaggaagaggacgaggctccggctgcgtcgtcgaacccgagcaccgcgccgaaggtcgagtcgaccgacgccggcaagtccagcggcggcaagcagggcgcgggcaagtaagcccggcgcgctgaagggagaacgaaatgggctggctcgaaaccaagcagaaggctcggcaaaccgtgcatagcacgtttggtctgccggcccaatttcgcccgaggtcgggcggtgctgtcgtcgacggcaccgctcggctgcactacaaggtccgcacgttcggcgacttggaccgcgaaggcttcgcgaccgtcaccgaggcagtggactacatcatcatcgacactcggattttcgtgggcgctgacgaaggcgaccgcgtgttcttcccgcaactcaaccgcgcgttcaagctcgatgtgcgcggcgaagcggaagacgacattttcatcaagtgggaagtgagcgaggtagcgccgtgacggtcgaggttggcttccgtggattggatgacgtgcgcaagcgcgtcgccggcataccggaaacggtagaccgggcatccgcgtttgcgatcaacgaagcggtcacgttcggtcaggccgagagcagccgccgcatccgcgagcaggttgcgttcaaggccagctacatcggcagctcggacgatccgaacgctcgcctgcgtgtgtcgaagaaggcgcgcgtcggcgacctcgaaggcgtcatcgccggccgcatgcgcccgacctcactcgcacagttcatgactggcgcgaagctcggcaaaggcggctacgctcgcgtcaaggtgtcggcgcacggtgcagcgcgtcgaatcccgaatgcgttcccgatgaagctgcgtcgcggtaccggcgtctacgacccggagaacgcgaacgtcggcctcgctgttcggttgcaggacgggaagctgccgggcggcatgaacaagaagcagatggtgcaggtcagcggcaatctctatctgctgtacggcccgtctgtcgatcaagtgtttcgcgatgttcgagtcgatgtgcaagcgccggtcggcgacgtgctcgaatcgagcttcctgcgcaatttcgggagattgaaccgtggctgatacgaagcgcctgctgctgctgaagagcctgtgcaactacctgctgaccgaaatcacgacggcgaacggctacaacttcgacctcgccgccgcgtatcgcggcaagaagaatttcggcaaggaagtgaagctgccggcaatcgtggtgttggagaacttcaacccggatcgtctgccggagaccatcggcggcgtcgtcggcaccaagcacaagtacgaccagatttacctcatcaacggatgggccgaaggcggcgatgtcgagcaggaagaggactcggctcatctactcatgggggacgtgaagcaagcgctcggcaagctgctggtgccgcgcaatcaaagcgggtttttcgatggtctcgcaaacacgctgtccatcgagcccggggttgttcgccctcccgacgagcaatccgagaaggcgtatttctggatgaggattcgtctggaagtcgtcgaaaaggtgggagacccgtactggattcgtgattaaccgttgtatcgacagaaggagaccgtaaatgggcagcgagaattacacccttggccgtggcgaactgcacttcgacaagttcgtcgccggcacgttcaacaagaccggcgagcgttacctcggtaacacgccggagttgaaccgcaccaccgagagcgaaaacctcgatcacttcaacagcgaccgtggtatccgcgtcaaggacaagagcatcgtgctcgaaaagaacgacagcggtacgttcatcgccgacgaaatcagcgacgagaacatcgccctgtggttcctcggcacgcagaacgtcgtggcgcagtcggcgtccgcgagcgtggtgcagaacatcccggccaaccgcgtcaagccgggcacctacatccagctcggcgagtcgaccgccaacccgaccggccatcgcaacgtgacgctgaccagcgtgaccagcgatccggttggcacgaccttcgacaacctgaccgactacacggtcgacgccgagctgggccgcctgtacatcgtgccgggcggggccatcgacgggaccgccccgctgatcgtgacctacgccacggcggcctcgacccgcacgcagatcgtggtcggcgagggcaccaccatcgagggcgcgctgcgcttcatctcgtacaacccgaccggcccgcgccgcgactactactggccctacgtgcagctccgggccgatggcgacttcgcgatgaagggcgacgaatggcagcagctttcgttcgcattcgacatcctgaagcgggacggctacgcttccgagtacatcgacggtcgtccgaccgtggcgtaaccggggtacgtcaaacgcggtcaaggccaacttagtcaagatcaagcgagccaagaccaacttcgacaggccgcctcggaacccccggggcggcctgtttcgcatcaccagccagaagaggaaagtccatgtcccttgccaacctgcaactccgcaccgcaaccgttccgtatgtcggcgcgaacgacgagtcgcacgacatcgtgctgcacggtctgagtgcgaacgccatcgccggcctcatcctgtcgcagctcagcaacatcgaagaaatcttcaacatcgtcgaggcggccggcgtcaagaagaccgaagacctcgccaacgtcaacatcgccgaagtcggccaacggcttctcgtgcagctccccgacttcatcgcgcacgtcatcgcgtactccgcacacgagcccgagcagtggagcaaggtcatgcacctgccggcacccgtgcaggtcgagtgcctgacgaaactcgcgaagctcacgttcaacgacgaagccggcttccgagaattcgtgggaaacgtggtcgcggcgctgcgaagcgcaaaaggcgtagtgccgcagactctcaaccgaaatcccgccgtcaacgcttcgccgaatggtggcttggcatccgagcagccgtctctttcctgacggctgaaggtcactcgaacgctggcgaatatccgctgggatatttgatcgtcgaatcggaaatcgcacgcgagcgggtgaacaacagaatcagaaccgaaatgacgctgacgcagagtgcaatcgcttcggcgctcagcaagaaagcagcatcggcattcaaagaaaacatcgaaggactataggcgatggccgctcagaacgaagttgaactgattgtacgtgcgaagaacctcagcacgcgaaccatcaaccagctcaacgacgagctgagcaagatcgcagataaccaagagcaagtcgccgatgcgaaccgcttggcggagcggtcgttcgagagcctgaagtctgagcagcagcagttgctcgcgatcatgaagtctctcaacgaccgcgcttccaagctggacgcatactcgcgtcaagagcaacaggtgcgcagtctgcgcgacgagctgagtcgcgcccgcgacaacctcaacacgctcgcgcagcagttctacaacaccgaaaagccgacgaaggaattccagcagcagttgaagtcggctgcgagcgaagtcacgcggctggaatcgtcgctgcgcaataacgagcgccggctcgacacgaccggcaacaagctgcgcgacatgggcgtggatgtcacccgcttctcgcagtcgcagcaggaagtcaatcaggcgctcaacagctcggtggcgctgtacaagcgctcgaccgacaacgtggagcgctacgacgcggccgtcaaggaagtgcgcacgacgcagcagcaggctcgcgaggccgagcgcgccgcagcgcaggaagccaaggactcggcggcgaagctggaacaggccgcccgcgagcgcgaagaccagatgcgccgcgaacagaaaatggccgaactgacggccaacgtctaccgcacgctggcccgggagaaggaaaaggcggcccgggcgggggtggacttccgcgccaccggcacgcaggcgctcgccacggcccgcgcgaccgctgcccctgccgtgggtagcgggtcgtctgccggcgcggctgcggcgggcgtacaggcgcttctcgacccggccaaggatgccgtcgcgacgctcgaccggctggaaaaggccgtcgaacagctcgacgaggaattcaaggcgctcacgccggacgctttgcaggccgccgatggcatggacaagctggccgatcaaagccgccggctgcgcgctgcgtcggatgcgctgaaggggcaggccgggctcgcggacgaattgaaccgccagaacaccgcgctgctcgccagccagcagcggttcgaggaagcgcggcaagaagtgatccagtacgcgcaggcggtcgagcgtgcagacaagccgaacgacgagctggcgcagtcgttgcagcgcgcgcagaacgagatgaagcaggcgcacggcgagctgacgcgccagaccgaggcgttcaaccgcgtgcagcagcgcgccgctgccgccggcatcacgctcaacaacctgaccggcatcgagcagcgtctcgctcaggccgccgcgcgcgtgcgcaccgggcaggagcaggttgcgcagacgatgacgcggttggagcagacgaccgcgaagaccaacacgcagttgaagctcttcaacgacggacagcgcaccgcgctctcgttgtatcagcgcacccgtggtcaggtgctctcgctggtgtcggcgtacgtcggcgtgttcggtgcgatcaacctcgtcaacagcgcgatggacgcagcaatcgagaaagagcgcgtcatgtcgcgcctgctcattgcgaataaggggaaccagactgcggcagcggaagagtacgactacctgcgcaagaaggctgacgagctaggcgctgcattcggcccgctcgccgagtcgtactcgcgcttcgccgttgctgcacgcgatgcggggatgagcaccgaggcgacgcgctacatcttcgaggcgttcaccgaggctgcgaccgcaatgcggttgagcggcgacgagacggccggcgcgttccgtgcgctggaacagattttctcgaagggcttcatccaagcggaagaactgcgcggccagttgggcgaccgcatgaccggcgcgttcaatctgttcgcgaaggctatcggcgtcacgacgcaagagctgaacaacatgctcgaaaagggcggcgaagtgaaagcagagttcgtgctgctcgctgcgcagacggcccggggcatctatggcccgcaagcgaaggctgcatcgaacagcctgctcggcgacctcaaccgcatgcagaacgcatggggcgacctgaagcgcgaaatcatcgacggcggtctcggtgatgcgctgcgccgcctgttcgtcgacttgacgaagtacctgaagagtgacgacggccagaagttcgccgagaacttgacgaaggtgtttgtcgctgcggccgacgctggcggcgagctgctgaaggtgcttgctgagaacgatgaaatcatcaagctactggcggacaccgttgcgttcctcatcaagaacttcaaggcgctgctcgcgattatgctcgcgatccaaggtgcgcgcatcgcgttggtgttcacgcagcttgcaggcgaaatcctgaaggcgcgtgcggcaacgctcgcgttgaacactgcgcttggtgccggcaccgccgcgtcggcgggccgtgccggtgctgccttgggcggcctcatctccgggccgattgccgcgatcctcgccatcgctgctgcgggcatcatcatcccgatctacttccagattaagggcgagctggaatcgaacaaggtcaaggtcgacgcgcagaagacgatcaacgacctcaaccggggcttcgaggtttcgcagcgcagcctcagcgacacgtcgaagaccaacgccgaacagctcgaacgtcaggtcacggccgcacagcggttgctcgacatctacgacaagcagaaggagtcgttgcaggcgcagattcgcgagaacactgctgtgcgccgcaaccaagtggcggtacgtgttgcgcagggcacgcgcgagcacgacatgaatttcccggccaagcagctcgccgccgttcgagaagtcgagaacgaaggcaaggcactggaagcgcagctcgccgcgctcgaacagcgtgccgcaccgctgcgccagcaggtcgccgccgccagtcgtcagatcggcgaagtgaaagcgcgcgaggcggctgcggagaacgatgcgctcgcagccgagtttaagcgcatccaagcagcggccgatgcggctgcggcgcgtgccggcaccgacgcaaaggcagcgaaggcggccgaggctgcacgcaagaaggcagaagccgaagagaagcgtctggccgcgctcgccgagcgccgcctgcgtctggaagaggacgtggcggaaaagctgcgcgacatcgacaacgacattgcggcgtcgcgcccggatacgctcgaagcgcgtctggctgtgatcgacaacaagatcgcggatcgcaaagccgaactggaacgcatgctgcgtgaagccgacaagctcggtcagtcggatgcagccaagggcgaaattcagcgcggcctcgacgcactgccggcgttgcagcaagcgcaggcgcaggcgaccacacaggagttctacgagcagcggattaatgacttgttgcagcagcgacaggcgtcgatggacgcgatcaacacgttgcaggaagccggtttgctgactagcagcgaagccgccgcgcgtatcgaggaagtcaacgctcgcctgctgccgcagctcgaagcgttgcgtgcgaaggcggctgagttcatggcgacgctgggcgatggtccgcaggcgcaggccgcgcgcgccagcctcgaaaacctcagcgcgcaaattcaggcgatgtcggtcgagctgtcggcacagaagcgtcaggtcatcgacgtgttcgtcaacggcttcggtcaggcgttcatggagaccgcaacgctcatctccgacacgctgaagggcgtgcaggatgccggtgacgcatggaaggcattcggcgacatcgtgctcaataccatcgctgacatcctcatccagctcgcgcagatgattattcagcaggcgattttcaacgcgctgaaggcagcggccgagaacagcggcggcggctggggcgcgatcatctcgcaagtcgccgggtacctgcacgttggcggcgtcgtcggttccggcgctggccgtcgttcgtcggtgccgtcgtacgtgttcgatgcagcgccgcgctatcacaacggcggcatcgcgggcctcgccccggatgaagtgccgaccgtgctgaagcgcaacgaggaagtgctgaccgagaacgatccgcgccaccgcttcaacggcgggctggaaggcggggcgcaaccggcaatggacgtgtccatcatcaacaccatcgacagcgagagcgtggtcgctgccggcgcgaacacccgcgcaggacgccagtccatcttcaacgcaatcaaggctgaccgcagctcgtacaagaaacttctcgcataaggaatcgacatgggacacgcaattgcaactgtaactggcggtagcggcgacgaggcgcactacaaggtgctcgctgcgatcaagacgctcgccgaggcgaacgggtggacgacgctgcgctacgtcaacaccggcaccgtgcgcgagttgatcctcaactccgctggcctgtcgggcaccgaggacatctacatcgggttccgcacctacagcagcgtgagcggcgactactacaacctgctcgtcggcacgttcaccggctacgtctccgcgaactcgttcgacgcgcagcccggcgcgaagctgagtggcgtgccttgccacaacaacgcggtgacgtatttcatcactgcgaacgcgcagcgcatcgccggctgcttcaaggtcggcactccggtctacacccacttctacgcgggcaagatgttcccgtactcgcgcccgggcgagttcccgtcgccgctggtgtgcgccggcatgttcgatggtgctgcgccgaagcgtttcagcgacaccgactatcgctttccgtaccacggtcgcgagtcgggctacacgggcggctcgtcgtcgaatgtccgtccgtcgtacctgtggctgcgcgatcaagccggtacgtggcgtcgactctcgcacttcccgttctacaacggcccggccggcagcgatgcgtcgagtgcctacaacgccctcgaaaactggaactacttgaccggcggcgatcaatcgcgttcgctcgtcccggccggcacgaactatcagccgcagccgatcatcctgtacacgaccagcgctccggctggcgtgtgggaaggtgcggtgtacggcgagctggatggtgtgtatgcggtgtcgggcttcaacaacaacgtcgagaacgtgttgcaggtcggcggtacctacgtcgacccggcgggcctgagcatcgtcgatcacgtcgctgcgatcctcgccgctggcggccgtgcattcgtcgtgctgcaagacgtgaatcaaaccgactggcgcagctttatcgctttggagatgacctaatggcttactacaccggcaacttttcctcgttcgctacgctgaagaactcggtcgagaccgcgcttcaggcaaacggctgggggctcaacggcgacggcgtgctggaaaagaacggcatgtacctgcgcctcactgcgacggctgcgcaactgctgttgcaggccggcaccggcagcgcgaccggcgcgcttccgggcgcagctccgaacggcgtcaagatcatggacttcgagggctcgccgatgaatttcccggcgacctacgacctgcacgtcaacactggcccggacgaagtgtttctcgtcgtcaactacaacgccgacaagtaccagcagctctcgtggggcaagtcgaacgtgcagcagatcggcggcaccggcatgtggttctcgggttcgttccacgagaacgctgcgtcgaaccagaaccatctcgtctacacgtcggcggatgcgagctacttcggcttcggttggtcgggcatgggctgcggcctgttcgccgagtattacacgcaggcgctcggctgctcctacgtccacacggggctcgacacgaccgcatggcggcgcgtgtatagcggcgacggcaacctcatcggctcgggcgatcctgtcgccggcctgctgcaagcgctgccttcgatgttcaaccagaacaccgtgctgctgccgttgctggtctcgcagcgccgactctcgcagggccagactatcgtcgtcgacatggcgaacgcgcgcctgtgccgcaacgacaaccatctgtccggcgaaatcgtcgaatacggcagcgacaagtggaaggtgtatccgttccaccgcaagaacgccgacgtgcgcaacggcgtctcgtggtcgacgggcgcgaaccactccggcactttcgcatacgccattcgctacacggggccgtaactcatggcaggcatcaccggacaattcggcagtgaggtcgagcgcggcatcgctaacgtgatgctgagcgaagacttggacgacaacaccgaagtcgtctcgcggttcgactcttacgaaatgcgcccgggccttcaaggcggctacgggcgctggcgtgtgcatgccgacaaccattgggcgatcaccggccagcgcaagtcgaccagcttcttcgacgactactacaaccgcatctacatcgtgccggccgcgctcgatgccggcaacctgctgtccacgcaggtgcgccacatcatcttgtggaacgcctacgtcacgccgcagacattggagaacgccgcgctcggcccgcagtccggcatctcgatgtcgttgcctgtcggcgtgagcctgccgtacgagatggagccgctgcgcgagctggacttcaccgtgcagatcgaactcagcggcccgccgaccatcgacagctatgcgaacttcaccgtcgagggcgtcacctacaccgtgccgatcaccggccggcgcatcgtgctgttccccttctcgccgaattggggctcgcctgtcgacgagacggtcacgatgcgttcgtgggtgttggccgccgaagacggcagcgagcagaccggcagcgagtcaggcgaggttccgcgccgcacgctcgaatacaacatcaacctgcgcaccgcgttgcaggcgcagcgctgcgagaacctgctgttcgcgtggcagtcgcgcttcttcggtgtgccgcattggggcgaggaagagcgcatcgcagccgacgtggcagcgggctcgctgacgattccgttcgacaccttcggcctgtctctcgaacccggctcgttggtggcgctctaccgcgacgacgagaagaacgagattcgcgaagtgcagtctgtcgctgtcgacggcgttacggtcacgaccgggttggagtacgactggccggaaggctcgcgcgtctacccgtgcttcgtcggcctcatgaacgatgcgatgagcggcacgcgcgaaacgtcgacggttggccgcatgcctatcgcgttcgactgcgagccgagcgtgaccccgggcaacgtagcgctcaacgcgccgccgctgacctaccggggcaaggagctgtttctcggccgtaccaactggcaatcggcgatgcccttcaccttcacgtcggatgtcaagcgcgtcgactcgaacaccggcaagttcgtcgcgttctcgtcggccgggttctcgaagatgtctcgccggcacaactggacgctgtacaaccgcgccgacattttcgagttccggcagttcctcggtcgccggcaaggcgtcgcgcgctcggtgttcatgccgagcggcacggtcgacttcaacatggccgcgccgattctcgacaccgaagacatcctcgtggtcgagaacaacgagtacggcgcactggctggcgcacacccggcccgccgagacatcatcatcgagctggtcgacggcacgtacttctgccggcgcattgtcggcacgagcgacttcgacagcttcacccgactgcaactcgattcgtcgctgggcgtgtcgctcgacatcgacgacgttgcgcgtatcagcttcctcacgctgtaccgtttcgagtcgccgtcgaccaccatccgccacctgaccgactcgaaggctacggttgaagccatcatggtcgctaagaccaccgaggattgaaatgagcctgctgcaatacgagcaagacaaggaactcagctcccgcgtggagctgtacctgttcgagagcgacgacggccgctaccgctgggcctacaccaccgacgcgcgcgaaaaggtgcttggccccatcgtctacaagcccgagtcgatcaagcgcggcgagctgaagcagacggccggcgacgcgaacgtcgagaaccttcaggtcacgatgccgttcgataacccggtggcgctggcgcatgtgccgtacctgccggcgcggccgatcaagctgacgatctacgcctaccagcgcaacgatcctgctgcggaaatcgtgcaggcgttcaccggcttcatcaccagcttcaaccagaagggcgcggaagcgacgctcgaatgctcgcagatcatcgacaacctctcgcagacggtgccgtgggcggtgttcaagagcggctgcatttgggcgctgtatcaggtcggttgcggcgtcgacaagcagttgtggaagaacgatgcgctggtcacgaccgtcaacggctcggtgctgggctcgcctgagttctcggccaagccgaccggctggtacaccaacggattcgcctacaacccgcagacgggcgagcagcgattcatcgtcgcgcacgatgccgttgccggcacgatcacgctggtgtacccgtttctcgaaatcaacggaagccagaccatcgaggtctacgccggctgcgcgcgcacgaaggaagtgtgcgccgacaagttcaacaacaaactcaattacgtcgggttcgatcacttcccggcctacaacgtcttctcgcaggggatcacctaatggtttgggtagccatcgtagttgcgctcgtcatggcagtagttggcgagctgcttcggccgaagccgaaattcaacgatccgaagccttccgctgtcggcgatttttcgttcccgactgcggacgcatcgcgcgtcattccgatcttcttcggtacctgcaagatgcaaggtccgaacgtcgtgtggttcggcgacctgacgatcatcacgctgaagaagaaggtcaagaccggctggttctcgtcgaagcgcatcgtcaccgggtacaactactacctcggcgtgcagctcgtgttcgcttatgggccgtgcgacgagttcatcgagctgcgtatcgacgacaaggttgcgccgatcaccagcaagaccttcactggcgacgtgtgctcgttcacgatcaacgcgccgacgattatcagcaacgacgacccgccgaacggcgtcaagggaccgtgcaagctgtatcgcggcaccttcgagcagccgccgaatatgtacctcagcacgcaatggaacgagccggagatgaccgcgtttcgtccgctgctgcacatggtcatggagaagtgctacctcggcaacaccgacacgccgccgcccatctcgatcatcgcgcgtcgctgcccgaaccagctcggcttgaccggcggccggcacaacgtcaacggcgactcgaatatcgcgtgcgcggtgtacgaggtcatgaccaacaatatgtggggcatgaaaatccccgaagacaagatcgacgtggactcgttcatcgcctgcggcaacacgttggctgacgagagcatcggcatctcgatgctggttcagaccgccatgctcggccgcgacctcgtggcggaaatgctgcggcacgctgacggcgtggtgtacgccgatccggtgactggcctgtacacgatgacgctggcgcgcgagattccgtctgacgagcaggacgagttgttgatcgtcgacgactcgaacatcctgcccgacaccttcgagttctcgcgttcgtcgtgggagatgacgaagaacacgatcatcgtgcagtacaccgaccgcaccacgttcgagacgacgccggttcagtaccaagacctcgcgaacatcgacgtgcgcggcggcatggtcgactccgaagaattcagctacctcggcttcagcaactcgaccgctgcgatgaacaccgccgcgcgcgtatcgaagatgaaggcgtcgccgctggtgtcggcgaagatgtcgctcaaccgcatcggctaccaactgcgtccgggctccgcgttctggctgcgcaagccgaaccggggtctggcgaacgtgctcatgcgcgtcatcgaaatcaactacggcacgctggacgacccggccatcaagatcacggcgatggaagacatcttcgcagtcaacgccgtggcctacgtgccgcccgatccgagcgactggacgccgccggtcggtgccgtcgtgccgttctcgcagcagcgcctcatcgaagcgccggccttcggtgccgaggatatgtcgcgccgctacgtcatcacgatgggagtgccgtcgagcaacggcgtgatcgcgtacgacgtttggacggacgccagcggcggcacgaatttccagcagaccaactccatcgacgcgctcacgccttcgggcgtgctggtgtcgggtctgtctcgtactggcccggaagtcgatgctgctggcttcaccgtcacgtcggtcgtcggcgtcagcgacatcgaatctggcactgcgggctcgcgcgagtcgggcgaaaacctgctgctggtcggcaacgaactcatggcatggcagaacatcgtcgacaacggcaacggcacgtacacgatcactggcgtgtatcgcggcgtgctcgacaccatgccgcaagaccacggctccggtgcgcgcgtttatttcatgtcggaaggtgcgggcacgaccaacgaggacggctacggcggcgacctgacgctcaacacgaagctgacgccgaagagcatcgtcgacacggtgccgctggacaatgctgcggcaatgtcgatcacgaccaacgctcgtgcgctgcgcccgctgccgccgggtcgcctgcgcatcgacggtgcagtcgtcggctccggcgcaacctacgatggcgacatgctgttctcgtgggcgcatcgcaatcgcttcgacgacagcatcgcatcgcaggccgatccgagtcgcacgcccgaggaaggcacgacctacaacatccgggtctacaccagctcgaacgcactactggcgtctgcactggaagtatcgagcgccgcgtcgaccggcaccatgcggttcgcggtgtcgggcgatatgcgcattgaaatcgaggcggttcgggacggctacgtgtcgtggtcgaagctggtcggctacttcagctatactccggccgccggggctaccgccaacgaaatcatcgtcgacgagcctgagtacgtcttggacgggggtggcgcgtaatggcacaggtagtcgttgcacaacgcatgtggcagcgccgcgacactgcggcgaattggtctgccaagaacccgatccttgcgggcggcgaaatcggcgtgcaactcggcgctacttcggacgagaccaagttcaagatcggtgacggcgtgaccccgtggaactcgttgtcgttcttcgagggccggctcatcgaaatcggcacgggcagcggctacatccgctggcgctatgtcggtgatccgacgtggatcaatctggtctcgctcgaatcgctgcgcggcccggccggcgcgaacggcgcgcaaggcccgcaagggctgagcgcgtatcaggtcgcggtcgccaatgggttcgccggcacgcaggccgaatggctcgcatcgcttaaaggcgagaagggcgatcaaggcgaccaagggccgcccggcattccgtcgcagcgtcgcatcctgcgcatcacgaacaccgacagcggctccatcgtgtgcgactggaatgcctacgacgaaattcgcgtgacgctgactgccgacacgctcgtcaatatgacgggcgcgctggacggtcaaggctgcgtgctgctgctgaagcaaggcggcgtcggcggtcacggcgtttcgttcggcagcaacgtgcgcttcaacaacctcatcccgatctacaacccgacaacgactgccggcaagtccgacaggctcggcttcgtttatgacgacgacgccggcttctacgacgtgcaggcaatcgtggatggaatctaacgatggcagacgactacatcccgccgttgtcgccgaacatcgtgtgggtcttcaagggcaacgactacacgcccccgctgaccccgaacatcgaatggatattcggtgcagatgatgaaggcggcggaaacgagcttcgcaaatccacctatatgctaatcctgacaatgtgaggtattgaaatgactgttcgcatctactcttcttccgacgctggcgctccggttctgcgcggcaacacgccgggcgacctcatcaacctgctcgaaaagtgtctcgtcaccggctacgggtcgaaggtcggcgcaggttggacgaagccatacaccggcacgaacgtcgctgcattccagcaaggcgcaggctcgaacggcatgttcctgcgcgtcgacgacacgagcacggcgaccagctaccgtgcagcgcgcatcgtgggctacgagtcgatgagcgatgtcaacaccggcacgccgacttcgttcccgacgccgacgcagcgcagcggtggcgcagcatggttcacgcactacagcagcggctcggtcgcgaacccgcgcccgtggcgcatcatcgctgacgagatgttcttctggttcttcctgtcgacctacccggaaaacaacgacagcggtttctactacaacgagagttatgcgttcggcgacatcattccgttcaagccgggcgacacgacgcataccgttctgctcgccagctactcggtcgactcgccgaattcctcggagccttacccgtgggatggcgtcagcatttcgagcgcgatgggaagcaatcgctacggcctgtgggcggcgcgttcgtacacgaatctcggcggcccgatctggctcggctggcacgccgatcacgttaaggcttcttcgagttggggccaagggttcctgtcgtacccgcatggcccggacggcggcctgtacctgtcgcctgtgtgggttcacgagtaccacgtctcgccgtacaacgtacgagggatcatgccgggcctgtgggtgccgtgccactaccaaggaatcctgagccagtatcaggtgttcgatggtcagggcgaattggccggaaggcagttcatggctcgccgccactacgagcgcacggtctgcatcgaaatctcgaatacttgggataggtaacgcgcgatggcgctcatcttcaacctgccgatgacggggccgaacggctccacgacgatcaccgacaccacggggaatttctcgtggtcggtgacaggcaacgcgcagattcaatccaacgctctcgtccttgacgggagcggtgactacgtgagcaccactgctgacgttcgattgaacttcgggccgatcaacgatttccgtatcgcgttcgacatgaagatggcggctgcggacaagggcggctataagatcatcttcgaccagctcaacacgggtgcgtcgaatacgtggacgtggcagctctacacctatgaaggtgtgccgtacttcaacgtctataacaattactacggcaatccgacgccggttcaaggcacgaccgatcttgctgacggcaactggcacacggttgaagtcattcgcactggcggcgctctctcgatgtgggttgacggcgtgcaggttgcaactgctaccgacaatcgcgactacgtgttccagccgcctttcggcatcggttcgcgtatcggctacaacgcatcgtcggcctacgactacaagggcgagctgcgcaacttgtccatttcgatcacgacgccggtcatcctgacgaatcgcatcgcgtcgtggactcggcacagcgacatcggctggaaccgtggccgccgaagcagcttcattcggcgcatggcgttctacccggtgcagccggtcacgaccaagaaggtgcagacggtcaaggtgacgcgcggcgtaccgccgtggtgggggccaagcggatcgaccacgcagctcccgacgtacaagctgcgcggccgagtgatgcagcgcgatcctgacggcgtgttgcccgacgccccggtacagtacgcgcgcgtcgtgctgttcttccggcgcttgcatacgctcgtagacatccagctctccgatgtcgacggctacgtgcaattcgataacctcatgccgggcagtcaagcgtactacgcgattgcattcgacccggaaggcgcaccgttgcagaacgcggtgatttgggatcgactgtcgcccgagcccggcccgtaaggagaagtgccgtgagcccgaacaacaccaacgagcagaacaggaaccgacgagtgacggacaaagcaggggggcttctggacgccgcgcaacaggccatccggcttgaacgcatcgaaggcgatatgcgtctgctcacgcagcgcgtcagctccggcatggagaacgtcagcgccacgctcgcggccgtgcaggtcgaagtgcgtggttgctcgacgaacgtgtcggagctgcgcgggctgcaaggtgcgcacgactcgaacaaggtagcaatcgacaaggtggagaaatcagtgaccgacctcggtgcgcgcttggagtcgtggttcgatgagttcgaggcaaagcaggaacagcggtggcgcgactatcaaaccaaccgcgatcaatggcggcgcgagcacgaggccgagaacgagaacgtcaagaaggacttggaaaaggaaatccgcagcgttcgcgaaaccgtcattcgtttcgtcgggttcggttccgccatcggtgcgctcgcgggcgtgatcgtcggcggcttcctgtggaatatcaactaccgcttcaacgaccataaagaggacgtgacccgagtcgaacaaacgtcattgcgcaaccgacaactcatcgaccagatgggtgtcgatcacggcaaagagctggccgacatcaagctctacctcgcgcgcggcgggcgaatccccgctgagccctatgtccctcaatcgcaaaggaacaacaatggaaacgaacaagactccggccaacccggaaagtgaaatgcccttccgccgccgcgcgtgggagttctggcggcgcaatcaaatcctgttgctgcaactaccgctcatgctggcgttcctcatcggcagctacgtcgtgctgaagtcggtcgactcgcgcatcggcgtcgagggtttcggcgacatcttcggctacgcgctcaacggcgtgcgcatcacgctcatcatcttcaccgcatggtggatcaagaagtggtgctggttcgacctgcacgacaagaccgagctggcgatgttcgaggcgatgaaggccggcgactggatggcgttctggatcgtggtgcgcgaccgggccgagtggctggctgcgctggcgttcgcgaccttctggtacacccgatgagcgcccgggtcgtagtcctcgctgcggccctcctgctgagcgcggcgtgcgctcggccggcagcggtacccccggtcgaccagaccacgctcccgccggccgtggagagcctgcctgcggccacgccggagccggtcgtcgagcaggtcgtcgcggctcagcccctaccccgggccgagcaggctgtttcggagaccgtcacggagccgcttctggccgcgcaggcggcgctcgaagaccttaccccgctactacccccgccgccggcccgggacgcggcttgccggcgcgctgcggcggccctgacgctacgctgggaagtgaccagcccggccttctaccggaagcggctcgaactgccgatctggccgggcggggcgtccggggtgacgtgggggatcgggtacgacgggggccaccagacccgcaccgtgatcgtcgacgactggcacgaccacgggcaggttgaccggctgggccagaccgccggcatcctcggccggcaggcccgggcggcgctgccgcgcttccgcgacatcccgaccggcttcgaccatgccagtcgtgtgttcgaggaacgcagcctcgtcgagtacgagcggcgcaccgagcgcgcgttccgcaacggcttcaccgagctgcggccgaacgcatgcggcgcgctcatctcgctggtgtacaaccgtggcgcggcgatgaccggcgactcgcgacgggagatgcgcaacatccgcgacaactgcgtgccgaagcaggactacgcctgcatcgctgcggagattcgctcgatgaagcgcctgtggcgtggcacggtcaacgagaacggattgtctgcgcgccgcgaggccgaagcgatcctcactgaaaccccgtagggagaagagcatgtggacgaaagcaatcgcgtggctgttcggaacggcaatgggtcgcggtgtgctgctgggcggcagcatcgcgataggcacggcgctcggctggtatgcgttctcgacgcactactacaacgagggcgtcgcgtcgtgccaagctggccgcgccaccgatacgaacgcggccaacgtcgcgcaaggtgaaaagaacatcgccgacaaccagaccagctccgacatcggcaaggccgccgacgccgaagcagcgaaggtcgcagccgatgccgaagaagcgaagaacgactcgaaggagaccatccatgacgtgtacaagcaaccccctgtcactgcgcctgttgctgttggttcttgcgtgcatcctctcgatgagcgggtgcaagaccggatcggcaaagcgcgagctgccgcagttgaagcaagaagccccgctcgttaactgcaagcagcctgcgtcgccggcagtgccgcgcgagccgaaggccgacgagtggatcgagtggaacccgccgcgccccggcaaggccgaaggagaagcacggcttagcgagcgtgccgtgaactggatcatcgacgtgctggccgtggtgcgagtgggcgagggctaccgccgcgtcgagcacaagtgcctcgacgagctggaagcgaaagggctcatccggcagtagttgacaggcccgaggcgctgcattacggttgatcccgctggtggcacttcgcgttgcatcggcactcggcagagggacagcggcgcggagaatcggcgctccgcaccgcagggaacgaggaaccccggactaacactccggggtttctttttgcgtcaagaccaagtgcgtcgtgaccaagttcgtcaagaccggaaaagagaaaagccccggtgctgaggccggggcttttcgggttgcgcgactcacgtcgggcggtgggtatcgaggcgggggttctgctgattccggtgtccgctctatgagcgctgcgccggctggaagggcatgtgtcgcgtcgatggatcgaacctaatgcggcacgccgcgcgtgtcaacaccttcgtcagtccttccacgtctcgacgagcttcagcatcttcttgcgcgccttctcgacgccggccgcccacttgtcccatgcgcgcggatcgacgtgcgtcaggatttcgttgcgcgccatctcgctcagcacggtcggcggcagcgcgtccagctcccagctcttgtcgccgaagcgctggcggtatttcacgaagcgcgcgtcggtcgtcttggccgggttcggtggcggcttcagctcttcgatctggtcgaggttgagcgccatgcgcttcagcgtgaactcgccgttccaaccgaacagctcgaagcgctcttcgaggtcgcgcgtcatgtcgatgccgctcgggtcgtgatccccgaagtgcaggatcaccacatccttgccgtcgctctcttcgatttcccgcttggcgaaatcgcgcacgaccgatgcgctcgggtagccgcgcgctgcgagcagcggcacgtcgaactcgtggcacacgcgcgaaaacacgccgaccagcgcttccttctcgacgacgaggaacaggcgcttctcctgcgtcgcccacgggtcggtgtggtactgccgcgccgacgccgtgagaatgtcctgcgggcgcgaccagcggctccgctgctcgaacgagcgcgtgcggtcttcgatggcatcccaatcaatcaggcccgcgatgcgtgcgtcgttgacgatgctcgtggtctgcttgtacgacttctcgttgttcggaatgatgtcgcgcgcaacgagctggtagtagagctggcgcacggtcagcgtgtaccccgcatcgagatattcttcgatgatcgcgttgatcctgtcgatctgttgcagggtcttcgtcttgaaggtgatttctttgtagcgttcgagactcatggcactcggctcctgttagcggctggcgggctgttcggcggcccggatgtcagtggcgcggatggattcgatttcaggcggcagttcgatgcgctcgaccgcgtagccaacatcgcggccgtagtacacgccgcgcacgtcgggcaccgggtagacgtggtagctgccggcgtgcatgtgcagcgcgtggtggatgcgctgctcgatctgcgggtaggtgtacgggttgtccgggctcggctgcacggtgcgcacgccgatgccgacgtagccgctgcgcgccagcgtctcgcggaacagcgcggtgtgtcccgcatgccacggctgatagcggccgatcatcgtgccctgcggcgtcaggtagcgcaggcacgcagcgatgcgttcgagcgtgggctgcatcacttcggccgtgacctgcaccgcgacttgctgcgggcgctcgaacatttcgtcggtgtccgggtagcggctcttctgcaccgtgtccatgaagacgatgaggtcaggcgcgaacgcctcgcgcgtctcttcggtcgggcacacgaacgacgcgacgacgatgccgtcgtggctgtccgcgacctcacgcatgagctgcgcttggcggatgcggcccggcgcactgaagtcccaatcgccgtgctcttcgcgcactgcgtcgccgtcgatgtgcgttgccggcaacacgcgcgcgagtgctgcgccgagcgtggtcttgccgctgcccggcagaccgcagatgagaattcgcttagccattgttcgattccttctgtgcgcgaagttcttcgcggatttccatgagcagcaggccgagatgattctcgcccttgccgtcgcacacgccccaaaaacggtcgccccaccaattcccttcgacgagcttcgacttcccggtcttcagcaggcgcgaccgaagcgggtcggtgccgaacttctggcgcagcaggtcgcgcatgacgccgaccttgatctgctcccaatcctcgcgcagcgttgcgtgcttgccgcgctgcttcgcgccagcggcgctcggctcgttgcgaatgcgacggcgctcgtcctcgtcgagcgtcttggctgcttggaaggcgtgctccacggtgcggtacgagtgcccctcgaaggcgatgcagcatgaccagaaattcgagaggaagcggtacgggccgttgaagctgtcgatggtcttcatggtgtcccctagtggaagtcgatcttcgccttgctgaagagctggcgctgcttctgcatgtcggtgcgagtgatctggtcttggatgggaacctgcacgttgcgattcatcatctggtgcaggtagcgcggctcgaccgcgtgcccggtcgcgaacttcgcaatcgccatgagaatttgcggcgagtgcagctcgaagaacgtgccggtcatcgaccacggttgcggtcgaatgtgcgccgcgatgtcgagcagttgccgctcggccttgcgcacgttgagcggcggctggatgccttgcttcttcatcgagtgctcgacctcgctggccgcgcgatgcacgacgaggtactgcgcgcccgggaaccggacgagcagttggtcgaagaagaacagcgcggccacgtccgacacgaacacgcggccgggcggctgcgcgtcgatcttctggcccagctcagcgatgctcgcgcactgctgaagcgggttgtgcatcgacgagacgcacagcggccgaaggaactcggccatccatgcgctgcggctgcgcggcaggctgagcatgatcgtcaggtgctcgtacgccatgtcagccctccttctgctcgcgcgcgttcttcgcgttgtcagcgtacgtgtcgagcacgcggacgaacgcatcgtgcagcagcgtgccggcgggcacgtagatcaccgtgccgccggtcaggtcgttgcgggtgtagatggtcggagccgcgcccgggatgagctggccctgaccttctggcgtcgcctgcatgcgatccggtgggcgcgagtcgaactcgcgcaccagaccgtccgcagggccaccgacgaagaagccacggacggacgtgttcatcgcacgtctccgtcgccctgcaacgtgccgcgctccctgcgcccgttgagcttttcgcggttgtcgaacagcagcttttcatagccgccctcgcagccgaccagcggccccgtgcgctcggcatattcgaccgagaccgcgatgacggaagccagcgcgccgcgcagctcggcgatcttttccgcgcgcttctcgccgctccacgttgcgccgtcgcgcatcatcttcttgatgacgcccaacacgcggcccgcgtgcgcgcacagcgccgattgcaggtcgtagccgctgatacgaacctcgcggtgctcggcgtcggcaaggcgctgcatgccttcctgcaccagcacgtcgaagcgcggcagctccggcgtctcggcgcacaggcgcgcggcgtaccactgcacgtcgcccagctcgtgccacgccttctggtagcgctcgacacgaaactcttccttgatggcttcttggtcgaacagctcggccagctcgccgacttcgttcgccagaccgatgccggtgtacagcatgcccgcgctcacgttgccggcgagctgcacgatgtcggtcgggtacttggccgtggtgacggtgaaggcgttgtacgcctcagcgaagatgcgcgtgggttcgacgcgcgcggcacgcgactcgcgtgcggtatcgagggacaggatgctcatgcgcggcccccggcggcgagcgcgtcagcgaagtcgttgctgtagctggcctcgaacttcgtcgccatgtcgtgcaggacgagcgtggggccgccgtgcgctgccgggatcatggcgaagtcgacgccgcgcaccagcgggttgcgctcgccgtcctgaccgatggcatgcacgaccaacgcttcggggttctcgcgcgcggcgcggcgctcggccttcaggatgcgccgcatggtcttgccgccgaacgccttgcgcagcttttcctcgggcgagccgtggtcgcggatggcgagcacgccggcaatgccgcccttcgacgtgcgcacctgacgcttgttcttgcgctgctcgttttcgaggtcgcgctgctggacgaggaaggcgtagttctcgtcgacggcgagcatgcgcttgcgccagtcgctcagggtcttgcccttctcggcattgtaggaacggaaaatgcgcttcaacaggttcatcgtgtggctccttcaggtgtgaaaaaagcggcccggccgatgtcgacggggccgcttcgatgtactacttcaacgccaccgggctcagcggccggcgacgaacttggtctgcttctgcacccggccgcgcttggtctcgcggaacagcacgatggtcgtgttgtcgtcggccatgatgctcgcgtcgtcgagcgcgttgctctcggtcgcgaacgggccgttcatggtgctggccttctgcgaaccgtcttcctgcgcggtcagcagcaggtacgcgaactgcttcgcgcccttcttgccgcgacgcacgccgaccttgcgggcggcggtcttcttgccggcgggacggccgcgcttcttggcgggcgcggcggcctcggtcttcttcgcagcgcgcttggccggagccttcttcgcggcggccttgcgtgcggtcttggcgggagccttcttggtggccttcttggcagcggcgcgcttcttcgcgaccttgccttcggtggcttcggcgttctcggacatctggtttctcctagcgttgttgtcgacaactcgcggaatgcgagcggggttcccttgcgggattcggttcagtccacgcagtacgcggggacttcggtgcggaacgtccggcactcggacggctgcgtgatgtacaggccggcgatggcggccagcagcaacacgccgtagacgatcttctcgcggcggctcatcactcgcagcccacggtggcgttcgggcgggtcggatgcgcggcggtgtactggctgaagtcgcgccagccttccgagccgccgcacgcgaagccccagcggcgcacgatggagccggtcatgaagagcgtccagcacggctcgtcgttgttgccgaacagttcgagcaggtgcatgtggtcggcgctcaggcggcggaagtcgcccgtgtggaagtgctgcgtgtagtcgaacttgtgctggcccgggaacttgcccttgtttcgcaacacgctgccttcgacgaacgtgcggccatcgttcggagtgaacagtcggtgcatgtacgagacgtgcgcgtccatgccttcggggctctcgtcgatggcgtgctcgtagcaccactcgctcgtgtgctcgatgtagcgaccgtcgaggatgagcgacgcactagcccacgggtgatcgtgcagtgcgcggtcgtcgtcgccatgcacgaacttgtgcaggtacaggttgaaccagcggttgcgcgggatgatgtgccagcgcgtcaggtacgggcggcgcgggccgccgtcgatgccgtcgagcatgatgaccttggacggcgagacgatgcgcgcgtacagcttgaacgcaccgacgaagagcggccacaggccgatcatcgagagcacgttgtagaaccggcgggagaccttgggggcgttcatggcggggaacatcctcggtatggtggggtaattcatgcgtcgggcgtcgtgtcggcggtggccgggccatccgcgttggtcgtgtcgacctgcgggcgaacgagcgggagcggctgcgagccatcgagattcttgaactcgatgtagtagcgcgtgttgagcgtcttcagtccggtgtcgacacggttctggaagacggtcagcagttcggccttcgtcagctctccggcgtgcatgccgccttcggagacgacgcggaagttttcggtgtcgccgctcgtgagcacggcgaggttgtggcggtcgaggatgagcttgtcgagcaagtcgcggatattcggcagttcggcgaagtcgattttcattggttctctcggcgtgagatgaagagcggcgtatcgtgccgcaagccgccgggttgacccttcaagcgctggggagtgcgccatccagttgaccgggggtatcgcctcggcgaccccgtgcagttcgtgatttaccccgtagggggacgaagtaaattcgttactgcggggccactctaacgccagcttttcggcttgtcaacacccttcctcgtgtcgggcgggcggctcagccgggccatcttccgctcgccccggaacagcctgtcgcgcagcatcttctcgctgacgtgcgggcagtgacgcctgatctgctcgaacgtcatctcatccccgtcgatggtgtacagcttcactcgtgcaactgccttcacttcgtagtcctcgtcgtcgaatttctgcctgctcatagcgcccgcccgtgtgtctcgatgtagatgtcgtgcagcatctcgtgcgcaatcgcttttcggaacgccggctgctgcacgagtgcgtgtgcgaagtcgcgcgctgtcggctccttcatgccgagatgcgccgtcatgcgcagcgcctcgtcgatgatggcctgcgcttcgccctcggcgtagccgtcgtccgcgagcagcgcgtggatggcctcgcggtacttcgcgtgtcgcgcgcgctgccgcagcatcgcaatgccggcgatgacgttggggccgataaccagaagcaaccaatcgaaccagctcatacagacctcgcgtacggacgctcttcgccttccttgggcttcggaacgtcatggagagtggacagtcctttcttgatcttggcagccatcgccttgccgaactccgacgcatcgccgtacatgaggtcgaggtcgggatcggcgcactcggccgcgacgttgcgcagcgtgtcgagcagcatcgggagctggtgctgcgcgctgtagttctcgtggatcatcgtccacgctccctgcgccttccaccactgctttcgctcgtgctcgttgagcgcgacgtactggtcgatcatcgccatcgcgaggaacggcgaccagaagcatgtgtcgaccggggtgatcgagtcgcccagctcgtcgagcgcgaagtacaccgcgaagacaggcgtggtgccgatgaggtagaccggctcgtcgagcgggtctttgtaggtggcgatggtgcagccccggtacgcggccatgtgtgcgtagcggcgcttgctggcgtcagggagtggcatgcggaaactctcgttgaagtacgggtcaagggacgctgaggcgtacaagcacgcctgcttgggctcaggttgtgcagctctcatggcggtgaagctgcgctcgctcatgcgccgccggcatcgcgcacgagcacgacttcgccgtcctcgccgtcaggcaggcacgcagccagcacgtcggccgcgccctgcgtgtcgccgagcacgagcagttggatcgcggcgcggatcgcggtctcggtctcgacggccttgcgctcggcggcgagcacgtagcccgcaccgtcgcacagctcttcgagcagatggcgcaaccactgcgcggtcgtgaggtctttccggtcgagcgtcacgccgtacttcttcaagccggcgtcggcgcgctgacggatgatcgagatgaggtcgttcgtggtctgcatgtcactcatggtcagaactccttggcgaaatctttctcggcgcgcagcaaggtcgaaaccttcgcgtcgaactttttggggttgtcgagcaggatgtcggcggcggcttgcgcgatgatcggcgagatgaaataggcgttgatcgggtgcagcacttcgccgaagtcgtcgacgatgtagtacgcaacgtgtaccgcgatgccgccgccgatcttgccgtcgcggtcatcgagaacgcgcagcggccggtccatatgcagctcggcgatgaacacgtcgcggtacggttggatgcgcttgaacttcatgcggctttgtccttcaggtggtcgagttgccagcccgcttcgattgcagcgaacagccgcagctcgctcgcgtcttcggtgtcgagccgcaggaactcgatgaagctgtcgatcatctgcggcgtcatcggtcgcttgtcgtagaacctgcggtacgcgctttgcggaatcatgtcccacaccgggcacaggtcgacgatgcgcttgccttcctcgcgaagatggcggcgcatgatgtcgcgcaccgtcttcgggttcttcttgaccgtgatctttcggccggtcgacggacggaaactcatagcccgatgtcctcgccttcttcacgcttcaacagccacatcggcttgcgcgagagcatcggcagcgggccgatccatccatcgacgagaccgtggtgtcggttccagccgtagttgtcccaccagcgtccgcgcttctggcccagctcgggtagccacacggcaatttccatttccttgtgcgcgggcagtgcggtcgggaacgggtggtgccagatggcgtagaagccgaactccggcgggtcttcaagcacttcgatgtcgttgtactgcatcggcccggcccagccgagcacgagcccgttgaacggcacgaacggcttttgcaggctcggtcgacgctcccaccacatgccgttcgcccagcgcatcaccgagtacatgcgcgggtcatgcacgatggtcgggttgcgcgtcagctcgacggcgtacatgccttcgatggtcggatcgtcgagcacttcgagttgttcaatcttcatcgcgtggagcctcgacgtgagtgcgcagtggccgcaggcgcggcagcgggccgatccagccgtggacttctcccctgaagtattggtcgctgttgaggtagcaccagcggccgttgaaccacatgaggaagatgtcgacgacgagcccgcgaccgtgcgggtcgtctacgcggcaagcgtagacgcccgtgtcctgcggcagtccgatttcttcgtactgcaccttcacggcatgcacttctcggcgtaggtgcggcagtcgcgcatgaagtcgatgtagacctcgggcggcaggtcacgcatcgtcgtcacgccgaacgcctgcatgtgggccttcagcctgtcggtgccgtggatgatgcggaacagccgcgcgtactcgtacaccatctcgcgcatgcgatcctgctcggtacgaatgcgctccggcccccacgagccgccgcgttccttcttcagcgcgtcgacttcgcgcgtacgcgattcgagcgtggcggccagcttcttgttctgctcgcgcaggtcgtcgttctccttgcggccgtgcatgcgcaccagcgtgcggatagcacgaatcgcgaggtcggtctggttgagcgtgggtccgctggtcggccgcttgtcccagcccggcagacggcgatgcagttcatcgaacacgcgcacgaggtcgaacaccgctgcgtcgtcgatggcctcgaacgcctcgtgcagcttgcgcccggcctcggccgcagcgtgcgcctgctcgccgacactacgcagcgcctcgctcgcgtccttcgtgtccagccgcagctcgacctcgacggtcttgcgcgcattgccctcgtcgtccgccggccgccacgttgcgagccacgtcgcatggtcgcggtaggtgaacttggtgcggtgcttgtcgccgtcgcgctccatcgtcacgtagtagtccgtgctgtcctgcttgcggcgcgcgtcgactacggtgtaggtgctgcccgagatgacggagaagtagcgctcgccagcggccggcggttgctcgctgccgtcgaacggcacgttctcgatgaagtcgcggaacagcgattcgataaggccgtagcccatgccgagttcgggcggcatcccgacgcgacgctcgcgcgcaggcttgaacgacacgtcgtacagctcggcggccatctgcgcatagggtgtcaggcccggcactttgtccgaagtcgtcggcgcgaacatttcgttccatgcgctcggcgtcgtgaacgtccactcgtactcgccgccgcgctggttgtcgacgcgcagcatgcggacatgcgagtggccctcgcactcgtgcgtgctcacgaccatgaagaagcgcgccgggcgattgcggtcctgccagtaggtgccgaccttcggcgcgaactcgtagcccgggtggccgaccgtcactgcacgcgcttccttgcggtcgctcgcagcccccgtggtcgtctgcgtgctgcccttcgagaagtcgcgacgcatgatgcgctcgatgaggctcggcgtgcccttcattgcctcggcgatggcgtccgggctgaagtcgatggtgttgatgatgtggatttcgggcgcgctcgggctctcggcgaacgacggcgcgggcaccttgccgttgtgcgcattgaagaagaactcgtgctggccgacgaacgtgttgcgaacccagcggtggatgcgctgcgcttccgcgcgctggatgtcgttctggccgacgatgccgccggcagcgtgcatgtcgcgcacgatgccgttgtcgtcgatgcacgcggcgaccgacacgatcatcggggtggtagcgtcgttggtgaactgcttttcggtatgacgagacattttcggcgtttcctcggttgggttaggtggtgctgacgtgaccggcggcctcgcggtcaagttgtaggtctgcgatgtcacgcagcgacgaaggccagtcgtcgagcggcacgagtccttcctcgtgcatggtgatctggtcgggcgtcaggccgcacaggtagtacgccttcgcgagcgacatgccggcgataagtcgatagcgcatagcggcgcggccatgcttgaaggattcgacttgcgcccgtgtcacttcgcccgtgcctcggcacagccggcacttcgtccccggcaagttgtcgtcgtgtcctgcgtcggggccgaacatctcgttgaactcgatcatgtcgtgccgcccttcgcagcgcgggcagacagtcttgtcacggagccaacgccacgccgcgcgcaccttcatccgcagggcggtacttactgcgcgaccgagcagggcggtagcggtgcgcagacgagacaaagggggtaccggagcattccgagaagccgcaagcctgcggcccaacattttcgcttcttcgatttcgcggcgtgtgtggcgcatggtgttggtcactccatccgggtgacagtgaggaaggcgaacatggcgtcgttgctggcgctcatgtaggtgccgcgctccatcttgaagcgcttgtgcttgtggtcgcccgctgcgcgcaccttcgcgatgccgccgctcaggatcgagttctgctgcttgaagtatttctgcgcctcgttgttgatcgcggcgatgttcccgttgtcgagcgggatgcgctggcagcgcgcgtgcgactcgccgatgtcgagcttgctgagctggtcgttgagcgagcccggcaggaagatcaaccggggcttctcgacgatgcgcacgcgcgggttggcgatgtcgctcttcttgatcttcgagcccggctttttgcggctcttcttcgcaggcgcggcgctgctgttcgtggtggcggatgccattaggtgatgcctcctgttccggggaagtaagcggacaagaaacatactactgcgcgcacccggggtcgtgtcaacccgggcgttctcggtcgtgaccaactcgcgcgccgggccagcgccgcacaacgatccggctaggttgtcgaagcgggcgcaatttcggaaccggctaggtcggcgaagcgagagcgcaaacggaaccggctggctttgcgaagcgggccgaattttggaacgggctaggttggcgaagcggggaggtttttggaattgctctcttacatgtacgtgcgtgcgagcatgcgcatgtgcgcacgacgcgcgctcgctcgcgcgcatcacgcggttcctttatgtcgccggatcgcatcgccggcacgtcgcagcgcatgcgacgcgatgcgcgcagcgtgcaagggagcgcggcgcgttgcgcggttcccttcatccgggcgcgcttgccgccttccgcgcttcctgaatgcaaagtaaacggactactgcgcgcagtaaaaaaatacttgcacgcggcgcggaaccgtgtagcctacgcataccggcaacgtcgccggcatcgcaaagggtcgcaaacatggcacgcatgaaccgttccgaattttccgccaatgccgcgcttgccgcgtcgcgtggcgcgtccgctgcgcgcaaggtcgaaaccgcgcgcaaggtccagacgttgcgcgatttgctcgcgcgtctcccctttctgttttccgtcgccgttgccgcctttgtcgcggtcgcggccgtcgccgtttccgtcatctaagggaatcaattcaccatgaacaagactcgccgaaacatgctcgacgcgctgcaaaatcgcattagcgcgctgccgctggaaaatcttttcgatgaaatgcgcgccattgcggaagagctggaaagcctgcgcgatgaagagcaagacgcattcgacaacctgccgcagtctttgcaggacggcgagcgcgggcaggacatgcaagccgcaatcgacgcgatggatacggccggcgaattgctgcgcgcattcgaggatatttgcgacaacgcatccgaagcgttcgcagcgattgaagatgcaaaggggatcgcgtaatgcgccgctatcttttcatttcatccgctacgctgccggttgtcgcctacgcggaaagcaaagacgcaatgcgcgcatacgtgcgcgacctgctagggattccgtacggtttcccgctgccgcgtcataccgtttgcagcatcgcctaacaattcaccagacaaggaaaattcaccatgcaacgtattagcctttcgcaagccttcgcacagtggcaagagctggcggccgacctgccgcaagatgacgcgcccatgctggcggaatcgtggaacgattacacggattcgctttgcaaggatggcgcattgtgcgacctgcaataccgctacgcgcccgcatacgatgaagagatgcccggcgacggttcgcgcttcgatccgctgagcgatgaccgcgaattcatcctagacgcgctaggcgtcaccatgcgcgcaacgcgcaaggatggaccgcgcgaaggatgggacgcgagcgcgtcacactggcgcgtcacgctgcgccgcgaccgcgcgagcatgacaacggattacagcatgggcgcggcgcatacgggctcgcctgagctggcggacgtgctgaattgcctgatgcgcgatgcggaatgcggcgcgcagtctttcgaggatttttgcgcggaccttggatacgacacggattcgcgcagcgcggaaaagacgtggcgcgcgtgcaaggtaacggccgtcgggctcgcgcggcttttcagcgatggcattctgcgcgacctgcgcgaattgttcgaggatttttgaccatgagcgagctagacattagcgcggttgtcgccggcatgcgcgacccttggaattactcggcgagcgttgcggaacgcgggcaggatgccggccgcatgacgtgggaagccgcatgcgaggatgcgcgcggcttgttcggcgagcatttcgaccgcgccgcgttcgatgagtatttttcgcatttcggcgcatgggacgcggaagaattggccgcgcatacggatgaagaatgcgccgcgcttatgctgcaattcatcgccggcgaaatgcgcgaggctgatttttccagctatgccgacatcgaaggcggcgcggaaccgttcacggatgaatggtggccgcagtatgaaaaagcgagcgaggccggaaccgtcgccggccgtttctgccgcgacgctggcggcgttttttactacattggagaatgaaacatgcaaagcaaatgggcaaagacaaccgcgcagcgcatcgcatccggcgagctggcggaatccatcatccgcaaggcgcgcgcgttgctgcgcgatgccgtgaatgctgaagagtatttcaagcgcgaaccgtcgccgtctgctaccgctgcggaagcgtgggagctggtggagatgattagcacgcatgcgccgcgcgtcacggatgcgcaagcgcgcaaaggcgcggaatggctgcgccgccttgtctacacgtcgcgcggcacggtgcgccgcacggaagccgcgcagcaattcagcgatgcggacctgcgcgttttgcaggcttgcatcgcgcgcccggccttccgtctggtggagctggaaccgcacagcgacggccgatacctgcgcgaccttgcgcccgtctatcgctgcatcggcgacaacggcgaatccttcgattacacggcgaccgcgtggcagtctggcggcgcgttcgcaatcctgcgccacgcttaacccttcccatccgtgacaagcccggagaatctgaaaatgtacagcatcgcaaacaacgcaaagcccgccattctgacgcgcacggaatcgcgcatccaatcgcagcgcgacaagcgaacgcgcgacacggaagcgcgccgcgcaaagtatcggcgcaacgctgcgcgctatctggccgcgtctttctggcgcggctcgcgcgacatcgccgatttttttaagggtcgcggattcgaccatgcgacgttgcaggatgcggaaaacgattgcatggataacgtcgatttttcttatctgtattcccgcgactatgcgcgcgagctggaaaaggaatacggcgacgacgcgcgcgaattgttcgcgtacctttgcccggatgcgccgctgagcgtgtaccgtgagcaaatcgccgacgacgtgacgcgcgcggtcgcagactcgcggcgcgcggattatgcgttgcagtttttcgactggtgccgcgatgcggtcgaggatgcggccgattcttccgggcttgtctggtgctggctggacaaggccggcaagcctacggatcaggaatacgatgcgcacgcggtaggcttcgcatgctcgcgccgcatgtacctttcgcgcaatgcggaatggtggccggaaaaatggtgggcgaaaggtgaaagcgtttggagcgattacgcgagcaatcgcgaacgcatggacgcggccgatgacgtgctgaacgaatttctcggtgagcatctggaaagcgaaggcgcggaccttgaatcgttcgatgagcgcggttcgcgctatgcggatgatgattattggccggaatacttcagcgactacagcgaagcgcgcgagcaatgggaaaacgacaaagcaaagatgcgcgcgcgtctgcgcgagatgatcgcgaaccgtgcgccgctggaattgcgcgccgcgcttgtcgcgagcgtgtacggcgagcccggccgcgcggccgatgaatccgaagattgaaagggagctaacgacatgacgacgattaccgcatacgcatacaatgccgcgcttcattgcccgcgctgcgccttccgttatttccgcgtcgatcctgcgaaggtgccgccgggcgcggatgcgctggacggttgcaaggatcgcgaagggaacgcgcccgcgccgctgttttccacagacgcgaacgcggacggatattgcgacacttgcgacatggcatacggcgacgcggaaccgcgcgcgcacgtcctgagcattgacgcatggcgcgagcccgaaggctggacgtggaataactggcacaagcgcggcacggtgccggttgcatggtgcgacctgagcccgcgcgcgttgctgcggaacctgcgcgcgcacgggctcgacctgccgccgggcgcggtatgcgtcgaggatgacggatacaacgtcgagattcaggcgcgcggcacgcgggaaccgttgtacgccatcgcctacggcgaggcgcagcgatgagcgctaagcccgacctagcagaaaagcgcgaagccttgcgcgctggcattctggcggatcgcatcgaacgcggcgcgcgctggctttgtttcgctgccatcgtatgcgcgggcgcgttgccgctggcctggggagcgttccgggcgcatggcatcgttagcgggctcgccgtgctggcgctggtgctggcgctatgctggcacgttaagccgcacgggcgcagcctagcggcgcaagcgcgcgagattgaagcccgattcaagccgcacgattaaaagcgcgctgcggcgcgttccctgcatcgcctaccctgagcccggccgcgtgccgggctttttattgcctgcgcgtctaggcgcgacctagcagccttgccggccgcacgtctgcccggccttccgtatcccttcgcctgagcccgtgcccgcatcgcttgcggccgggcttttctttttcccgctgcccggccttgctcgggctcgcatgcgtgccggcctgcccgctgcccggccttacatggtcgcgggcttatccgctgcccggccttgcatgcgtgcggcatagctgcccggatgcggcattgtggaattaacgcattgcctgagcgcataggcgcgcgcgtgcggcctttccgaatttatttattgcatcgcatgcccgcatgcgtgcgcgccgcgctgcgcgcgttgtggcgcggcaggaagggataaagggatagccgctaggcgactaaaaaggtacttccggcctgcgcgaaggcgtcgcggggggcgctgaccgatcgga

SEQ ID NO: 4 - DNA, 20 bp, synthetic construct
  source 1..20: mol_type = other DNA
gcgcagtcatgagatcgaga

SEQ ID NO: 5 - DNA, 20 bp, synthetic construct
  source 1..20: mol_type = other DNA
gttgagtgcaccgagagtga

SEQ ID NO: 6 - DNA, 20 bp, synthetic construct
  source 1..20: mol_type = other DNA
tgggtcacttcggtgttacg

SEQ ID NO: 7 - DNA, 20 bp, synthetic construct
  source 1..20: mol_type = other DNA
gtggtgaaaggtgcggtttc

SEQ ID NO: 8 - DNA, 20 bp, synthetic construct
  source 1..20: mol_type = other DNA
cgtagtcgcgattgtcggta

SEQ ID NO: 9 - DNA, 20 bp, synthetic construct
  source 1..20: mol_type = other DNA
accactgctgacgttcgatt

SEQ ID NO: 10 - DNA, 20 bp, synthetic construct
  source 1..20: mol_type = other DNA
gctaccggtacgactacgtg

SEQ ID NO: 11 - DNA, 20 bp, synthetic construct
  source 1..20: mol_type = other DNA
gatctggaaacagccgtcca

SEQ ID NO: 12 - DNA, 19 bp, synthetic construct
  source 1..19: mol_type = other DNA
tttcggtggcttggatttt

SEQ ID NO: 13 - DNA, 20 bp, synthetic construct
  source 1..20: mol_type = other DNA
atttgcgagaagtacaactg

SEQ ID NO: 14 - DNA, 20 bp, synthetic construct
  source 1..20: mol_type = other DNA
atcccctttgcatcttcaat

SEQ ID NO: 15 - DNA, 20 bp, synthetic construct
  source 1..20: mol_type = other DNA
ttccgtcatctaagggaatc

SEQ ID NO: 16 - DNA, 20 bp, synthetic construct
  source 1..20: mol_type = other DNA
taagcccttcgtaaagttct

SEQ ID NO: 17 - DNA, 20 bp, synthetic construct
  source 1..20: mol_type = other DNA
aagcattgaaaaacgaaacg

SEQ ID NO: 18 - DNA, 21 bp, synthetic construct
  source 1..21: mol_type = other DNA
actaggagaagattagatggc

SEQ ID NO: 19 - DNA, 16 bp, synthetic construct
  source 1..16: mol_type = other DNA
ctggtccgtaagggtg

SEQ ID NO: 20 - DNA, 20 bp, synthetic construct
  source 1..20: mol_type = other DNA
gatatacgagcaacgtcttc

SEQ ID NO: 21 - DNA, 20 bp, synthetic construct
  source 1..20: mol_type = other DNA
atttgcgagaagtacaactg

SEQ ID NO: 22 - DNA, 20 bp, synthetic construct
  source 1..20: mol_type = other DNA
gttattgcgacggttaaaga

SEQ ID NO: 23 - DNA, 20 bp, synthetic construct
  source 1..20: mol_type = other DNA
tggattaaatactacgccga

SEQ ID NO: 24 - DNA, 20 bp, synthetic construct
  source 1..20: mol_type = other DNA
ctggcaaaacaacctcatta

SEQ ID NO: 25 - DNA, 20 bp, synthetic construct
  source 1..20: mol_type = other DNA
agttaccacgaggatttcat

SEQ ID NO: 26 - DNA, 19 bp, synthetic construct
  source 1..19: mol_type = other DNA
gtagatgttcggttcggta

SEQ ID NO: 27 - DNA, 20 bp, synthetic construct
  source 1..20: mol_type = other DNA
caagccaattcacatcgtag

SEQ ID NO: 28 - DNA, 20 bp, synthetic construct
  source 1..20: mol_type = other DNA
attctgtttcaacaaccctg

SEQ ID NO: 29 - DNA, 20 bp, synthetic construct
  source 1..20: mol_type = other DNA
cagacatccaggaacttttc

SEQ ID NO: 30 - DNA, 20 bp, synthetic construct
  source 1..20: mol_type = other DNA
catacctacgatatacggca

SEQ ID NO: 31 - DNA, 20 bp, synthetic construct
  source 1..20: mol_type = other DNA
gactactcgctctacatcaa

SEQ ID NO: 32 - DNA, 20 bp, synthetic construct
  source 1..20: mol_type = other DNA
atggcctttcttcattcttg

SEQ ID NO: 33 - DNA, 20 bp, synthetic construct
  source 1..20: mol_type = other DNA
agaaaatatccgggtgtgat

SEQ ID NO: 34 - DNA, 20 bp, synthetic construct
  source 1..20: mol_type = other DNA
tagattgtgattcacgcaac

SEQ ID NO: 35 - DNA, 20 bp, synthetic construct
  source 1..20: mol_type = other DNA
gaagacgaaaaggcaaaaac

SEQ ID NO: 36 - DNA, 20 bp, synthetic construct
  source 1..20: mol_type = other DNA
atattgaactccgaagtcgt

SEQ ID NO: 37 - DNA, 19 bp, synthetic construct
  source 1..19: mol_type = other DNA
ctaccaaactgggggatag